European Patent Application EP 4 636 085 A2, published October 22, 2025. Title: COMPOSITIONS FOR MODULATING MECP2 EXPRESSION. Applicant: Ionis Pharmaceuticals, Inc. The sequence listing filed with the application follows.

SEQUENCE LISTING (340 sequences)

SEQ ID NO: 1 - DNA, 80001 bp, Homo sapiens
  source 1..80001: mol_type = genomic DNA
gctaccatcaactctttctcctagactgttccagggccttgcaactagccttgtgctgtagttttgtttcatcacgtccagttctccactctacacctgcaacatagatcagacagctcctggctcaaaatcctctgagggcttctcatcttagaataaactctcggttctggccgggtgcggtggcttacgcctgtagtcccagcactttgggagtccgaggcgggcggatcacttgaactcaggagtttgagaccagcctgggcaacatggtgaactcccatctctatcaaaaatacaaaaacttagccaggcgtggtggttcgcatctgtggtcccagctacttaggacgctgaggagggaggatcgcttgagctcagggtggacgttgcagtgagccaagattgcgccactgcactgcagcctgggtgacagaatgagaccccatccccaccccccccaaaaaagaatgaactcccagttctcatagtggccccagctgcctttccaatcacattccctaccactctccagcaacactgacttcctcgttagtccccaacatgccaggcatagtctctcctcatgtcctttgaacttgcctggaatgttctttccccagatattcatatgagggagtaaaatgagggtgaaaaccagcagatatctaaatagcacccccttcacttagtttatctttctcaaagcccttatcactatgtgaaatgatatattatacttatttgtatgctagtatgaatcttcccggcaagaatgttagtttgctgtctgttcagtaccgtgcatccagagcctggaagagtgcctggcacatagcaggtagtcaataaatgaatgggggcaagcagccaaatcagaatcaggttttcttgctaagcatagaactaacagaaggatcattgaatggattggataatgactggcatcagggtaaggtccccttaacaaacactcctgtcctgaacacctggttagctaacagttttctcatactcttattttcccaaaacacaattgctggatctcagctccaaatcaactcttctaggaaagtgaaaaattgctggatctcagctcccaaatcatatcttccaggcagagctaacattgccccttattcacacctccaccaaaccatctgatccaacagtgacaggtgtcacgaggccttggcatgcactctcttcccccgccagagttctgcgaaagccagggttgcgatttgttgtcagtttattccccgcctctatgagagtgtgagcactgggcaggctcggatgaaataatgcattgagtaggcctctgaaaccaaggcccctcagctggggcaacgtcaggctccagggtgggcaactttgctgcttctgccgaagatagtgatattgagaaaatgtgggtgcaatgaaacgcttattgcagcgcactcggtgcatctgtggacagagggtcaatcgcccctcagagcagcgcaaacaggcgtcccaagcctaggccttcacttgccccagcatccgcaagggtccattaatccttaacattcaaattccgcccactaaaccagtccctccgcgcccaagccgcctcttttccccaaacgacggccgaaagcagccaatcaacagctggaggggtccgcccccttttccctggccgaaatggacaggaaatctcgccaattgacggcatcgccgctgagacctcccccctcccccgtcctccccgtcccagcccggccatcacagccaatgacgggcgggctcgcagcggcgccgagggcggggcgcgggcgcgcaggtgcagcagcgcgcgggccggccaagagggcggggcgcgacgtcggccgtgcggggtcccggcgtcggcggcgcgcgcgctccctcctctcggagagagggctgtggtaaaagccgtccggaaaatggccgccgccgccgccgccgcgccgagcggaggaggaggaggaggcgaggaggagagactgtgagtgggaccgccgtggccgcgggcggggacccttgccggggggcgggggtcaggggcgggacgtggcgcgggaggggcccgcggggtcggacgacacggctggcggatggcgtccctcctctctaccctccccctcccgccgccgccggtggcgactctcccctcggcccgtcacccgtgctcgcgggtgaccgtcctcggcgcggcctccctggagccgccttcgcctgacgcccctcttcctcccgccctcgacgcgcatcccggcccccggccccgcgggcgcccctgtcgccggggttcgcctgtcggggctgcgcgcgctcctgcccttctcggggctttgggccgcggcgccgtcgcgcgcccgcggccccggcctctccctggatcgcgctctccccctccctccctcgcgcgccccctctcccgttactcggcccccccaccggcgcgcgtgcgcacttcgcctcccgtcgggagagtgcgccacaagggctcctgagctctcacccccatctctgggctttgcctccccctccttctcgcccattccatgaatttctgccccccgctacccccccgcgagcgagtaggtccaccggctcctttccccatctagcaggaacaagtaggtggggattattatccacaaaagggactagacattgtgttctgggtcccacaactcatcataaagaggtggttatagttcccatcaggagccgtgggtaggggactgtgcgtccagcagcacccgaggctcttcggcgccagaggctctaaggtgcgagcgtgtccccagggtgctcagaggttctttggagtgctgtggcctcggaatgtgagcaccctcccatcctaccctccccttcgccggcgatcttccagttacataagtggagtgggacatagtaggtaacgggctctcatcgccctggagcgctcgggatcaccggtaccagatggggcaagttcatcgcgacgctgtggctcctgttaattgtgcctgaaaggttatcctctgttcagtttggtcatgaccgaatcacccaaactgaaactcagatgacttttatatggcagtggcaatgtttctgtggttttgcactaaagacttaaggtcattatgaagagtgtaaaaggattgctgtcgcaggggagaccgtttatgacattgctaagtatggaccccgagggggaaaaagctcattctggaattgctctgtggcggttgcttctgttgcgagtgtgttcgggtgtgggttggtcacagcagaaatgggctccaccacaaaattgatattcctgactcatggtcaggcagatgtgtgcttctggttatttttccaggaacaggaatgggctctgccgagcctttcacacgttgtgtctctgctgtgcgggatcagtaccccagactgtgagataacaggatcgaattcaggggttggttggtgatccaggaaccatacctacttggatgtgatactgagtggcctagacgttgtaggactctcataagttttagacattttgttatactgtaaaaatgaagcatatacggcctcagtagtaacattgcactaataggtaattattactctagagaattttgggttccatggctggaatgttcatcagtatctcagcaatttcagttaataaccagattaagctgacctcttgagtcttttgaaatctgctgggtccctataataagacagggtctggattttttaatcttttgggaatttccaccaaggatttagggaaataggcttttatgggcttttcaggatttctatttcaaatcccaatgaggaagtctaggaaacacttgcttttattttcttgcctgaatatgtcagaaccttaaatcacccaatcaatctagaagtactacagttgattaaagtaagtcaccacaggtcacccattcgtggcaggtcagctaggtggctgatcactggaatacagtcatatccccaggcatacacacgagcctcacttgacgatcccaaagtttgtacatctgagcttgagacgtgacaagttgaggtctctgctttgttcttcatagttggcagtttgtctcctcgggtgcccctccggttagctgtttatcatacgtctagccctatcaacagtgcaggcagcttccagagtatagttttctctgcaaagtgcctggtggaggggtacctccttttccattgtcctaatggctccactgggcttccataccagccctttccagtgtcttaacagctcaaagaaacccatctgtggctttcttgttagcactggcctatcacaccttcctattgcctgttaactaaaattttgcctggaatgctttaagcttagagtactgggtctttgtttcacccgattgataggagagtgtcatgcagtcagccgaactccgacttctgtgctgtttaaatccttaggtaggtctggggcaaggcacaaaccactgtgtattcaaagggttatggtgcttgcattctgtgtgtatatgtttgtaatttccaaccagagtcgtttcccgtgcctgccctgcctctgtgcaatctagtctagtagggtagggaggcaagctgtggagtttgaaaaaaaaaaaaaaagctagatgagtttaataggctgttaccccctccagaacattcctcccatgtggagatgaaacgagaagttcatttctttaacctaaaataaagaacaacagagataaaattgttagttccttattggagcctggtttccattgctaatgtacctgcttgggactctgcatgataaatgacgtgtcctggaacctgaaatcttttataaaggttaatatcagcagaaatcttttaattagctaagagcagcttgttctcaagctgcccgagttatcttggaggagagaatcacaggaaatgtttgatatttctagtaaccagtgttttcagtgcgtggggtaaagcacactcctagactggccagtcccaaagagtgtggcaggacacctgcttgttttccctgccctctgctatggtgacatccttgcagaccagtcttgcgtggctggcagacgcaatctttttttcttgggtagagcattatcaccgctgcgatggaaggaccttgtcctcggtgcctccataccagccctttccagtgaaactactgctgtcccggcaagcccctgtgcgtgtgcatcattccgggtaggacaagatgtgaacaggtccctcttctttgggcttaagtagaagttgtgctcttctgcttttacctgtgtgctcttctgcttttacctgttctcttctgcctttctcttgcaagaaacctgtcgaaagcttgctttgcatgccattgcttaaatactttgatggtatgtatggtatgtgggataactgagtgggagccggaattggggggtgggcagggcatccccacccccacccccacatcaaagggggaatgaccatttcgttagagaataaagcctgagtcttataacttcttcaagcacatgtatgctgggtctcctggcgtgtgaatgtgttcccgctgtgctgtgtggctgttttgcagttactgtagacactgtagtctgggctctcattattgcctctgaagttgacaggaccaagccttagtaaggatgcacttgtcttcctagcccaagagctaggggtgttttatatatatattaactttcttttttagatttcataaactgctctcattttctcttttctttctttctttttttttttttttttttgagacagtctcactctgtcacccatgctggagtgcagtggcacgatctcagctcactgcaacctctgcctcccgggctcaagcagttctctgcctcagcctcccaagtagctgggattacaggcacctgccaccacgcctggctaatttttgtattttttttttttttttttttttttttttagtcgagacggggtttcaccatcttggccacgctggtcttgaactcctgacctcgtgatccacccgcttcagcctcccaaagtgcagggattacaggcgtgagccaccgcacccagcctctggctcttttctttttgacatgaaatcttaagttaattatcttaaactttaagaactagaaggattcttagtccagcaccatcagtttacaaacaaaaaaaacttgtgtccctgagaagttgtgacttttccagggcctcctagccaggataccagtttggtttttattatatagctagccgagtaatactattaacttgacttctgggatttcaaagtattctatgacttgactgtttaagggaattatgaggcctcactgaacctcaaaagataattttaggtaccatcctggtagctgtagagcagcaacagaccagtaaaagacttggttggtgttgcccttcttctgggtttgattacatgagtaattgtgtgaatagtctctaagttgtatgctctgagctttcgtttttagcttataaaagtgctactcttgggccagcatagtatcagaaattagctaattcatatggggcagtttaggctttaactaggaaatgatggttatcttaatgacaaaaaaggtactgacaaaagtccttttttgaacatgtgttcaaaagaaaaagagaaactatcaaactaataactgagtttgttgaacatcgagattgactgatctgagaggcttaaaactgattgccctgaaatagacttgcatgttttggatgatggctttgggtctcccagagcacttggtttcccttggtgctgattttttctctcaggattaaagcccctttatgtgatgttgttacagcagcttattgcaacttcattcagctgcttgaaaaagaagggagactgcctctaggttccatgtgttctttcagggatggtattttgatgttgcgtattctcttgaacatgtattcttccctgagaatttctgtgtgccgtggtagaagaaatacttgccagaaatcgccactcatggtatgcttttgtagtgtcgaagtgtcccctagaggtgacaaggcttgtgatagtgttgattctaacaagcatgaatctttcctttattttagcactgtgtgttacgtgccagtaatttgcagcttatcctttgtttctagctaggtaagctgggaaatagcctagtactttgtctatgtgtttatcttcaaaatgtcccaaatagccctgggaaaaaggtcgtgcagctcaatgggggctttcaacttacaattttctttgttttaggctccataaaaatacagactcaccagttcctgctttgatgtgacatgtgactccccagaatacaccttgcttctgtagaccagctccaacaggattccatggtagctgggatgttagggctcaggtaagtaaccttcctttttttttttttagtatatgtcctggtttggccatctgttttttttttttttaaaaaaaaaaaaaaaaggaaaagaggaaaaaaatatactactcttggacagtataaaagtaccccaaagactaaagacataactgtgccaaactgtgccatataataaaaaaaagtcacttccctgagccctgaaaggtcagtgtgtgtagggttacttggtcgccacagcgtgatctgggggcgggcgtcagattagagccggaactggtgatctgcaacttcagttcaccttgaagcaggtcagctgagctgagagcgcttgcactgagcccttttgcgctgctgctgttgccttagcggtcttcagcatgtgtttgctttggtttggggtaaatggcttagtggtcaacattagtgagcagtggtaatgcattttcagatatgggaactggtatgtggttggttccctagaaggacaccctcctgaaagctgtctcagaacaccgggggccatggctaatgtcatgtgcttgctacactcctcccatggtaactaaagagagtacccagatatacatctggttcttgggactctagaggaggatgagtactttgtaaaaacctgggggccccagtcattctaggtctgacactcaggtgctgtatcagctgcagtttgaactacttggcaccattgtgtggactttagttttgtaaaaatgaatggttccttaatttctcaaccttcaggctcaacatctcaagctgtttgttgttgttgttgttgttgttgttttgttttgtctttttgattagtggtcactccgcatttgatgttttgacatgtggatttcagaacttctgtgtggtaaagcagaatgttccaattgaattttcccattttttttcccctaagcaaaaatgtgagttttcacttatgcggccattgtgattccgactgagaccctaagtcgttctttgttgtctctctagtggtttctgacacctcagtgtgaagctgttgtagacatccataagaaatagcctgcttagggattatgtgagggcaaggtttggctgaaggagaatagaaggtgtggaaggaagcggaagaccagaagagcatcacactgcctcaagtcccaaatttgattctgctcctgatcctgtgactcaaattgtcattctcttttactgctgtggggtgtgctctgggcccagctgacaggacattctttgtactccacgtatttatgctggtgggagttgtatggctagtgctttgtgctttgtctcagaaattgtgtggactaaatgtaatatgggcagtgaatgggtttcttctggaagatgttaggcctggagggtggtttgggtttttacgagtctttttctcagattacagattacgaatggatgttataaaacaggcagtgttgacaccatacagtttctcctaagaaatgtacagagagttcaacctgaggaagctaattgaaaataaacttttaaaaagaaatgtagaaagaggaaatttaaaaagtatcttatgaatgggaaagatgtagccatttgagcttcaaagaacttttgagggaattctcaaaggacagtacccgtctttagtagataaatgcttgatatctatttttcttcttttactttttaaagaattactaaaataatacatggatttatagaaaaatcaaaccacttaaaaattgatcaggtggctgggcaaggtggctcatgcctgtaatcacagcgctttgggaggcctaggcgggtggatcacctgaagtcaggagttcgagaccagcctggctaacacggcgaaaccccatctctattaaaaatacaaaaattagctggccatggtggcttgagcgtgtagtcccagctactcggaaggctgaggcaggagaatcacttgaacctgggaggcggaggttgcagtgagccaagatcacaccactgcactcctgcctgggtgacagagtgagactcggtctcaaaaaaaaaaaaaaaaaaaagtatcaggtaaaaaaatgaaagctccccgcttaatctctgctcccactacccagaataactgctgttaatagcttaatgtagatccttctaagtcttctaagactaaactgtgtactttttgtgttgtaattaacaggagggtttttgttttgttttgttttttctttttttgagatggagtcttgctctgtcatccaggctggagtacagtggcacaatcttggctcactgcaacctccacctcctgggttcaagtgattctcctgcctcagcctcctgagtagctgggattacaggcgcctgccaccacacccagctaatttttgtatttttagtagagatgggtttcaccatgttggccaggctggtgtcgaactcctgacctcaggcgatccacctgccttggcctcccaaagtgctgggattacaggcgtgagccaccgtgcctggcctcaggatggtgttatatatacatattctgcatttttccatctcatatattcatctctgcctcatttcttttaaatagcagtgtagtccagggctgacttaccgtcatgcatttcgttgtctctctatgttattaaaaatgctacaggattgaaattcctcatgtgccagtcattttgaagaatggctgcctagacttggaatttctggtggataccaccacatcactgtccaaaatggctatcccagttcccacaacagtctgagaaagtgccattttcccatatcgtcccagaattggatatacatcttttaaattggtgccgcttggattattactgaggctaaacctcaataatcattgtcatagctcttaatgtattaaagatgttaactctttgtcatgcagatattttcctgttttgtcttacgtcttgattcttgtctttctgatatataaaatttatgttatgatttattcttttgctttcatacttaggaaatccttttttactctttttttttttttttttttttttttttgagacggagtctcgctctgtcgcccaggttggagtgcaatggcgtgatcttggctcactgcaagctccatctcccgggttcattccattctcctgcctcagcctcccgagtagctgggactacaggcgcccgccaccacgcctggctaatttttttgtatttttagtagagacagggtttcaccatgttagccaggctggtctcgatctcctgaccttgtgatccgcccgtctctgcctcccaaagtgctgggattacaggcgtgagccaccgcgccccgccaggaaatcctttcctactcttaacaacagatcaatagtcatctatattttcttcctaaaaaacctgatgatgtattatattcatacatacgtatttaatacatacaaaagggccagatgcggtggctcatgcctgtaatcccagcactttgggaggctgaggcgggtggatcacctgaggtcaagagttcaagaccagcctggccaagatggtgaaatcccgtctctactaaaaatacaaaaattagccaggcgtggtggcgggcacctgtaatctcaactactggggtgactgaggcaggagaatcgcttgaacccaggaggcagaagtttcggtgagccaagatcacgccactgcactcctgcctgggcgatagagtgaggctctgtctcaaaaataaaaaataaaaataataattttatagttaagttgccctgtgtttttcctgtgattaaaaaaaaaaatacctgttttgtatttaactttggggtgggataaggtatagcccacttagtcagttgtgtctaagccacttgatgaaccagtcaatccagtcttcacctttaacaaatgctgatttcttcaagtgagcaaaatatctcttaaactttttcctattttctctataaagttgcttttttctgaattttttctttatgaggcttgatgggcagccctatcagcagacaatcattcattcacccaacaaatatttgagtatctgcttcaagccaggggcagtgctaagccctggaagtggtatcttctccttatccgggagtggggctacagtgttcattccagaagactcaagaaaatagcagatcatcacaaaagtaggttttacataaatgaggaggaatccacagggttgtgtatatgtgtgtgtattttaaattctgacataagttggagctttagggtagactgtgacataagagtagtttgttttccaactcatgtaattgccggctgatttttgtcttgaattatgataatggtaacttctgttgaaacaattctgtattcatcttagcttggttgggatgcaataaaagttttgtactggtaaaaatgataattttcttccatgatgattttgaagcttttctgtaacacctgataaaaatagaggggccaggcatggtggctcatgcctgtagtcccagctactcgggaggatgaggtgagaggatcccatgagcccaggagttttaggctacagtgagccatcatcacaccactgtactcctgtactctagcctgggcagcctcgttctttagagtaagacactgtctctttaaaaaaaaaaaaaaagaaaaaagaaaaaaagaaaaggcttttagtgaatatatttttagggtagcaagtgtaatttttataaattgcattatttgaatctaataaataccctcaaagctgaagtcgaattctgattttgattgaaaatattttttacttaaaggaagagggatagaataaatgacacgattaaggaaaagacttcttgtataaggccggggttttttaaatgattttttgaatagttagatggacaatacggaattaaaaaggtggtgtaaaaagttatacggggctgggcacagtgactcacgcctgcaatcccagtactttgggaggccgaggtgggtggatcacctgaggtcaggagttcgagaccagcctagccaacatgacgaaacatcatttctactaaaaatacaaaaattagctgggcttggtggtatgcacctgtaatccagctactcgggaggctgaggcagaagaatcgtttgaacccaggaggcagaggttgcagtgagccaagatcgtgccattgcactccagcctgggcgacagagtgagactccatctcagaaaaataataatagaaaaaagttatatggggctgggcatggtggctcatgcctgtaatcccagcagtttgggaggctgaggcagcttgatcacttgaggtcaggaattcgagactagcctggccaacatggtgaaactccgtctccactaaaaatacaaaaattagccaagcgtggtggtgcgtgcctgtagtcccagctacttgggaagctgaggcaggagaatcgcctgaacctgggaggcagaggttgcagtgagccaagatcatgccgttgcactccagcctggacgacaagagcggaactccgtctcaaaaaaaaaaaaaaaagagttatattgtaaagtatctctgctaccctgccccaaacattcatttctttccctggaggcagccactattacctgtttctttaaaaaaaaaaaaaaattgtggccgggcacggtggctcacgcctgtaatcctagcactttgggaggtggaggtgggtggatcatgaggtcaagagatcgagaccatcttggccaacatggtaaaaccccatctctactaaaaatacaaaaaattagccgggcatggtggcgggcacctgtagtcccagctactcgggaggctgaggcaggagaatcgcttgaacctgggaggcagaggttgcagtgaactgagatcacgccgctgcactccagcctggcaacagaatgagactccatctcaaaaaaaaaagcgtgtgtgtacccgtgtgttaaatttttattataaaatatatataacaggctgggcgtggtggctcacgcctgtaatcccagcactttgggaggccgaggcaggctgatcacgaggtcaggagatcgagaccatcctggcgagcacggtgaaacctcgtctttactaaaaatacaaaaaattagccgggcatggtggcgggcgcctgtagtcccagctactctgagagcctgaggcaggagaatggcgtgaacccaggaggcggagcttgcagtgagccgagatcgcgtcactgcactccagcctgggcgacagaccgagactccgtctcaaaaaatatatatcgatatatataacaatttacagttttaatcatcttaactgtacagttcagtggcactgagtacattcacattgttgtacagccattactaccatccatctctacaacctttcgtcttgcaaaactgaaatttcatacctattaaacactaactcccacttctcccctttcccccaccccaccctctggcaactactattctactctttgtctctattggacatatttttgtgtgtttaggtttgtgtatatattttacatgtgtgtataaatacacaagggtatgtgggcgttgtgtttttacacatactataaaatattgtgcacatttgtttattttaatgtatcctgtagattatttagaatcggttcatacagagccgtatcattccttttaagggttgggtttaaatagtctgttatggatgtaccacaatttatttaaccagtttttaaattttttacttattttttttaatgtttttttagagacaggatcccactccatcacccagactggagtgcaacagcatgatcatagcttactgcagccttgaactccggggctgatgtgatcctcccacctcaggctctcttgtagctgggactacagggatgtgccgccatgcctggctaaattttttatttttatttttatttttatttttggtagacacggggtttcactgtgttgcccaggctggtcttgaactccttgggcttgagtaatcctcctgccttggcctcccaaagtgccgagattacaaccatgagccatggagcccgacaagagtagccttttatttgcagaccattagagaaaaagttgcgtgtaagtagataagcatacgaatttatcactgcaatactgtttgtagagatcacagagctgttaggctaggaagaagtttttagcagttagcactagaaagcaaaactttggaaacttccatttcatcaaaagtgacctcatctgagtagggcatgtgagggaaggacctttttactcgacaaggggaacttgccagttcttgtttgtgaaccttgaagaaagtggagcatttttattttgggaccattctaggttgtggtagttccttggtactcggggttggagaatctccctctgctgctggaccttctgcctcctcatgctgtaatatgcataagaggtgtcctagaagtattcaggaacaggctgtggttgctttgttgttctgtgactgttgaactctttatatagcagtacttttttaagctgtactaattgagcatttattatgtgtcagttactgtgctagctgctggaaactatcctaccctcagcagtcttctggtctaatgggaggtacagacaggcaaatgggctatgactttacaagaggctaacttctgtgatggagagaagttccagccactaagggagcacataaaaatcagaggagatcctaccaagaattgggaggtaggtcagggaggagacttctttgaaaaatggcatctaagacctgaacagcaaggaaacattagctaggtcaaggacaaagcatcagtggggagagatgcatgagtcttttggaaggaccagcatgtgtagaggctctgacaggagagaatctctcaggcccattcagagagtccactgtgtgaagacgaggcatgaacaaccagccaggacatgtggagaggagcatttttctttttttcttttttctttcttttttttttttttttttttttgagacgtctttctctgtcacccaggctggagtgcaatggcatgatctcggctcactgcaacccccacttccagggttcaagcaattcttctgccttagcctcccaagcagctaggattacaggcacccgccaccatgcccggttaatttttgtatttttagtagagacggagtttcaccatgttggcctcaaactcctgaccttaggtgatccacccgtctcggcctcccagagtgctgggattacaggtgagagcccccacgcccggccaggctcggctttctttccaggccccgtcacactcttagatgttccctgggccccagaaggcagcgtgaggtgctctgcccatctatgctgtccttttccaccccaccctatccactgggcccctggggctcccactccactccaggtctcttcatggacccttctttcccttcacttctgtcccaggagacctgggagactcatgggaacaggcatcatcttctccagcacagttcattgtctaatgcacgaaagtgctgggctgtgagaaggtcaggagcttacatggaatgggagtcagctgtggtacaaagtacgctgcttagttctactgattttttattttttatttttacataagactttgatggtaaaggaagcagtgtgtgagcaagctgactcctgtcttgtcaagtaccaggtccactctgatgagcccctgtggacagcactgctgtaactccccaagcctgggctcaggaggtgggccctaagcgctgttcccagctcttcctccatgctgtcagctcttccaccattcttcctggcgtcattctaaggtcctgtcttcccccgccctcttccttcctggcttctacgctcagctcaagtagtagctgtttgggtacttttcacccagacttaggaaatgttatcagttggtcgtattcctgtcagccctcttactatggaactcaaataggacagattcagctgaattcccagccctgtggttgcactctttgtctgccctgcttccccaaggtagcctgctccctaaaggtcaccgagatactccccatgcaaggtttttgttgtattacacatgacaacatggaataaagtgttttgcaaatttactggatgatatcctactatgtggaacatcctacaacttactcttttcactcaacatttgacttttgaacctggtctgtattgctccgtgcagaccaatgttcattcatttgatatgtctccttgtgccatagaaatagttttacaatagaagcctgtccagagccatgagggagaaggggattgtagagaaacaaggattggcatctggtttatgtttacatcctttagtcctgttaaccgagaagaagatatttttatttccatgtttgcgaaagctttccacaaaaaaaagcatccattttctagacttattaatagggcagtccaaaggttttatttttagatttgaaagaaagcaaagtaggcttctgagatatgcacatttccctgtgtccctgtctcttttgcaacattccacattgctgctaaaacttgaacatgagcactttcaagcatgtgcttactttctatgtatgactcattttttaaaacattaaagcattttcggccgggtgtggtggctcacgcctatattcctagcactttagaaggccgaggcgggtagatcacttgaggtcaggagttcaagaccagcctagccaatatagtgaaaccccatctccactaaaaatacaaaaattagccgggcatggtggcgggcgcctgtaatcccagctactcgggaggctgaggcaggagaattgcttgaacccaggaggtggaggttgcagtgagcagagatcgagccactgcactctagcctaggtgacagagcgagactctgtctcaaaaaaataaaaataaagcattaaagcactttgtctggtggtatgtaagttttggcattacttagataagttgtattttaagtctttctacacacaataacttatttttaaaatacaagtttctgtgtacttccgggttttgtgtttttgtaaacagcagaaggtattagtccatattaagtactaatttgttctaatattttcagctgtttttggaattacacttggcaaaaaaatagacaaatgtctgcagttgtgacagtttgtttttttgttctttttaactccagaataaataattctagtgagtttttttcttggcttgtaagaacatgggaatgattagagtcatcataacacttaagtagttatagaaggttgaacatctgtagtcagttgtataaaatttcctagtcatccttccaggttgtttaagacaaacaaatacatagtatttattaagctcttataaattttaattgtaaaacatcattgtacaaaactttgaaaatgcgtataggtacaaagataaaaaattaggccaggcatgccatggctcacgcctgtaatcccagcactttgggaggccaaggtgggaggatcttttgagcccaggagttcaagaccagcctgagcaacatattgagaccctatctctacaaaaatatcataaaacaaaatagaatcactctggcgattccactatccaaaaaaaaaaaaaactgctgttaatatttggtatgtatctttctagaccaaggcctccaactttggttgagaattcagccgggtctgtgaccttggatgggaaaaacattcactctttattttcactaatgtctctgaaaacccagatttttagctgggcatggtggctcgtgcctgtaatcccagtgctttggaagcccgtggagggcagatcacttgagcccaggagtttgagaccagcctgggcaacatagcaagaccctgtcttttaaaaaaaaaaaaaatccagccgggtgtggtggctcatgcctgtaatcccagcactttgagaggctgaggcaggcagatcacctgaggtcaggagtttgagaccagcctgaccaacatggtgaaatcctgtctctactaaaaatacaaaaatcagccgggcatggtggtgggcgcctgtaatcccagctactccggaggctgaggcaggagaatcacttgaacccggaaggtagaggttgcagtgagccaagatcacaccattgcactccagcctgggcgacagagcgagactctgtctcaaaaaaaaaaaaaaaaatccacattttcttcaatgacaattgtaagcaacagatcatggtagtattagaatagcagtgactgtcaccagtagagatcaaagatactttcatatcatattatagttgttacagatattttgaaatatatatgtccatcactgcttcaaacttaaggtaattattagacccatctctagatctggttatttaatgatttactgaagaagcacatattatttgagaacgaactcttgaaatatgttgttaatttctgtgcattttacacatttcaaaacattcttctgaggaggggtccagaaggccaaaagggtccatggcagaaaaaggttaagaacacctgttctgtactttgtaccatgtggctacaaatataaaaacagacgttaagccgggtatggtgatgcacacctgtagttccacctacttgggaggctgaggtgggaaaatcacttgagcccaggagtttgaggccagcctgggcaacagagcaagaccccatctcttaaaaaccagtcagcacttgactagtcagttagtgggggaaaacacaggtacagtaaaaggagtcaaaattacacttaaacttaggtcatcttattatatcaaacatttattaacatgtttagtgttttgtgtatattatgcaaagtgtaatgcaactaaaactgtttaacacttctcgatatcacataaatttgttggtgcataatagcctaaaagttacttttgctgttggcattttattttattacttacttatttatttatttatttatttattttgagacagagtcacactgtcgccaggctggagtgcagtggtgcgatctcagctcactgcaacctctgcctccctggttcaagcgattctcccgcctcagcctcctgactagctgggactacaggtgcgcgccaccatgcccagctaatttttgtatttttagtagagatagggtttcgccatgttggccaggatggtcttcatctcttgaccttgtgatctgcccacctcggcctcccaaagtgctaggattacaggcatgagccaccacgctgggcctgctgttggcattttaaacatccttctagagtctttcttatttgcctgtaagcacgtacacatgttgttgttgttttgagacaaggtctgtcgcccaagctggagcacagtggtgcaatcacagctcactacagcttcgacctcttgggtgcaagtgatcctcccaatcagcctcccaagtaggtgggactacaggtgtccgctaccatgcccagctaatttttgtattttttttgtagagacggagtttcaccatgttgcccagactggtctcaaactcctttgctcaaacgatccttccgcctcggcctcccaaagtgccgggattacaagtgtgcacctctgtgcctggcccacatattgttttagatgaatgagatcatatatgtacttttgtaacttgctacctttcctcaacaaaatgttgtaaatatccatgtccataaaaatagacgtatatcttcacttttccctaaaatgaaaataacttaacttgcattttcttttttgtttttgtttttgttttgagacaggctcttgctctgttgctcaggctggagtgcagtgatgtcacagctcactacagcctccacctccagtttcaagtattccacctacctcagcctccaagatagctaagactacaggcacatgtcacgacgcctggctaatttttaaaatattttttgcagaaatgggatttcactatgttgcccaggctggcctcaaactgctggcctcaagtgatcttcctgccttggcctcccaaagtgctgggattacagtcgtgagccactgtgcccagcctgcattttcttattataaaagtaatacatgttcaatggacaaaaaattttcagaaaatatgcaaagatgaaaagtaaaaattgtccataaatctgtcatctacagataaagataacttctggataatgtttttctaccatcatttttagtaatcacataacatttcgttgtatgtctatgccttcatttaattaagaggcatttccattatttctgcatgttcatgactctgaatgatgatatgtctgcctgctgatggctacaaccctgtttctgcatttcaaacctctctcttgagctccagatttgatggcctcgtcagcatttacttgagttgctcataagtgtctcaaatttaacaagtcccagtcttgatttttttcccccttcaaacctattcctcatgttgtctctatttcagtaaacaatatcaacatccacccagttactcagtccaaaattctaggagtcatccttgattctgctctttctttttttttttttttttgagacggagtctcgctctgtcgcccaggccggactgcggactgcagtggcgcgatctcggctcactgcaagctccgcttcccgggttcacgccattctcctgcctcagcctcccgagtagctgggactacaggcgcccgccaccgcgcccggctaattttttgtatttttagtagagacggggtttcaccttgttagccaggatggtctcgatctcctgacctcatgatccacccgcctcggcctcccaaagtgctgggattacaggcgtgagccaccgcgcccggcctcttttttttttttgatacggagtctcattctcgtcatccaggctggagtgcagtggtgcaatcttggctcactgcaacctccgcctcccgggttcaagcaattcttctgccccaacctcctgagtagctgggcctggctaattttttgtatttttagtagagatggggtttcaccatgttggccaggctggtcctgaactcctgaccttgtgatccgcccacctcagcctcccaaagtgctgggattacaggcgtgagccactgcacccgccctgattctgctctttctctcatcatccctgatctgtcagcaagtcctgttaggccaaccacttctcagcatctgcactgccagtatgctagtccaagccacaaaacacctctcagaggtacgcaacaggactttgttgttgttgtgtgtgtgtgtgttttttttttttttacggtagaattattttataacttgaagtgtagggatgaccttccttttaaaattttatttattttcttaattttttattcccatagattttaggggaacaggtggtatttggtgacatgagtaagttctttaatggtgatttctgagattttggtgcacccatcacccgagcagtgtacactgaacccaatttgtagtcttttatccctcaccccctcccaccctttccctcaagtccccaaagtccattgtatcattctgatgcctttgcatcctcatagcttagctcccacttatgagtgagaacatacggtgtttggttttccattcctgagttacttcacttagaataatagtctctagttccatccaggttgctgtgaatgccattaagtcattcctttttatggctgagtagtattcctttgtatatatatgccacaatttctctattcactttctgattgatgggcatttgggctggttctatatttttgtaattgtgaattgtgctgctataagcatgcgtgtgcaagtatcattatgcaacgggacttcggatgacatattgaacaacttcctcactgatatccttgtgaaacgctacatatttcatgggtctgtttgttataccaacactcaattctgaatgatggaattatttcacatttagtctctttttcatctagccattatagtttagtttaaacaccaagttccattcctgctgcatgctgaaggatttgcagtacatcaggctatagtccatcaattcattccacaattgagtaagtaaggtatctatagtacctcaggccctgtgttaggcagggatggggtaacctagacagatttggtacctgtcctcatggagcttgactttagcggcagagacagatcttagataattgtaccagtacttaagtgttcagaaggacaagtatggaggtgggagccactccagtcctctacagtcacgtgctgcacaacaacgtttcaaccgacaacagagcacacatacagtggtgttcccataagattagaatgccatatttttactgtaccttttctatgtttagatatacaaatacttaccattgtgttccagtgatctacagtattcagtatagtaccatgctgtacagttttatagcccaggagcaataggctatataccgtatagcctaggtgtgtagtatgctacaccatctagatttgtgtaagaacactctctgatgttagcacaaataaatcgcccaatgacacatttctcagaacatatccctgttgttgagcgactcatgactgtacaatgggggaacagctcagcctgccttccccaaggaggcaacgccgatgcagggaaccgagggttgaacagaagtgggcaaggtgcagagaggaaaaaggctttccagatggagaagagcatgtgtgaaggccctcagtctggcaagagcttagtcctgtgtggcaggagctgaacgaggggttaggggagagtggcaaagggtccgggccatcagagaggtcaacaggggctggatcatgcaggattttgaatgttaacatcagagcgatagaaaacatgaagggtaaggtggtttgggttttgaatttttatcaaaatattgcaactactcggcaacaagttagatataacaaaagaggtcatcgtaaaaacagcagtctaccccttccccttcccttccctgactcagacatgacagcttttaactgtttctgattttagttcctttgatggttacctccaaaattaaatcatatgcttatacatctttcttgatttgccaactttagggaactgtgttaactccctgaaatgaaagagaatgacttagcttacgttacctccccatgttgaaattcatattcacatttctctgtaattttttttttgagatggagtctcactctgtcgcccaggctggagtgcagtgatgtgatctcggctcactgaaacctctgcctcccgggttcaagcaattctcgtgcctcagcctcctgagtagctgggactacaggcgcacaccagtgcactgggctaatttttgtatttttagtagaggcggggtttcaccatgttggccaggctggtcttaaactcctgacctcaggtgatctgcctgccttggcctcccaaagtgctgggattacaggtgtgagctaccatgccaagcccacatttctctgtaaattttaaacagtattttagtccatatgtcagttcccctctttttaagataaggatattaataaccctacttttccttccactttccctccttaacttctgcgtcttaaaagctgtacttgaccatacccattcttgcatttgttaacatgtgtgttctgccctgcaaccacagccaagttgtagcttaattctaaagtcgaaaataacattatttacattattacacatgtgagtattgttcttggcgagaccaaataatgaatgtgcccaggattacatttccttctttacagatctggaccactcaaaggagaatgaccaatcaaggtcaaatggattcccttttcttagactctgtcacctgcttaaaatccttgctaggatttaatctacttcatattcaaaccttggcttgcttatatagctctttgttttgcccaccatttctagttgcctttttattttgtttactattcctccttgattatgttgtaaaatgctattagcagtgctgtttatttcgtacgattcggctttttccccactgaagacctttctcttggaaggcctctgcccttctgcaatctgggcaagtatctgctctttgatttaaggttgcatatacagctgtacctggaccttctcctcactgggctcttgggttggagcccgtgtcttaaaacccatatcttcctttcacatggtttactccctcgttttctggactgcatccttaaataatgtgctcagatagagtgcatggggagtaaactgtagtggataccgttgtcacctaccccatatccatttcttctttgcccattcctaacagaatcctgatattattcacctttctaccttattcccaacttcagaaaggatccttaagtcattccacacattgcattcctttggcaactgttactggtcaaggatggacatacgatctaagttggttcactcagactgaagggaaggacttccatggcacgttcagggaagactttctctttttctctcactggagtaagtgagaaaggtgttgctgggggctcttctgtaacctcagactgagggacaaagcctgaggataaagcctgctcaccaaggaaggcggagcagagaaacgggaagaacctgggtcttgatgccgttgcttagctggtgattgcactgtggctggggcctgtcctacctgagctagggactcagataggatggactttcttactgaatgagccagcttcagttttcttttctgttacttgtaaccaaaagcattgtaacagataggtcttctgagtcactgcatgcctgaaatacctttcttctactcttacacttgattggctgagtatagggttccaagttgaaaatcattttttctcctaactttggaggcatctcttctagtatgcagagtaacaaatgcaacaaatgcctgatgccaatcttattatggttcttttgtaggtgcccttcttttctcttccttccctggaagtttttaggatttcgtctccttatttttagtgtcctgaaatctcatgagaatatgtctagagttgtgtcttgttcactcgttgtactgtggtcattcaatctgaatacttttgtcaactcttttttttaaaaaaaaattactaatttacatgctttcattttctctatggggactactgtttaactttggacctcttatattggtcttctgtcttctctcatatttttcatttattgggcggtggggggtgctctgaattttggaagatctcctgcatttattttctttttccttttttctttttttttgaggcagagtcttgctctgtcacccaggctggagtgcagtagcctgatctcggctcactgcaacctctgccttccaggttcaagcaattctgcctctgcctcccacgtagctgggattacagacctgcaccaccacgcccggctaatttttgtatttttaatagagatggggtttcaccatgttgccaggctggtctcgaactcctgacctcaagtgatccgcccgcctcagcctcccaaagtggtgtgagccaccgcacccagcctcctgactttattttctatcccttctgttaaattctttatttcagccaaacctttttttttttttttttaacttactgtgaagcctgtgtgcctactgcctagattagacaattgttaacattttggcgtattttcctggtctgtatagatagggtgcatttttatacctttttgctcaccatttaaaaggaactcacagatgtcacgacatttcacccctaagtacttcagtatacatctcctaaaaataaggacattttccaatataagcacaataccccgatcacatctttaaaagttaacaataattctctaatgttatcaggcacccactttaaattcagatttcctccaaatgtctcttatcgctgttgaggggctccaaagcaattaagatttatacattgcatttgaatatgcttcctttgtctcttatttatttatttattttattttgagacagagtctcgctgtctcccaggctggagtgcagtggtgtgatctcagctcactgcaacctccgccttccaggttcaagcgattctcctgcctcagcctcccaaatagctgggattacaggtacgcaccaccacgcccagctaacttttttgtatttttagtagagacagggtttctactaaaccatgttggccaggctggttttgaactcctgacctcaagtgatctgcccgcctcggcctcccaaagttctaggattataggcgtgagccaccatgcccagcccctttgtctcttttaacaagaacagcctacccacctctccttcacttgtgatactgactttttgaagcagtcagcccaattgtcatctagaagggcccacattttaagatacatatttttagagatggcgtgtcactatgttgcctaggctggccttgaactcctggcctcaagtaatcctcctgcctcagcctcccaggtagctgggactacaggcttgtgccaccacgactagctggcccacattttagatgtctctcttttcttgtgatataatttaacttgtttgtccatatatattacttgtagacaagaagttaggtctacaggcatgttcaggttaaacattttgggcaagaatatttcataggcagtactgtgtacttcatatagcatcagctcaccaggcacttaatggttggttaccctgtggtttgtgatgctacgttttaacacttgattaaagaaggaggtgactgccaaatctccccattgtagacatacagttttcctgtggtaattgatatataatctgtgatgtgatgctttggcaccatacaaatatcctattgcccaacagccatttgcataattattttagcattcattgatccttgcctgaaaccattattacattgggggttgcaaaatgatagtttttttaattgtcacctcttctacatttagtactgtcattcctctgtaatgaattttccctcatcaaataaggaggcattatatttcctcctaaaaagacagtatagatgcttaatctttgcctttattacatttcagagtaaggagttggtagaataatcacctcaaatggtggcaaaatatttgctgttgtgtttccttttctctttcatgtcaatatggactcatagggatttatttattaaatgttttacaattcaaattgggtcaacaagagtcccttcatgttggttcctatattctcctggcataccctcattaattagtctttgagcaatttcttgttttctggcacaagatattccatcccaatatgtgcttttcgtgtcctagaactgattccaaggagctctggttccttatagtggcaacggtatttagaatccaacatgtgggtactaaatgtgctgattcttactggggtaacattatatctaggcactttcagaggacatcgctagaaaatatattcagtttttattttttatttttaatttttttgtagagacaaggtctcactatgttgcccaagctggtttcgaactgagctcaagcgatcctcccacctcagcctcccaaagtgctgggattacatctgtcagggcaaactgctggtaaatattttcacaaaagaaaaataaaaaaaccaaagtgctgggattacagatgtgagccactgtgccctccattttttttttaagtcataaatacataatgatgtcttctatggcaatttaacattacagggttcttccttaacttttttttttttttttcttttttttgaggcagggtcttgctctattgcccaggctggagtggtgcagtggtacaatcctaattcactgcagcttcaaatgcctaggcttcaaacaatcctcctccctcagcctcccgagtagctaagactacaggtgcatatcaccatgcccagctaatttttaaaaattttttgtagagatggggggtctcgttgcgttgcccaggctggtctcgaactcctggcctcaagtgatcctcccatctcgatttcccaaagtgctgggattacaggtgtgagccaccatgcctggccaacttttatttgatctgtatatatcttttccttacactgaaaatgttgggtcttactaatgttaacatagttacttatttgctttatcttgtaatagacataaaattacaaaattataataccaatattacgataaatagctgggcatggcggcgctcgcctgtagtcccagctactcaggaagctgaggtggagggactgcttgaacctaagagtttgaagctgcagtgagctgtggttgtgccactgtactcctacccggacaacagagtgagtggggggaaaaaaaagaaataatggaagatccagagaaagccccaaatatttaaaaattaaacaatacactttgcagcttcctcacctctctcagccttcatagaattgaagagagttagggccttgcactagattaggctttgccttaaggaaatgttgtgtttgatttgatcttttatccagaccattaaaacttccttaacgtttattagtaataaggctatttcactttcatatcatttgtgtgttcactggagtagcacttttagtttccttcaagaactttgattcacaacttggctaactttggtacaagaggcctagcttttggcttctcggctttcaacatgcctctcactaagcctgatcatttggtttttggtttaaagagaaagacatatgactcttccttttacttgaatgcttagaggccattgtagggttattaattggcctaatttcagtactgtcttgtccaagggaatagggaggcccaaggagagagagagagatgggggaacagctgattggtggagtagtcagaatatacacatttatcacttaagttttgccatcttttctttttctttttcttttttttttttgagacagtcttgctctgtcacccaggctggcatgcagtggcatgatctcagttcactgcaacctctgcctcctgggctcaagcaattctcctgcctcaacctcccgagtagctggtattacaagcgtgcgccaccatacccagctaatttttatattttttagtagagacagggtttgccatgttggccaggctggtctcgaattcctgacctcaagtgatccacccgccttggcctcccaaagtgcggggattacaggcgtaagccactgccgcctggccaagtttgccaccttttttattttttttattttttgagatggagtctcactccatcacccaggctggagtgcagtgatgcaatctcggctcactgcagtctctgcctcctggattcaagcgattctcctgcctcagcctcccgagtagctgggactacaggcatgtgccagcacgcccagcttgttttttgtatttttagtagagacggggtttcaccatgttggccaggctggtctccaactcctgacctcaggtgatctgcccggctcagcctcccaaagtgctgggattacaggcgtgagccaccccgcccggccaagtttgccatcttttatgggtgcagtttgtggtgccgcaaaatgatgatagtagtaacatcagagagcattgatcacagatcaccataacaaatataataatgagaaatttgaaacattgtgaaaattaccaaaatgtgacagagacatgaagtaagcacatgctattggaaaaatggcactggtaaacttgcttgatgcagggttgccacacaccttcaatttgttaaaaactcagtatctgcgaagtacagtaaagcaaagcacaatcaaatgaggtgcgcctgcatattacaaccaagaggcttttcgcagaaacacgagtgtgcttcaacattcaaaaatcagttggtgtaattcaccacattaagataataaaggaggccgggtgcggtggctcacacctgtaatcccagcactttcagaagccgaggtggacagatcacttgaggccaggagtttgagagcagcctggccaacatagtgaaatcctgtctctactaaaaatagaaaaattagccgggcagggtggcacgcacctttagtcccagctattcgggaggctgaggcaggtgaatccttgaaaccaagaggcggaggttgcagtaagctgagatcacgccaatgcattctagcctgggcaacagtgagacccagtatccaaaaaaaaaaaaaaaaaaaaaaaagataataaaggagaaaaaccatatagtctattcaataaatacagaaaacgcatctgacaaaattcagtgccctttcatgataaaaattcagcagattagaaatagaggaagtgcatgtatgaaagagctacagatagattgtacttaattgtgaaatattgaacatgttaccccgaaaatcaggaaaaaggcaaagatgtccactctaaccacttctattcaacattatactagaggtcatagccagtataatgaggcaagaaaaaacataagaggcattaatatttaaaggaagtaaaactgtttctatttgtaggtaatgtcgaaaatgtgaaagaaactatcagaacctgctagaactaaaaagtgaattcagcaaggtctcagggtacgagatcattcaaaaactaatcagaaatgaaatttcaaatgcaatatcgttaggaataatttaataagaaatgtacaagatttacacgctgaaactgaaaatgttgctgaaagaaattaaagacctaaataaatggaatgttgtaccatgttcatcagctgaaagactaagtgtctttacagtgtcagttctcccttcattgaactgtagattcataaccccagtcataactgcagggttttttttgtagaaattgattgtaaaatgtatatggaagctgggcacggtggcttatgcctgtaaaccagcactttgggaggctgaggcagacagatgacttgaggtcaggaatttgagaccagcctggctaacatgacgaaaccccgtctctacaaaaaatacaaaaattagccagacatggtggcacacacctgtaatcccagctacttgggaggctgaggcatgagaatcacttgaacccggaggtggaggttgcagtgagccaagatcatgccactgcacgcccgcctgggcaacagagtgagactttgcctcaaataaataaataaataaaacgtatatggaaatgcaaaggacctagaacatccaaagtaaacttgaaagagaacaaaattaaggggcttatgtgatgtgactttatagtcatttgatttttaacagaggcaccagaacagtccggtgcgggaaaggaaagtcttttagcacgtgccggatgatggcaaatgacatccataccagacaaaaatgaaccttgaccttaccctaaatattagtttcttagagttgccacaaactaggtggcttaaaaccacagaaatttggctgggtgcggtggctgacgcctgtaatcccggcctttgggaggccgagtcgggcagatcacctgaggtcaggagtgcaagactagcctggccaacgtggtgaaactttgtctctactaaaaatacaaaaaacttagtcaggtgtagtggtgcacacatataatcccagctagccaggaggctgaggcaggagaattgcatgaacctgggaggttgcactgagccaagattgcaccactgcactccagcctgggtgacagagtgagactccgtctcaaaacaaaaccacagaaatttgctgtctcataattccagagtctagaagtccaaaatcaactgtcatcagggccatggtctctgtgaaacctgtaggggagtccttccttgcctcttcctagcttccagtggttggcaacctttggcattctttgatttgcagctgcattacttcaatatctgtcttcctcatcacacagcattctccatgtatgtctctgtctttacatggcctccttcttgtaagaacaacagtaatattggattggggcctgccctactccagtgtgacctcaccttaactaattacacctgcaacaacgctgtttccaactaaggtctcagtgtgaggtactgagggttaggacttcaacatatcttttttgggggacatagtccaacccatgacactacttcacaccatacataaaaattaattcatgagagattatagacctaaatgttttaaaagctaaaaatataaagcttctgcaagaaaacataggagaatatctgtgcagtccaaagaataaggttttttttaaacacaatttcactctgttgcccaggctggagtgcagtggtgcgatctcagctcactgcaacctctgcctcccgagttcaagcgattcccatgcctcagccttccaagtagctgggattacaggtgtgcgccaccatgcctggctaatttttgtatttttagtagaggcagggttttgccatgttggccaggctggtctcaaactcctgacctcaagtgatctgcctgcctcggcctcccaaagtgctgggattacaggtatgagccaccgtgccaggccaaaaaaagatttattaggatacatgaagcaatagctattaaaagaaaaaataaattggacttcattaaaatttaaaacttttggtcctcaaaagataccattaagaaaatgaaaagacagagctgggcgtggtgaggcttgcctgtagtcactactgggtacttgagaggctgaggcaggaggatcacttgagcccaggagttctaggccaacataggcaatatagtgagacagtgtctcttaaaaaaaaaaagaaaaagaaaaaacaaaagaaaataggctgagagctgtggctcatgcttgtaatcccagcactttgggagtacaaggcagatggattgcttgagctcaggagttcaagaccagcctgggcaacagtgaaatcccatctctacaaaagatacaaaaaattagccaaccatggtggcgtgcacccgtagtccatagtcccagctactcgggaagcagaggcaggaggattgcttgatcccaaggaggtcaaggctgcagtgagctgaggtcgcgccaccgcaccccagcctgggtgactgagtgagaccctgtctcaaagaaaatgaaaagacaagtccaccaagaaaacagttgagaccagtcatagaaaaaatagaaagtcatatctgacaaaggatttgtattcagaagaattcctataactcggtaataaaaagacaacctgatttttaaagggtgaaaatattttaatggatacttttttttttttttttgagacagagtctcactgtgtcacctaggctggagtgcagtggtgccatcatacatagctcactgcagactcgaactcctgggctcaagtggtcttcctgcctcagcctcctgcgtagctaggactacaagcacgtgccactatgcctggctaatttttaaattttttgtagacatgggctggtgtgtgtctgtgttgtctaggctggtcttgaactcctgggctcaagtgatcctcccacctctgccccccaaagtgctgggccaccacgcctggtgtggtgtcaccagagatgagccaccatgccctgcctgatacttttcttttatcatctgtttatttcttgtttatgggtgtttctgttctgattttatgactattctgtattctaagatttctctgagaatattatttgtttcctctaaggacagacttggtctctcttccatggggctggttcttgagccgccagggatggggggaggacctgggtagctgctgcgctgccccttctctgctgtggtggagtggcccgttgcctgcggggtctgtctctgaagggtggtttggagaagttctgtggaggcgaggcaggggtcagctcttgccccatggaccctcagagactgggaaaaggtaggcatcacctgggctgctgccagccacatcaagagcctttggggtgggtggggtgggggccggggaagggaaggttctagctgttgatttagaaaagacccattgatttcttgcctgagggaagaagtggcaccttgccactccaagtttgctctgctcaccagccccaacagcatcagcctcacctgggagcttattgaaggtgccctgccccaaagcttgtgggtcgggatctggcagtcagcagcccccaggtgttgcacacatgacagcactgcttgcccctcctctcgtctggtctggtctggtctggtctggtctggtctgagagcttctttggggctctgacaggtatacaggctctcatctgctctacagctctcttgtagtacattcctctctgttccattagtcaacatgttcttgcctacttccagcatctagaaatttgctgagtgtatcttatccgttcagaggtcctctcctgctattgcctctgttagaaatttcttccctttcatatgtctgtacttcggtttctttgaggtttgaagggtcaagtggcaattacatgtaggcagttggccatcctctggtgaaggctttaaagcccaggaataacaagatccattatgtctaaaactagcaaaaaccctacctgtcacatggtgaactgaattagaggtgatggggacagaagccagattggagtgagtggaaggtgagggagtggagattgggtatagacaactctctttaagaagttttgttgtgatggtgaccagaaaaataggagtggggtagagggggatgagggtgtttttcacgtgggtgaatatgagagcatgtttacatccttctgggaatggcccaggagagaggggagcgtgagaaggaggaaatggggacctggaggagcagactccttgtgtggaggggggaagcggcatctagagctgttgcaggaggtgggctttgagtaaatgcttcctctttggtaaagacggggaacgggaacggtagaagttgcacggaccctttgttaaagctcagaagctgagcgagaattagagcttaagtttatggagtagtcagaataaagtacccctaactgtattcttgcacagtgcaggaagccaggggtctgaaatcaagatgttgcagggctccattccccccagagcctctagcatggatccttccttgcctcttccagcttttggtggctgcctggcagtcctagactttccttggcttgcagttgcattgctccattctctgcttgtgtcttcacatggccttctctgtgtccccgtattcttctctggatgcttgtcactgtattaggcccaccctaaatccaggatgatctcatatcaagatccttcacttaattacagaagcaaagaccttccaaataaggtcagagccacagggtctgggggttaagacatacacctaactattcggggctaccatcgaacccctgtagaagcctgtccatttccaggatagcagagcccaaggaagggccagaagtccccccaaaacagttgtttgcattcaccagattctaagctataagcagatgggcagtggcagtcggtcctaatccatataccattggcaacaatagtttagttcactgtagacataatgagatgcttatcttctgctaagtagtcctcatggtaacagccatattactcctggctttgagtgacagcgctgtgctcttgtctggtgcccatatacttcagcagctggaaacaagacagtgctcatgattcaccggaaagtttctgtagttaaaatcaagtgatcccttgagtctattctaatatttgtctgtaccatgttctgtgacgagacatggaaacaaaacattaagaagtgaaagtatctttgattatgctcttgaagacaactttttgtttgtttgttttgtttgagacggagtttcactcttgttgcccaggctggagtgcaatggtgtgatctcggctcactgcaacctccgcattcccgggttcaagcgattctcctgcctcagcctcccaagtagccaggattacaggcatgcaccaccacgcctggctaattttttttattttagtagagacggggtttcaccatgctagtcagactggtctcaaactcctgacctcaggtgatccgcctgcctctgcctcccaaagtgccgggattacaggtgtgagccaccgtgcctggccgaagacaactttttaaagatgcatatgctctgggctgggtgtggtggctcacacctgtaatcccagcactttgggaggccaaggcgggcagatcacctgaggtcaggggttcaagaccagcctggccaacatggtgaaacaccgtctctactaaaagtataaaaattagccgggtgtggtggcgggtgcctgtaatcacagctactcaggaggctgaggcaggagaatcgcttgaaccccagaggcggaggttgcagtgaattgagactgtgccactgcactccagcctgggcgacagagtgagacttggtctcaataaataaaataaaataaagatgcatatatgctctgaaggctggctacattttattttttctcaaacaacttttacagtggatagtgctgtaaaagttgtttagctctggtcattttatcttttttgtgatctgcaaaaggagatccttttccttttcactgcctctaatacccaactccaatactcctttgacctcacaggcacttagaatccatcagtggctccatcttttctcagacttcacctccttcgtatccttattcctctcctttgtagcttcagtgccagtcagacgtcgttactccctggcacactacctcagcccttcggcactttcttgctttgttatattcagtcgacaaagccccagcctcatgaaattcagtcatgtctgccccatgcctgctccgtcctgaagctgaatgtgactccttcattgattccccctttaagttcatgtctaccccaggtaaacttcttgccgccaagcccacctgcatactgcagttccccggtctctcctagcccctcccaccctcctcatcagctgtcacacctccttgcagctgatatcttagttcccagagagcacagaagcaagctcaagagagtgtctacaggccagcgtctactccttcgctctgcctccctcatgctgtcacggagcgcctgtcccaggccctcactcctgttctaaggcatctctccagtcctctactgcactctcccccatcagagattcctccctcgcctgccctagaaacttgttgctacttctcccaccttgacaaaagctgctcccaaccccccacctgtctagcatctctgttttcctttaccagcaagactccagtccctgtctccacaccctcttcaaccttctccagttgttcctttgctgccacagctctgccaagctgctccatgaggtctccagtgatgaccttcatgttgttaaatctgggagctgcttgtcacttcttttcccagagctgtcgtcgtcagttaaccccaatacccatacgagacaatcctttccctcccttgagtctctgcactgatgtgcaccttctcagtgcaaaccacagcttttgtctctttctagctgaatacatgactgactgtgcttatcttagctgtcacccctgctggagcagaagctccacaggacaggattgtctccttgattcacagatgtagctcaagctcctagaacagtgcctggtgtctgtgggtcctcaggaagtcctaggtgagtgtgtgaatgtctgtcctcctcggtcttttctgtttcgcatgtgatgttggaaggcctcaggttcaggcttttcttctccaccctcactcccgaagtgattccgtccagcctcatggctcccaaatttatgtctccaggctgactgggtcacgggaactccttatcctccctagaccttctctttccctggtcttctcctttccagtaaacagcaactccaactcctgctcctcaggccagaaacctggcgctggttacctcatttgttcacaaatactgttactccacctgcaagatggatacaaaatctcatgagttcccctgcctccatggcccccaccctggtccaggtgtccagcttccctgcctctgcccttgccccctggttctttgtttagtcctgcaatattgtgctcttctgttcagaaccctccagtgggtccctgcttgctcagagtcacagcccaacaggatcacctctcttgccactctcccaccactcatgcactgcggcctcactggcctcctggctcctccctggaccctccaagtatgcccctgcctcaaggccttgacctctcctctgccctctgtcccaggtatcacacatgtctgctcaagtgtcaccttcccaatgtggccttccccgagcacacccatgtctgtaagtcaggcagcctgcctctgccccaccagttccccctgcctagcataggacttgtcaccatctgccacaagctgtgttactgcttggttttgtttgtgctctcccactcccttcccctccctccctctccccacccctatagaatctgagtcccatgaggacagagatttttttttttgcctcttcctcaatatatccccagtgcctagaatcatgcatattttaatttattgagtgaattaacaaataaattctgcagtgggacattgctctaaggttttgtcttataagagggacagaagaacatgcagcctgctctgctgttggctccttagcttctccatggctaacaggaacaatattgtttatgagataatcaaagccatagtcatgagttagaaggtacatataaaggcaaatatgtggagattgagttactttggcgggggcggaggggtgtgtagttatctgaaaacatggaacaaatcaatgagagtctaaatagcacccacatatttgcccctcttttaaaacatacctcctttatgagtgtagaatttaacagcacagtttcccagtgcagctttgcgaaacaagagaaatgaattttaaaggctgtcaggtgcctttgcaatctgtggcttagtatttgtgtaacaacatttgtgttttgccaacagatgtactgcttaaagtacccatgagaatggcctctgtggttttctactttctcggatggaaccttaggaactgattattgagaagaggctgatactgcccacctcagctcccaggcaggcttcagggccttggttactactcctttgggccctcactgacccttgcagacgtcttttgcaacctctgtagccagaagagacaactgctttctggcatgttgctctttccctaatggctttatgagcttcttgaacaccaaagcatgtgtgacttcctcacgccttcccctgtatagtatagcacccctaactgtatgtgtaaggagaaggagtgagcaattgatggcgtccccctggatctccaagggaatgggaaggggcagggtttctggattcagtcatgtggaatctggtcgttggtgtctaaatgtgcctgttacttgtgcccaatgtccaggttcaccaggaggcttagcctgctcatttccctgctagtagctatattttgggagagcattttttatgctctaattgaactttgtgggtctcagcaatttgaacaatgttttgtttttcttctggtcaggttacaaaggaaagaaaaggaatctggtgttgtaggaggtggtgtgttgtgtaattacttgttttttttttttaagtttttttatatttttgcaacaaggcaagttttctttgaataaataatgctgggagcttatcacatagaaggcatatgtgttgtactcagtacattctgaattatctgggtttatttttatctcttgaattcacttataaacaattcaaaggctgcttttttagctaacagaaataggaagagaatctcagaatctgttttgtcattttttcaatgggttgagttatagtgattatgctaactcggtggaaaagcagtgtagtgagtaaaccccacatacggcatatcatgaacattttgttgcttttttggcttctgaccatcttcatacctttttttgtgttaaaagtctccccattgtgtatatcttagtaagaggcaggtggaccctagtttctacctaagaaaacctgaagatggggttgggggcctgtggtgtacttccttctcatgctgtccatgaccactgcagtggctttgtaaggatccaggacccagggcccctcagtgggtgtcttccatttctcaagattgcctcttggttgtgagatgacggttgctgctctagtcattgcatccactcctccaggtaggaagaaagaggtcataggggaaaggcaaaatggcacttgacatcttaacttctaggcccattcaatatttccatttccatcttcacacccatcatcttgtcctagggaacaaacagcaccagcagctcagtagctataacagcaattattatttctcacacatgggtctgggtcagctgcaagatgggattcagatctgttctcaagcctgtcgttccaggacccaggagggagaagcagctgccaggggaagtctcttcgtaggcggaggtcaggagtccaagaggagtgagcagagtcacagaagcctcttaaagcctcttcttcccccatcccatcaacacgtgagcaagcccagagtcagtgggtgggaggtgtgctccgcccatagtcagtagaacaagagcaagcttgaaagagaacgatgaacaggagtgcactcggccactgtctccttagccataacgtagtcccatggtctgctgggaagcggggaataactctccttagctgagcgcagggtctcattagtaaggcagatggagaacatggatgttgggggacaactggcagtgcctgccacaggggaatggatatattccctccccttgctctctggaaactaggggatggcgatgaagcctaggtttggccaaacccattctgccttcagggactttgactcttgagggacagtgagggattagtcatggtggtggcagttgagtcacaaaaccagcagtggtggctaatgtccagtgatgacatgcaacagtgcccagggtgggtgtcccaaccagcaggtccctgcagtataaccttggctgtgtttgcagtggtgcagcctctattcctgctgcttttctgagcctagttctctagttctctctccatttccagatctgctgcccaagaactcctttgtgattgaatttaaccagagttgatttctgttgcttgaaactcaggaccttgatgcagtgtgcagggtctgggcaaggtaaaaacacactttcatgatttcgcctcaagtatagtagatgagcttaggctttttgagccaggtagccttgggattaattctcagctcttgcacctagcaggtgacctcagcaatcaagtcacttgccctccttgagcctcagtgttgccctcagttaaacattgctctcgtgtgttgctgagcattcagtgagattgtatataaagtgatcattgtgaaggtattgggacataatttgggaaagcgtcctggtctaagcttttgattggctctccatcatttgggtaatgggatagtgatttaggagtatcatagcagctcaaggggcccttctggaaagggtatgaggaaggtcagggacaagtctgaaatgaatcatcctaggcttaatgcctgtgactgggcagtgggtacaattatctcaggctagtcagtagtcatttattgtgagaatacatgggcagattttttaatttccttctcagtctagacttgaatgcaaacagttcttattgctaacttaccactagtcaccactaatgaacaaagactatgaacaggaaattcataaaagaagagatacagatggccaatgaagataggaaaagagttctgcctgctggtaatcaaagagatgcaaacgagaacaaaaatgatgccttttcacctaccaaatttgtcaagattaaaaagaaagcaaagagccagcgtcagctgatgttcatacctgcacctgctcggtagcttgctaatgttctgcctgctccacacgccaggccagcctccacggcgcagccaggtgaggcctttccttgtatacaggcacgtttggattcactgttgcataagtgagacatgtgcatgcttcacaattcaggaagtgcaaactccagagtgatgcaaggtctgagtgtccctgctgccctggtctcccagctgcctaggcctctcttcagggaacggctgcatccagggtcttgtctgtgtcttttgaggtgttctatgtacacgcagacacatctaaacctatttttattttccctgcacctgcttgggctactgtaagctgttaaatttttttttctaggaatttgtccattttgtctgactagcataaagttgttcatgttatagtttatacatttgcaacatctgtaattatgtctgctttttcattcctagtgtttgttgtttacttgtaccttctcccgtttttccttgtcttggtaaaagctcattaggttcattggtcttacaagaagcagacatgtaggcattattgccctgtattactctgtgtctcttttctagttcattaaattctgcttttgcttttatctttattattttttctatggtcttagagtacattctctgtgttttgttgttgttgttgttgttgtttgttttttgttttgagagagagagtcttgctctgtcgcccaggctggagtgcagtagtgcaatctcagctcactgcaacctccacctcctgggttcaagtgattctcgtgcctcaacctcccgagtagctgagatttacaggcatttgccccacacccggcaaattttttgtatttttagtagagatggggttttggcatgttgaccaggcgggtctcgaactgctgacgccaggtgctccacccgccttggcctcccaaagtgctgggattacaggcatgagccaccacgcctggccctaacttcttaagttataaatttggttcattgatttttctacccttttttcaaatgtaaacatttaaggctaaccctctggaactacttcaactgtatctagcaagttctgatagtattgtcactttaagttagcccaaagatattttaaattttctttgtttcttcctttgactcacatattattttaaaatgtgtttttcaatttccaagcacatggctttgggtttgttttttttttttcctagttgctctagaaaaaaaaattgactgcatgaggtggctcatgcctgtaatcccagcactttgggaggccgaggcgggcagatcacctgaggtcaggagttcgagaccagcctggccaacatgccaaaacctcgtctctactaaaaatacaaaattagccgggcatggtggcacacacctgtagttccagctactcgggaggctgaggcaggagaatcacttgaaccgggaggcagtggtcacagtgagccaagattgtgccagtgtactccagcctgggcaacaagagcaatactccgtctcaaaaaaaaaaaagaaaaaaagaaaaaatcaacttctaactaaatggcactgtgatcaaagaacttggtctgtgtgacaccagttcttgcagttggttgagaagtgctccatgacacattatccacaaccagtggacagaatatgtcaccaccaagcatgggtgcaggattctacatatattcattacctctgtcttatccgtttgttgtgaaagtattttctcttcttactgtcattttgtttacttgatttatcaactgatggaatacgtgttaaaacctactgtggtgatggacacatcagtttctccacagagtttggtcattttcattttattatttattttgaggccacattttcagttttagatacagtttcacattcctggtgtattgaaccctttggtattatgaagcgaccatactaatatgttatttttttttaaattattatttattttatttatttttctttcttttttttttttttgagacagggtctccctctgtcacccagtctggagtgcagtggtgcaatctcagctcactgcaacctccgcctcctgggctcaagtggtcctcccacctcagcctcctgagtagctgggattacaggcttgcaccagcgcgcctggctaagtttttgtatttttagtagagacagggttttgccatgttgcccagactggtctcaaactcctgggctcaagcagttcaccagccttggcctctaaaagtgttgggattacaggtgtgagccaccacgcccggccatcccagttttttattttcctcctttctgtgtctttatgcatcagtgaggtggagcttttgaaaatgtcagatagctagattttttttttttgagacggagttttgctcttgttgcccaggctggagtgcaatggcgtgatctcggctcactgcaacctccacctcccaggttcaaaacaattctcctgccgcagcctcctgagtagctgggactacaggcacgtgccaccacacccggctaattttgtatttttagtagagatgtggtttcaccatgttggccaggctggtctcaaactcctcacctcagctgatcacccgcctcagcctcccaaagtgttggaattacagacgtgagccaccatgcccagctgatagctagattttttttttttttttttttttgagacggagtcttgctctgtcgcccaggctggagtgcggtggcgcgatctcggctcactgcaagctccgccccccgggttcatgccattctcctgcttcagcctccagagtagctgggactacaggtgcccgccaccacgcgtggctgattttttttttttttttttttttgtatttttagtagagacggggtttcaccgtgtcagccaggatggtctcgatctcctgacctcgtgatccgcccgcctcagcctcccaaagtgctgggattacaggcgtgagccaccgcacccggcctcgagattttttaaaaaatccattgtctgtttcgtcctttaacatctatttgatttctgatgtatttagattcatttatagcatatttgtgcattctatttttccatattttctgttcttttaaattttccttctcctttcttgccttctcttagacttttaaaaaaattgtagtaaaatacacatcacctaaaatttaccatttttaaatgtacagttcagtggcattaaatacaaattggaggccaggcatggtggctcatgcctggaatcccagcactttgagaggctgaggtgggaggattgcttgaacctggaggtcgaggttgcagtgaggtgtgatcacactactgctatagcccaggcaacagagtgagaacctatctaaaaaaacaaacaaacaaacaaacaaacagattggcatcacacagtgtgtgtgctgctgtgctgtgctgttatcatttaacattaaaacataaacatcagcactgttatggactgaatgtttgtgtcccccaaaattccagtgttgaagctcaaacctccaatgtgatgttatttggagatggggtatttgagaggtggttaggtttagatgaaatcaggagggagggtgggtttcgcatgatgagattagtgtccttataacaagagacagcagagagcttgctttctccaccatgtgagtatgcaatgagaaggcagccatctccaagtcagaaagagagccctcaccaggggctgaatgtgctgacaccttgatcttggacttctagcctccagaactgtgagaaatttcagttgaataggccccccagtctgtactattttgttatagcttgagcagactaatacacccatgttatgaaaagctataaacatccctttaaaggccacctaacgcgtcgtattacctcatgcatcttctctgctgagctttccaaaagagtggcttaggctgggcctggtggctcatgcctgtaatcccagcactttgggaggccaaggcaggtggatcacctgaggtcaggagttcaagaccagcctgaccaacatggagaaatcccgtccctactaaaaatacaaaattagctgggcgtggtggcgcatgcctgtaatcccagctacttgggaggctgagccaggagaatcacttgaacctgggagatggagggtgcagtgagccgagatcgtgccattgcattccagcccggccaacaagagcgaaactccatctcaaaaaaaaagagtggctggccgggcgcagtggctcacgcctgtaatccccgcactgtgggaggccgaggtgggtggatcacgaggtcaggagttcaaaaccagcctggccgagatggtgaaaccccgtctctactaaaaatagaaaaactagccaggcgcagtggcaggcgcctgtaatcccagctacttgggtggctgaggcaggagaatcgcttgaacctggggggcggaggttgcagtgagccaagatggtgccactgcactccagcctgggtgacacagtgagaccccgtctcaaaaaaaaaaaaaaaaaaaaaaaaagtggcgtatgttcccggtctccacctctcattcgccagcccctgtgaccaaacccctgggattagatctccatcgggtccctcccctcaccctaacctcacatgcagtggttcctgagaagctgctgtttatctgatcacgggatccagcaggatctgagggctcattcactgaatctgtactacccaacaaggcaggcttgtccttacccacacttttcaggtgaaaacttaatcagattcaagcgtttatcttagtggcctcttcgtggtgtgtgatttccttcttgcagctctttactggctaaaactcttcactgggagttaaaccaggtgtggtccttgaccctcatcattttgtcccatctcctatgctgggctctgtatccttgtctccaagcagtctcgtgtgacagggaagttacctattattgtatggtcccctcttcttgtcacctctggtgtggcacttgttccatttcttgttcaatgaatgtgatttgtgaatgtgccacatctgtgggaggaaggcagttcgcagcaagagttgtagttcccttgctttgccctgagggccaggactttacactagatttttttgttgcattcctgcactcataaagtacacgtaaacttagaggtggtgtgttaaatgctagaacttaaaactgagttcagctaggctcaagtgccccacaatttttgtcccaccagacaatttcatgaatatctacagattgttccctcaatatgcctcaatattgaggcatattgatttggggagcacagacaagtcaaggttgatgtgcatccgctgaacatgatcttaagttgttgaagtaggtattattaatgaacgaacgtctattttagctccaagagcccctggtcttccagaagagactcccaatgatcttccagaagcagctgggcttcttttggtcctcccccacccaggtgcagtcccgttctccctgcctgggtgagtttgattcctctgccgtggaataggctaggctgctacctcttgagcctcttccaccaggccatccattaggtggcgacagagagcactaaaaggaactactatggaaataaaacttgttttgcttcttggggggaaaaaaaaagaaaaaggcttgtggggcgtgtgtgcattttagtcagattttactgtgcaaaacatttgagagatttctgccctctttctcccttccattcttctcaacccactgggcgccctaccacccctgtctccttcaagataaggtagatcagaagaccaaatagacaaatgccatgtccactgttttctgtcacagttgatagccataccagtcacccaagctggaaacccaacaggcccctgcccttcactgcccacatccaagggagccaccaagtcccacaaattgttcctttaactgtttgtccctcttttgtcttctgtcatcccttctaccgctgtcctggttcaatccctcatcttgctctgggactcccatgataacttatgatctttcctccacctctctatcttccacacaatccctatcatcaatctcattcccctgctttaaacccaagagtggcaccctgtgtttgagtgacatcagggcccctcatgtggctcctgcttctctttgtggccccttctgttgctgctgcttttcttatggacatagccctcagcagtccaggactgcttgtagttcctcccaggtaccatgtttcttgcactcctggcctttgtcattggctcccctgcccaagtccccttctcttctcctttccttcccctgtggccttgccttgtcgtgcttatccttgaagaccctgtcaggtatctcttccccaaagagccctgcctaaccaccgcccccctcccccccgcgacacacacacctgggttaggccctgcctctccacgcctgtgcctcctgccaagtcctcagaggtctctgatcccatgtgcctccaggcatggcatagggggactgtgacacagcctctcggcccacagacccctgattgtgggcttgctcactgccccagtcagtcctcttattgaggattccgtgccagttcctgactccagcacacacacgcatgtaggccgccctcctagtgcctggctccttccctgtctcttctgccactcattcccatggtcgtatcctggagttggtcatctctggaactccacccacggagttctaacttagctctgcctatgatgaggacttactgtcttcccagcttgcagtgtcaaccactgtttgatgcccctgggactccattggtcttccctcctcttgtgaactgtgcccatcaccagacgaacttgttttagaatttaccatcgtaactgagctcccttcagcgcatacctccttggctcctgctcagtctctgtttctccttttagccaaactctctaagagttctctccactcatgggccctcttccttgcctgctgctccttgctcagcttgctccatgaacacttgcttttccacattccatgaaataatcttaacagtcatcagtggctgtcactccttctcagccctttccttgtgtctcttctggtacctcatactctccaggtggccatctcacctcacatcttgaaccctctgggtttgggagaattctcacctcacgagttgatgggaggcctggcgacctctgattgtagtcactgcaaatgccagatgcttatttgcctagcttccctttcggtcagggcagcagttggcaaacggtatctcaagggccaagtccggcccactgcctgttttcgtaaatgaagctttaccaggacccagttccaccccgtcctttgtgcattgtccaagactgctctcctgtacaacagcaggtgggctggttgtgacagatactgtctggcccacaaggtggaaaatactatctggccccttacagaaagaaattacctgagttctacacgagggtgtaggtatgtaccctggcctctgccagtcagactcacatgctaggaggagcagggccaggcaggagagccgtgtctcctggcattggggctgcaggaaagacgagctcctaggccacagtgccagtggccagtgctgctgccttgcagggtcgcacaggcagtgctggctgtttggactggcttggcagaaggatttgaagtattgttcctagccaactggactcaaacctgttcctccaaccctctagggattctcttatcacccagtagccttttccccctagttttaaaaattgcagtaaaatacacaaaagataaaatgtactgccttaaccatttttaagtgtacaattctgtggtattgagcacatttatattgtgcaaccatcaccacatgcatcttcaatagcttttcatcagtccttgtctgcataaatcagctagagttggtttctattgattgccaccaataatcttgacagatatgtctgatcttccttctctgcactgactcctctttctctgtctcctctgctgattctttctcctcatcacaactccaaatagcagggggagggttgtttacacttatattcagcacgccctcacgcactcgcctggctcttcagacctctcccctgaactccagattcatacatccagctgccctttaggcctctagaaagctaaatacctcagtatcaaaaacatgagaaacggaagccagagtcctggatctctcgccctttcgctgtcccggtgcccatgcccttcagggatggcacctagaccagctccctgcatccctgcctagactctgcagtagtctcacgtggcagacccggaggtcactctcctctctggatgccctgcggacactccggttagcctcagctgcaagagcctcctcacccaaggtcacgccatttccaggacagcaccctggtgactgagcgaggtaagggtacaaggcccttatagggccttctctttgacttcttcccacctccctttatggatgtcagttcctgatgaacatcttacacctcaaaccgtgacccaacatctgcttctgcagagcccccctgtggcatcttgtgccctcctgccccactccctctactctatatcttcccatagttagaatgggctttttttttttttttttgagataaggtctccctttgtcacccaggctggaatgcaatggcacagtcacgactcactgcagcctcaacctcctgggctcaagcagtcctcccacctcagcctcccaagtagctgagactacaggtatgcaccaccacacctggctaatttttatattttttgtagagactggggtctccctatgttgcccgggctggtctcgaactcccaggctcaagcaatcctcccgccttggcctcccaaaatgcaggattacaggcgtgtaccagtgtgcccagcctcagatgggctctttgaaaaatgtttattagatcaggttactcccttgagaaaaaccctctcagaataaaacccgaagtccattacttgaaagcagagccagcttcatgggcctttgtaactgcccatgggcttgctggaacccaggcttggtttaatactctactctcaccatctcaaaattcttaatttttgaacaagaggccctgcattttcattttgcaccaggctccacaaattgtgtaactgggcctgcctcagcagccacatggaacatgatccctccttgcctatttgagctcattctctaccattctctcccttgctcacctggctcccactgctcttgctcttcctggaacttgccataatgttgctagagtcagagccttggctcttgctgctcctcattggctggacccctctttacttgacctgctccctcaccactcacttccttcagatctgtgttcagatttcgtcttctcagagaggcttttggcccctgtccatctctctgaatttacctctgacctctcccccaccaccactgcgctaagctgcctcagaactttgtagacattctgtctggtcttctgatgtttcccccttggaagaatcccaaggtgcctgaagaatgctttctttatccttgaagttgagtaggttgactagagtctggcttgctattgagcattctttatcaaattgtcctgggaacatggtgtattctttcagtctgcagatgtagtcgttgctgtttcaggtcagctctcttatggatctttgacagcatcttctgttccatttgttgagttctgtacttcagggacacaaattcctcatgttggattgtctttgtctctcttccaatgctattagctttgccgtaattggtttagcttttgtctttttcatctgcattcactttgtctaatttgattttcagctatgtatattctgtttctggctgtttttcaatgtatttattagtttcataatgatgtgttttggtctgcagtttgtttctctaggttggaaatttgtcttttcatcttattctgttttatcatcccatctttgaactcttttattgggaacatgttcttatgaagttgtggggaatttttttcccttccttgtgtattctcttcttggtgggagactttgcctttctcgtgccatctccctccctgggcctcttttttttcttctggccataatatgtttgcctagttaccatgtcacttcttttcgtcttggctcaggcttggatggctctgcatagtcgttctgtttgctttgagacagtggaggaattcttggctctctcttcccagtttcttggcatcttctcttgctgttttcccctctgagctatcgcgtgcaggcttgttatcttgtatccggagagaatttgcacgctggagggagctgcagccatgtagtcttcagccctatctggattcttctctttgttctaagaactgtgttggatgtcttactaaggctcactctagctgcacgagggatgtgtgtgccatttccatggggatagggggcacctcagtctctgggtggttccataatctgtgtatacctaagagcagttgcttcccacagagctgggctggctcactgggcactttgccatttctcctgcacctcccagctggagtttctgggtctaaaaggaaaaagtgaaggactcccacttggttgcttctctccagcttactgactgcaaattcccagggcgttgcccgctccctagggtggtttctgggggacggggcaggagcctggctttgctgctgctttgtcctctggagtcttttctcagactgctttgaattacacccctttcctttgtgtgctgaaatcttcccttcacactctccttccctgcctttcttttgtgtcttatcttactaggactggaagagggcagttgtgcaggaggtctgcatctaattccctaatccatgtgagagtgctcctgttgtgtgctttgtgacatgatggtgagaaatactccctagagcagtggctaccagaaggaagccatccccccccctgcacacacacacacacacacacacacacacacacacacacacacacactccttctggctgtcctcagatgcctattctaggtaaatgtcagattccaaagaaaatccagttgagatcttttttctttttttgagacgagagtcttgctgtgttgcccaggctggagtgcagtggcacaatctcggctcactgtaacctccgcctcctgggttcaagcgattctcctgcctcagcctcccaagtagctgggactacaggcgcgcaccaccacaccaggctaaaatttttttgtatttttagtagagacagggtttcactgtgttggccaggctggtctcgaactcctgacctcgtgttctgcccgcctcagcctcccagagtgctgggattacaggcttgagccatcgcgcccggcctccagttgggatcttgactggaatgactggtgttcaatcattatagtttccacctaatttgtatttgtacacaggacagttactaatttgttggtacttgtttgatccccagtccctagagttgtttatggggtggagcttcagtccctgctgcttcccctgtggcagcagctggagtcagggtggggacccagggtgctgctggcagattcttgagacaggtagaatctcctctatattggtgtctctctctgtcccagcagtgcccaggaaaacctggccagcctgtcactgacctctccacctagggcactggtggttcaggtccttctatttgccaccggcaaaccgtacttctgccagtctggctcttaggcccagtttctctgatcttgcagattttcttgggctctgctacggaatcctcatacctccggcaggtccctcctttgcccatgtgtttaactgtggtggaatcgtgtgagagctgcttctctcgcatggatcccagccacaccacattctacagcggttcctctgaaggcattgatagagatatttcctcctgttttgcatttcgttggtcatttcagtagaatcagggtgaaataaacatgggggctcagatgtcagcattacgaaccaagtacgtcaggcaggctgatgtggactgacctacactagtgagacgcaagatgacgaaaacaagggcactcactccaagttactgatgagatgtttggatcaaatgagccagtccttaagcagagttctctagtaaaagagatctcctttctgccctttcttgttccccaaaatgtgttgccttcatggtgaaaatttattttggcagattttctcttctttgataaaagcagccaacactttgttaaaagtctgtgaaacttatttacatgaagtatgtaaaggtaagaaaaaaacattatcaacaagaaatggagaaagccagcagctgaggacagaaaagtcatgcacagtgtcagtgtctatggaaacaggccacttggaccttgaggactaggtatttggaattggaggtgagcttggcctggtgagtctctaaccacttgtgtgtaggatcagtgtgagaaccctgctagaatatagtggcagagatgcaaggggaaatcattggagaagttaccagggaatgatgagctaatctgaaaaaaatacatgtttctaagttgggcgtggtagctcatctgtagtcccagctacttgagagcctgaggcaggaggatcgcttgagcccagcctgggcagcacagcgagaccctatctccctaaaaaaaactttttcgttgtttagttttgggatttttttttttcctggtcttttttccccctttttgtgaataacgggatctcactatgttgcccaggcagatctcgaactcctgggcccaagcaatcctcctgcctctgccttcctaagattacaggtatgagccactgtgttaagcaaaaaaacttttttaaatgaaaatcattttttaaaagacaggctttccaggggagggtattattccacttatatgaagtgtcaacagtaggcagatttgtggagacaaatagattagtggttaccaggggctgagaggagtgggagtggggagcaactgcttaatgggtaaagggttgtctttggaactagagagtagtgatggtcgcatgacattgtgaatgtactaaatgctattaatgataaattttatgttatgtgtattttaccacaattaaaaaaaaaagatcaaatgtcctcagaatagccaacaaccttccacttggctaaatgcctactcattaaacttcttgaactaaattcctttctgattgtcatggttattgtgtcctgggcttcagagtttcacattcaggttggcttggtccagtctgtcatgtatcactataggtccccacattggcctcttcctcagacggacagcccatctatctgccggggctctgtgccacagccagatagacttgctctgagacagctgtgtgggctctgagcactggccaggcatcacaaaacctatctttatgatttagaataattggtggtcagctgctgttttaatgttgttgttttttttaatttagatataattcacataccatgaaatttactcatttaaagtgtacaattcattcttcagtataattcataggctcacagaaaaaattgtttaaaaataaaatgtgcaattcagtgtcttttagtacattcacagagttgtgcaaccatcgcctctgtgtcattccagaacactttcagcacccaaaagaaaccccagacacaggagcagtcacctcttattacccgcagcccctggcaacaactcatccacttcctgtctctatggatttgcctattctggacatttcctataaatggaattatgcactatttggccttttgtgtctggcctctttcactgagcgtaatgtcctcaaggttcatctgcattgtagcatgtgtcagaatttctttcctttttgaggctgaatgatattatatcctatagataatgaggttttgattatccacccatcccttgggaatgcatatttgggttgcccccaccatttggctgttgtaaactgtgctgccatgaacactggtgtacggatatctgtttggttactggttttggttttttgtttgtttgttttggttttttgagacaaggtcttgctctgtcgcccaggctggattacagtggcacgatctctgctcactgcaacctccacctcccaggttcaagcaattctcctgcctcagtctcctgagtagctgggactacaggtagcactcaccaccatgcccggctaaatttttttgtatttttagtagagacaaggtttcgccatattggccaggctggtctcaaactcctgacctcaggtgatccacccacctcagcctcccaaagtgctgggattacagacgtgagccaccgcacccggcatagttgtggctttttgagagtgtatggctaggagtaaaattgccaggtcatatggtaactccatgtttaacatttgagaaactgccaaactgttctccacagcaggaattttttaacctgtatgtggtgggcttgtgtttcggttttcattttacacatctataaagatgagatttgctgtatggcactggttgcctgtatttggggagggttctgcttttggttggcaagaactgcattttatttaagcttagcaaaacataactggtttctcgcatcttctcaaaagtggaggattaagaaatggactgcgaattcagagcagggcagctgaacctcaggctccacccttgtagccttcaagctgaacctcattctctcttgctccctggagaccactgagacactctgcctgtgccagtttgatttctcacatttttaaagggccaaagcttgtgtctcaaagtgctatagcctttattgattcatgcagagaagcctccttgattccgtaattctgcagctaatactggaagtagaaagaattggaaacaccatctggatgacactttagggtggaagcagccagtacaagggggggctcattatttcctctggtcccagactgttcacctggagctgtagccaccaccctgcccttaggttaactgcctcgagtggtagtttagctctttgtgctgtgccgagggataactggaagtgaaaggtgctgagaaatgccatctcctgaaagtggcgagcatgagtgaatttacgaaaggttgggatattgctggggctctggaagtttctctggagctcactccaggggacagggagggggctggattccaattcaagtgaaaaatacctttcatctgccttgttcacctggcttttttgcctttttgtaaaatctgaaaacctcagggattgagtagtctttccttaactgcagttgcctgtctggccacacctgccagctgttgcttgtacccctgtaatttgcacggccttccgggcctttctcacaagatcactgcaggtcacattcatgaggaaaatgcaggcagttcctgccatcagacccctcaggatgtcatggtttggcctgaaaacaagattcctgcaactctaattttcctttgctagatcaaatgaaggatttgatctaatgtttgcattctagcagcaaaatcattgaatattttatttcttaagagccttacttcatattttgtaggtattttaagattttgtaaaggcctttctgcttcaacgtgtgatgtgtgcattcttagaaaaagatcttgtgttctgtaaatcacacaataaaaacatgagttcgtgcaggaaaaactggggcggggtggatcactccaaacttgtgtggtgtggtaactggagctcactgatgaaaccatgaacagttctggctgaaagaaccccacagtacactgaggtctgttggcatcgccgccagcaccgccccggtccctttgtgcgcgccaccacacctggctaattttttatttttagtagagagggggtttcaccatgttggtcaggatggcctcgaactgacctcgtgatccgcccacctcagcctcccaaagtgctgggattacaggtgtgagcctccgtgcccagccttcagctttttttcttaatgtctttgtgtaatatgaaggcattctctttaattgttaaaaagcttgcctaccactgcttcaaaatattactgtcagttggcatagcttctgattatattgatgtcatctcccttcttttaaacatgttaccatattggcactgtatttcccctagcccattgatcacttgagagttagtcatagtcctcgtgctgtttcactcctaaacgtttaagcatgcctttcctaagagcagacagtacagttaagacactcaggaagtttagcaatgagctaacacagaaccttacatttctccacataccccataaatgccttttttagagcctttgagcctggaatgcagagtccaggactgtgtgttgtattcgattgtgtcatcccttcagtctcctttatcagaaatgttcccccacccccttgttttctctcatcatcttgagtccagaccgtggttgcatggcacgccctctctggactcttcctgctgtctcctcacggtaagcttcagtctcctactcgtgatgctggttcatctcagcagcactgaggggcctgagctcagtttggtcgtgtgttaaggtggtgcctgccagatttctccacagaaaagggccccgtacttttatttgctcttcagcctgtgtattccttcctttcttgccagcttgtgggtggcttctctagcagcttctgtaagatactcagtttggcagttgtagttgtttcagcaggagaggtgtctgcatacctgaccaccacatggctagaagtcgatccatcctctggcgtaaccatcctccatgctactgtccctggggcactgaggccctcctcagtgacttcctccacctcatcttccgccatctccaagccaccagtgtccaacggactactgatatgtcccaaactcatcatttgtttattcaccaattcagagcccacctttttttcagcactgagctagcctctccttgctagaagcttacggtcgaaggtctccagccatcagaagaagcacgtggagcgctgcgtccgtgttgtggttattcatccagcatgtgttgagtaagggttgcacctgtgcctggcattatgcattgagcggggagatgggggttggcacgcacagtggggtgttctaagtacactgagggctcgggtgccctggctcatagagcagggagggaggcaggagcagggaaggtgtctcagaagtgccatctttttttttttttttttgggaagtggaatcttgttctatcgcctggtctggagtgcaatggcactatctcaactcactgcagcctccgcctcccaggttcaagcgattctcatgcctcagtccccgagtagctgggaccacaggcgcacaccaccacacccggcaaatattttgtatttttagtagaggcggagttttgccatgttggccaggctggtcttaaactcctggcctcaagtgatctgctcacctcggcctcctaaggtgttgggattacaggcatgagccactgcgcccggtctagaagtgccatcctaactgaacctgaaagatgaaagttctccagatgaacctgaaagttctccaaatgaaaaggtgggagggggtgacagggttaggcccagagcctctggtgacacagggtgggcatcattggtcactttttcctcgagggaggggcgtcacacgggtgatagggtgggagctataaccatgttgatagtgccgcctctgcccatctggcctggcatgccctgagccctctgtcccacctgtggaactcataagccctgacagcccactcactcctgattcattatccacacccctgtgcttccgctgtgcctggagcaagctttcttcagggggaagggaggctggaactatgttgtagttacctatttgtcctcccttccaaactgtgagttcttggaggtggaaggatgctgcaggatctggctcaggacgaaggcagttggtgaacagacacgtgtgtttttgactcacggtgatctcagacaagttcctctgtctagtcgaacttctttttttccatctgtaacactcaggagttgaataggtggtttttctgaggatacttcaactgtaaaatgtatgaacttgtgaactagctatttagttctcctcataatcaagattgtgtgtgtgtggggggttctgattagagggaggatgaagagaggtgtatggggttttttttgttttgttttctgtttgtttgtttgtttttgagatggagtctcactctgtcacccaggctggagtgcagtggcacgatttcggttcactgcaacctctgcctcctgggttcaagtgattctcctgcctcagcctcctgagtaactgggattacaggcatgcaccaccatgcccagctaatttttgtatttttaatagagatggggttttcgccatgttggccaggctggtctcgaactcctgacctcaggtgatccacctgcctcggcctcccaaagtgctgggattataggcatgagccaccacacctggcaggtttctttgaaaaagtttgtgtttcggcaaacaccataaaccccctgggggacagccttggggagtcacctggcaccctagcccagcctccctcccttgggtcctgcagtgaaggcttagtgagggtgtgcaaatgcccaggtcaccctgggactgggcaggccctctgggctaagggtaaactcatttggaatacctgttttctatcattgttttttatttgttaaatttaaagggtacaagtgcagttttgttgcgtggatatattgtatagtagtgaagtctgagctttcagtgtaaccatcacctgaatagtggacattgtacccgttaagtaatgtctcatccctcaccccctcccacccttcccagtctctccagtgtctgccattcctcactctgtccatgtgcacatgctattcagctcctgcttctaagtgagaacgtacggtatttgactttctgtgtctgagctgtgtcactgaagacaatggactccagctccatccacgttttttatcatttttacctgcactccacacccagcacaatccaggcttctttgtgggttttttgaaatttgtctttaattataaaagtagcagccagcaaattaacaaacacccatgtgcctttcattgcacagaattgaaaatcatcatactatatttgcttcaagtaatttccattagaaagaactagaatattacagtagagttaaagaccctttatttcccatcttcagtgctcttaaaagttcatttagggccaggcatggtggctcacacctataatcccagcactttgagaggcccaggtgggtggatcacctgaggtcaggagttcaagaccagcctggccaacatggcgaaaccccatctctactaaaaatacaaaaattagctgggcgtggtggtgcgcatctgtaatctcagctactcgggaggctgaggcaggagaatcgcttgaactcaggagggaggcagagcctgtatgcagtaagccgagattgcgccaccacaccccagcatgggtgacagagcaagactccgtctcaaaaaaaaaaaaaaaaaagttcattcattgtacacttagaaatagttaaaaaggtaaactttgttttgtgtgtgtgtgtatatatatatatatatatatatatatatatatatatatatatgtatttttttttgagacatatatgtgtctggtttgttcgcccaggcaggagtgcagtggcatgatcaacggctcactgcagcctcaacttcctaggctcaagtgatcctcctgcctcagcctcccgagtagctaggattacaggcacacaccaccatgcccagctaattttttttttttttttttttttttgtagagacagggttttgctatgttgcccaggctggtctcaaactcctgagctcaagcgatccacctgcctcacctcccaaagtgctgggattacaagtgtaagccaccacacctgacctgttttgtatattttaccacaataaaaagcctttaaaaccccaagcagacagttcattttcattcaggcccaactcagaatctgatcacagcggggtttcccccctttctagcgagtagctgaagaactgttttctctccttgatggtataactgtctctgtgggtgttgctcccctgccgctccagtggttttgtttttgtttttgtttttttgagacggagtcttgcgatctcagctcactgcgacctctgcctcctgggttcaggcgattcttctccctcagccttccatgtagctgggacttacaggcacctgccaccacgcccggctcatttttgtatttttagtagagacggagtttcaccatgttggccaggttgggctcgaactccagacctcaggtgatccacctgcctcagcctcccacagtgctgggattacaggtgagagccactgcacccagccggcccctcagtcttttccttctcaatcagtggcaccaccatcttcccaggctttggacatggtccctgactcacccttgcccctcacccccacactaatccacctgcgagctctgttgcttcaccacctagaccagccccaaatcctcaactgcccccaccctgggccacacctggaccactgctagaggcctctcatgggccctccctgtttttctcttgcactccccgggctttctggcacaagatgccccagaagcagaatcacatatctctcctgggagccaatctagtgtgtttactgcccctggagtgttattgttggccttagaatatgtcccactacaggtttgcagagcactgtagtcaaaagtcatttgaaataaatcttttctctgtggtatattgtcaatttgatatagaattaaatttgtttcttttcttttttcttttctttttttttttttttaagagacagggtcttggccaggcgtggtgtctcatgcctgtaatcccggcactttgggaagccaaggtgggtggatcgcctgaggtcaggaattcaagaccaacctggccagcatggtgaaaccccgtctctgctaaaaatacaaaaattagccgggcgtgatggcaggtacctgtaatcccagctactcgggaagctgaggcaggagaaggcttgaactcaggagtcggaggttgcagtgagccaagatcacgccatggcactctagcaagactctgtctcaaaaaaaaaaaaagagagagagagagacagggtcttgctctgtcactcaggctggagtgcagtgatgtagtcatggctcactgcagcctcatactcctgacctcaggtgatcgacccgcctcggcctcccaaagtgctgggatcgtaggctgaagccaccatgcctggcccgaactcatttgtttttatttgcattaagtgtaataaggttttgttacttttagtttgaattttattttgggtaatataaacatttacatgattcagaagtcagaattacactgaggcatgttcagctaggcctcactcctgtgcctgtacccttacctttttccccctaccccatgcagggaatcaatttcattagttcctggtgtgtccttccttaatacccccccttctttctttggtagaatgcagtagatatgtttgcgctttgctccctttgcttcacagtggatcctggaaatgactccatcgcagttcttagagctcttgtttagtccctttggatctgcacagtactccagtgtgtgggcgcaccataagtttattcagcaagtgccctggtgatagggatcgggggtattggaagcctttggctggtaaaaataatgttgtagcaaataacatcatgcatatgttctttgagatttctggaggtgtctctttagcatagatttctagaaggcattccttacgtcacgtttaggtttatagtttgacctcatggtgattaaggtatttgggaaatgcaaatgagagtttcgaagaagccagatctttcccattagttcactgtttttctctgacattaggaccgtccgggttctagggagcagccctggcgttaggcagtgccatgatggattgtgtagaagtagcgattcccatctgtctgctttcttggcccactctgctggtggctccccttccctccctcctttatggggagctggggagctgcctaggggtccattctcaaaggctgatctctggtgggcaacaggccacacctagctttccagggttcttcgtcatttcccattgagagctgtaagactcagagacatgaaaaggaagctctggctgggcacggtggctcacgcctgtaatcccagcactttgggaggctgaggcgggtcgatcacctgaggtcaggagttcgagaccagcctgcccaacatggtgaaaccccgtctccactaaacatacaaaaattagcctggcgtggtagcacacgcctgtgatcccagctactccggaggctgaggcaggagaataacttgaacccggcaggcggaggttgcgatgagccgatattatgccatcggcaacagagcgagactccatctcaaaaaaaaaacaaaaaacaaaacaaggcgagctctgtgctgggacagattagggacccctctttacagcaagaaagactgctctgtgggttgtaggatgcctttgtgtatgcagtggctctaggtgactctggcagccacactctgggccctaaacttctggaggaagatacaggatagggaggaactcaggggtgagtcatggtggggacaagacattccctcactctaagaccttgtcactagattggaacatctcttgcctccctacacctgacctgatggttctggagagatacgtccttgcagcttctgagtcccagcactaagcagcctttggtaacttccctacatcatttgagttctggtttcctaaggatgcttgccagtgagtgccatggtgccctcattgcacagtctgtgcagtgtagacaagaggggaagtctcttggggtagaccagccgcaaggcggtgactagcactgatgtgaaccacatgggacaggggagttgtggggctgagaacacggagggtgggagtagtcatgctcttttccagaatgaactgctaacgaagggactcgcaggtggctgctgcttctttccaagctgcccctgttgttgcagaggctctggagtcctaggaggtttcacggtggcatactcgacagagtactagagcatcatggccagatagtgatgctggggtgtggggcctcacggtggccatttctgacgagaccccaccgggccaaagtgatgtgtagagaaggagctgcttcggtcaccagaaaagaacggggaagcctcccacactagaataggtagggtgctcttctccaccggcaggaaggggatgtatggctctgcctggaccacacctttttccttgctcttccctccgcatctgctgtggccgaggccattcctcatcagggaacatgtgttagaggctcacgccacctgggaccacttgtcttatcacccccaggaccctaggcggtagtttcctgtggcctgagttagctgatatttatatagtgccattgtgccttttctcctgtgatgctcacagtaaggatgcctagatggggttacctgttgtcaagataaggaaactgaagcacagaatgctgaggtcatttgctgggttcatgtttggaaagcggcaaaggatttcagtgcaggttggctggctccaaacctgtgtgtgctttccatgacactgtactgtgtgcctcattgagcctcattctagaaaaccaaaaacacacccaaggcccggccttcacaaaggagacccctcccccatttggctccctttccagcagtcgacggcctcttgtcagccatcgagcccagagtcccttgaagtgcgactcatgctggggtggtatgctcaggagccgcagtgtttccgctcagaggaaagggctctgattctcctgcagtgctaggagacttgtgggtggccacagtgcaggtcaggcacaccggccagcaccacccacagcccaaattcctaaagaaatatttgggtcccagcttggcccgagtctctgttgtcctggggaaggacatcaagatctgagtgtatgatggcctggggccttgcatgtggtgggggtccaagcctgcctctgctcacttgttctgcagactggcatgttctctgtgatacttacatacttgtttaacacttcagggaagaaaagtcagaagaccaggacctccagggcctcaaggacaaacccctcaagtttaaaaaggtgaagaaagataagaaagaagagaaagagggcaagcatgagcccgtgcagccatcagcccaccactctgctgagcccgcagaggcaggcaaagcagagacatcagaagggtcaggctccgccccggctgtgccggaagcttctgcctcccccaaacagcggcgctccatcatccgtgaccggggacccatgtatgatgaccccaccctgcctgaaggctggacacggaagcttaagcaaaggaaatctggccgctctgctgggaagtatgatgtgtatttgatcaagtaagtaagagcaactcctatctctacagggcagggagggcagggacaaggatccctcatggagcaggaaaatgtatgtgcccagggtggggtcggggggaacataaacaatgaacactgagaccaggtgtgcttgaaatgaccgtgtacagaggtcgctgccctgagtgggaagttctcaaggtagcaggccctctatcctctccacacctcaagtctttatctggggatggaatagctgcggaagcagaggaacttgcagagctaggggttcagaggggtgaagaagcatgtttcagttctgccttttaaatgatcccaaaaaggttagcagttttcaaatgacatttgcagacagcctcatttaattccatgagaagggtgagcaaaggattatcttgttgaaactgattcctggagagactgagcaccgtacctgagttcaaacttgggaatgttctagatggtgactcaggcccaggcaccaaccagcagaatgggcctcagcctgacaacccttctgtaccaggcctgactctttggttgctgaactttggagaggcctgggggggtcagcggcaggcagacgagtgagtggctttggtgacaggtcctcaggggcagccaggcagtgtgactctcgttcaatagtaacgtttgtcagagcgttgtcaccaccatccgctctgccctatctctgacattgctatggagagcctctaattgttccttgtgtctttctgtttgtccccacagtccccagggaaaagcctttcgctctaaagtggagttgattgcgtacttcgaaaaggtaggcgacacatccctggaccctaatgattttgacttcacggtaactgggagagggagcccctcccggcgagagcagaaaccacctaagaagcccaaatctcccaaagctccaggaactggcagaggccggggacgccccaaagggagcggcaccacgagacccaaggcggccacgtcagagggtgtgcaggtgaaaagggtcctggagaaaagtcctgggaagctccttgtcaagatgccttttcaaacttcgccagggggcaaggctgaggggggtggggccaccacatccacccaggtcatggtgatcaaacgccccggcaggaagcgaaaagctgaggccgaccctcaggccattcccaagaaacggggccgaaagccggggagtgtggtggcagccgctgccgccgaggccaaaaagaaagccgtgaaggagtcttctatccgatctgtgcaggagaccgtactccccatcaagaagcgcaagacccgggagacggtcagcatcgaggtcaaggaagtggtgaagcccctgctggtgtccaccctcggtgagaagagcgggaaaggactgaagacctgtaagagccctgggcggaaaagcaaggagagcagccccaaggggcgcagcagcagcgcctcctcaccccccaagaaggagcaccaccaccatcaccaccactcagagtccccaaaggcccccgtgccactgctcccacccctgcccccacctccacctgagcccgagagctccgaggaccccaccagcccccctgagccccaggacttgagcagcagcgtctgcaaagaggagaagatgcccagaggaggctcactggagagcgacggctgccccaaggagccagctaagactcagcccgcggttgccaccgccgccacggccgcagaaaagtacaaacaccgaggggagggagagcgcaaagacattgtttcatcctccatgccaaggccaaacagagaggagcctgtggacagccggacgcccgtgaccgagagagttagctgactttacacggagcggattgcaaagcaaaccaacaagaataaaggcagctgttgtctcttctccttatgggtagggctctgacaaagcttcccgattaactgaaataaaaaatatttttttttctttcagtaaacttagagtttcgtggcttcagggtgggagtagttggagcattggggatgtttttcttaccgacaagcacagtcaggttgaagacctaaccagggccagaagtagctttgcacttttctaaactaggctccttcaacaaggcttgctgcagatactactgaccagacaagctgttgaccaggcacctcccctcccgcccaaacctttcccccatgtggtcgttagagacagagcgacagagcagttgagaggacactcccgttttcggtgccatcagtgccccgtctacagctcccccagctccccccacctcccccactcccaaccacgttgggacagggaggtgtgaggcaggagagacagttggattctttagagaagatggatatgaccagtggctatggcctgtgcgatcccacccgtggtggctcaagtctggccccacaccagccccaatccaaaactggcaaggacgcttcacaggacaggaaagtggcacctgtctgctccagctctggcatggctaggaggggggagtcccttgaactactgggtgtagactggcctgaaccacaggagaggatggcccagggtgaggtggcatggtccattctcaagggacgtcctccaacgggtggcgctagaggccatggaggcagtaggacaaggtgcaggcaggctggcctggggtcaggccgggcagagcacagcggggtgagagggattcctaatcactcagagcagtctgtgacttagtggacaggggagggggcaaagggggaggagaagaaaatgttcttccagttactttccaattctcctttagggacagcttagaattatttgcactattgagtcttcatgttcccacttcaaaacaaacagatgctctgagagcaaactggcttgaattggtgacatttagtccctcaagccaccagatgtgacagtgttgagaactacctggatttgtatatatacctgcgcttgttttaaagtgggctcagcacatagggttcccacgaagctccgaaactctaagtgtttgctgcaattttataaggacttcctgattggtttctcttctccccttccatttctgccttttgttcatttcatcctttcacttctttcccttcctccatcctcctccttcctagttcatcccttctcttccaggcagccgcggtgcccaaccacacttgtcggctccagtccccagaactctgcctgccctttgtcctcctgctgccagtaccagccccaccctgttttgagccctgaggaggccttgggctctgctgagtccgacctggcctgtctgtgaagagcaagagagcagcaaggtcttgctctcctaggtagccccctcttccctggtaagaaaaagcaaaaggcatttcccaccctgaacaacgagccttttcacccttctactctagagaagtggactggaggagctgggcccgatttggtagttgaggaaagcacagaggcctcctgtggcctgccagtcatcgagtggcccaacaggggctccatgccagccgaccttgacctcactcagaagtccagagtctagcgtagtgcagcagggcagtagcggtaccaatgcagaactcccaagacccgagctgggaccagtacctgggtccccagcccttcctctgctcccccttttccctcggagttcttcttgaatggcaatgttttgcttttgctcgatgcagacagggggccagaacaccacacatttcactgtctgtctggtccatagctgtggtgtaggggcttagaggcatgggcttgctgtgggtttttaattgatcagttttcatgtgggatcccatctttttaacctctgttcaggaagtccttatctagctgcatatcttcatcatattggtatatccttttctgtgtttacagagatgtctcttatatctaaatctgtccaactgagaagtaccttatcaaagtagcaaatgagacagcagtcttatgcttccagaaacacccacaggcatgtcccatgtgagctgctgccatgaactgtcaagtgtgtgttgtcttgtgtatttcagttattgtccctggcttccttactatggtgtaatcatgaaggagtgaaacatcatagaaactgtctagcacttccttgccagtctttagtgatcaggaaccatagttgacagttccaatcagtagcttaagaaaaaaccgtgtttgtctcttctggaatggttagaagtgagggagtttgccccgttctgtttgtagagtctcatagttggactttctagcatatatgtgtccatttccttatgctgtaaaagcaagtcctgcaaccaaactcccatcagcccaatccctgatccctgatcccttccacctgctctgctgatgacccccccagcttcacttctgactcttccccaggaagggaaggggggtcagaagagagggtgagtcctccagaactcttcctccaaggacagaaggctcctgcccccatagtggcctcgaactcctggcactaccaaaggacacttatccacgagagcgcagcatccgaccaggttgtcactgagaagatgtttattttggtcagttgggtttttatgtattatacttagtcaaatgtaatgtggcttctggaatcattgtccagagctgcttccccgtcacctgggcgtcatctggtcctggtaagaggagtgcgtggcccaccaggcccccctgtcacccatgacagttcattcagggccgatggggcagtcgtggttgggaacacagcatttcaagcgtcactttatttcattcgggccccacctgcagctccctcaaagaggcagttgcccagcctctttcccttccagtttattccagagctgccagtggggcctgaggctccttagggttttctctctatttccccctttcttcctcattccctcgtctttcccaaaggcatcacgagtcagtcgcctttcagcaggcagccttggcggtttatcgccctggcaggcaggggccctgcagctctcatgctgcccctgccttggggtcaggttgacaggaggttggagggaaagccttaagctgcaggattctcaccagctgtgtccggcccagttttggggtgtgacctcaatttcaattttgtctgtacttgaacattatgaagatgggggcctctttcagtgaatttgtgaacagcagaattgaccgacagctttccagtacccatggggctaggtcattaaggccacatccacagtctcccccacccttgttccagttgttagttactacctcctctcctgacaatactgtatgtcgtcgagctccccccaggtctacccctcccggccctgcctgctggtgggcttgtcatagccagtgggattgccggtcttgacagctcagtgagctggagatacttggtcacagccaggcgctagcacagctcccttctgttgatgctgtattcccatatcaaaagacacaggggacacccagaaacgccacatcccccaatccatcagtgccaaactagccaacggccccagcttctcagctcgctggatggcggaagctgctactcgtgagcgccagtgcgggtgcagacaatcttctgttgggtggcatcattccaggcccgaagcatgaacagtgcacctgggacagggagcagccccaaattgtcacctgcttctctgcccagcttttcattgctgtgacagtgatggcgaaagagggtaataaccagacacaaactgccaagttgggtggagaaaggagtttctttagctgacagaatctctgaattttaaatcacttagtaagcggctcaagcccaggagggagcagagggatacgagcggagtcccctgcgcgggaccatctggaattggtttagcccaagtggagcctgacagccagaactctgtgtcccccgtctaaccacagctccttttccagagcattccagtcaggctctctgggctgactgggccaggggaggttacaggtaccagttctttaagaagatctttgggcatatacatttttagcctgtgtcattgccccaaatggattcctgtttcaagttcacacctgcagattctaggacctgtgtcctagacttcagggagtcagctgtttctagagttcctaccatggagtgggtctggaggacctgcccggtgggggggcagagccctgctccctccgggtcttcctactcttctctctgctctgacgggatttgttgattctctccattttggtgtctttctcttttagatattgtatcaatctttagaaaaggcatagtctacttgttataaatcgttaggatactgcctcccccagggtctaaaattacatattagaggggaaaagctgaacactgaagtcagttctcaacaatttagaaggaaaacctagaaaacatttggcagaaaattacatttcgatgtttttgaatgaatacgagcaagcttttacaacagtgctgatctaaaaatacttagcacttggcctgagatgcctggtgagcattacaggcaaggggaatctggaggtagccgacctgaggacatggcttctgaacctgtcttttgggagtggtatggaaggtggagcgttcaccagtgacctggaaggcccagcaccaccctccttcccactcttctcatcttgacagagcctgccccagcgctgacgtgtcaggaaaacacccagggaactaggaaggcacttctgcctgaggggcagcctgccttgcccactcctgctctgctcgcctcggatcagctgagccttctgagctggcctctcactgcctccccaaggccccctgcctgccctgtcaggaggcagaaggaagcaggtgtgagggcagtgcaaggagggagcacaacccccagctcccgctccgggctccgacttgtgcacaggcagagcccagaccctggaggaaatcctacctttgaattcaagaacatttggggaatttggaaatctctttgcccccaaacccccattctgtcctacctttaatcaggtcctgctcagcagtgagagcagatgaggtgaaaaggccaagaggtttggctcctgcccactgatagcccctctccccgcagtgtttgtgtgtcaagtggcaaagctgttcttcctggtgaccctgattatatccagtaacacatagactgtgcgcataggcctgctttgtctcctctatcctgggcttttgttttgctttttagttttgcttttagtttttctgtcccttttatttaacgcaccgactagacacacaaagcagttgaatttttatatatatatctgtatattgcacaattataaactcattttgcttgtggctccacacacacaaaaaaagacctgttaaaattatacctgttgcttaattacaatatttctgataaccatagcataggacaagggaaaataaaaaaagaaaaaaaagaaaaaaaaacgacaaatctgtctgctggtcacttcttctgtccaagcagattcgtggtcttttcctcgcttctttcaagggctttcctgtgccaggtgaaggaggctccaggcagcacccaggttttgcactcttgtttctcccgtgcttgtgaaagaggtcccaaggttctgggtgcaggagcgctcccttgacctgctgaagtccggaacgtagtcggcacagcctggtcgccttccacctctgggagctggagtccactggggtggcctgactcccccagtccccttcccgtgacctggtcagggtgagcccatgtggagtcagcctcgcaggcctccctgccagtagggtccgagtgtgtttcatccttcccactctgtcgagcctgggggctggagcggagacgggaggcctggcctgtctcggaacctgtgagctgcaccaggtagaacgccagggaccccagaatcatgtgcgtcagtccaaggggtcccctccaggagtagtgaagactccagaaatgtccctttcttctcccccatcctacgagtaattgcatttgcttttgtaattcttaatgagcaatatctgctagagagtttagctgtaacagttctttttgatcatctttttttaataattagaaacaccaaaaaaatccagaaacttgttcttccaaagcagagagcattataatcaccagggccaaaagcttccctccctgctgtcattgcttcttctgaggcctgaatccaaaagaaaaacagccataggccctttcagtggccgggctacccgtgagcccttcggaggaccagggctggggcagcctctgggcccacatccggggccagctccggcgtgtgttcagtgttagcagtgggtcatgatgctctttcccacccagcctgggataggggcagaggaggcgaggaggccgttgccgctgatgtttggccgtgaacaggtgggtgtctgcgtgcgtccacgtgcgtgttttctgactgacatgaaatcgacgcccgagttagcctcacccggtgacctctagccctgcccggatggagcggggcccacccggttcagtgtttctggggagctggacagtggagtgcaaaaggcttgcagaacttgaagcctgctccttcccttgctaccacggcctcctttccgtttgatttgtcactgcttcaatcaataacagccgctccagagtcagtagtcaatgaatatatgaccaaatatcaccaggactgttactcaatgtgtgccgagcccttgcccatgctgggctcccgtgtatctggacactgtaacgtgtgctgtgtttgctccccttccccttccttctttgccctttacttgtctttctggggtttttctgtttgggtttggtttggtttttatttctccttttgtgttccaaacatgaggttctctctactggtcctcttaactgtggtgttgaggcttatatttgtgtaatttttggtgggtgaaaggaattttgctaagtaaatctcttctgtgtttgaactgaagtctgtattgtaactatgtttaaagtaattgttccagagacaaatatttctagacactttttctttacaaacaaaagcattcggagggagggggatggtgactgagatgagaggggagagctgaacagatgacccctgcccagatcagccagaagccacccaaagcagtggagcccaggagtcccactccaagccagcaagccgaatagctgatgtgttgccactttccaagtcactgcaaaaccaggttttgttccgcccagtggattcttgttttgcttcccctccccccgagattattaccaccatcccgtgcttttaaggaaaggcaagattgatgtttccttgaggggagccaggaggggatgtgtgtgtgcagagctgaagagctggggagaatggggctgggcccacccaagcaggaggctgggacgctctgctgtgggcacaggtcaggctaatgttggcagatgcagctcttcctggacaggccaggtggtgggcattctctctccaaggtgtgccccgtgggcattactgtttaagacacttccgtcacatcccaccccatcctccagggctcaacactgtgacatctctattccccaccctccccttcccagggcaataaaatgaccatggagggggcttgcactctcttggctgtcacccgatcgccagcaaaacttagatgtgagaaaaccccttcccattccatggcgaaaacatctccttagaaaagccattaccctcattaggcatggttttgggctcccaaaacacctgacagcccctccctcctctgagaggcggagagtgctgactgtagtgaccattgcatgccgggtgcagcatctggaagagctaggcagggtgtctgccccctcctgagttgaagtcatgctcccctgtgccagcccagaggccgagagctatggacagcattgccagtaacacaggccaccctgtgcagaagggagctggctccagcctggaaacctgtctgaggttgggagaggtgcacttggggcacagggagaggccgggacacacttagctggagatgtctctaaaagccctgtatcgtattcaccttcagtttttgtgttttgggacaattactttagaaaataagtaggtcgttttaaaaacaaaaattattgattgcttttttgtagtgttcagaaaaaaggttctttgtgtatagccaaatgactgaaagcactgatatatttaaaaacaaaaggcaatttattaaggaaatttgtaccatttcagtaaacctgtctgaatgtacctgtatacgtttcaaaaacaccccccccccactgaatccctgtaacctatttattatataaagagtttgccttataaatttacataaaaatgtccgtttgtgtcttttgttgtaaaaatcaagtgattttttcataaggttcttttactattggaaaagatgggcagcacgcagttttattttatttttgtaagttttttaatacatgtgaaagcaaagaatactcagcatgcctttctaagtgacgcgtttgcaccttttgttgggaagtactgtatcctgtgctgttagcattctcgataaatctctctgtgaaagtgactcaaggtctgggctttcattataagacagaagtccccctccagctcacatgacagcatggtgctgcgtttcctcattggatctggctgtccctggacacaggtagctgccttcaggcctgccacgagcggccaagggaagcctcctccatatgctggcctcgctggcccctcagcttcttccaagccagtgctctccaggcacactgctccagcgtgtgacgggaagggcctggcatgagtcagcctgcagcacaacctccctgctccagacccgtatggtaggggcaccccctaggtctggatgtgctgtggtgcttttggacacccccacccccgcaggctgtggctcctcctgtgtctcattctggccaggaccctcacgtgccctctgttgactgctaacgtggttctctgaccaggcaagggcaggctgaggggtttgcccaaagggggcccccttgttactggcttccttggctctcaggagcagcctcaccaggttggtaaggggctggaggagacaactgctcaaaggagtccagcttcacatgcacatgctagaaggtaccctcggaaggcctggccttcaaaggtagatcccagggttgaaaagtcaacttgtatgcattgagcatctcgtatgccagccctgttccgtgagctgatgggcctttgtgtgtaagtaggaccaagtgcccccgtggaggttagcatgggtgtgcagtcatttcagatacttgagttggtacatctcagtaaagtctgtcccgtgagaagccatgggtttcatggtatggttggcatcttccttgggagtggccacagtggtggtggcttcaggaaagagactccaacaggggccagctgtgggccttgggcacttctcgtttctaggaaaagtcctaagtctgtagggctaggggtggggaaccccttcgctgtcaggatcaagagggcaaggggaactgtcgctggaggagacatccagctggagaaacaaaagagtaagtctgcgttgctgcttgtggggtcttccccatctcagggcggggaccgggggtggcggtccagacaagtaatcaaggacgatgcccaggaggggacaggtacggggtggcaggagctctgccggcgggctcaggaagccttcaccacagctgcctgagctcacccttgccaaatgagggctggggcagcagcaacgcatacactcacggctgtggcgggcagcgttctcggcatatttcaggacacctaaggagactgaatggctcaaggctgctgccgtgtgcagggggctagacgtggggcgggcaggcagggctcctggtaacagccctgcaggccgcagtggagagcagggttccggcagggccgcccaggagctttcggaaggcccggccccggcccctttccgagcagcccgggcctccgccctgccctctgtccccaacgccgggagccgccgttcgtcctccagagccccgcccgggcgagcccgggaggccgatcgccgctcgcggaacccgccgggacccgggccctccccggcgcggggcgcccccgtgtgacccagcgcgcggccgcggcgcgcaagatggcggcgggcccgggcaccgccccttccgccccgccgggcgtcgcacgaggccggctcgaaggggaagtgagtcagtgtccgcggacccggccggcccaggcccgcgcccgccgcggccctgagaggccccggcaggtcccggcccggcggcggcagccatggccggggggccgggcccgggggagcccgcagcccccggcgcccagcacttcttgtacgaggtgccgccctgggtcatgtgccgcttctacaaagtgatggacgccctggagcccgccgactggtgccagttcggtgggtggcggcgggctgccggggggcgggaggcgcgcgggctcctggcgccgacgcctgacgccc

SEQ ID NO: 2 - RNA, 10241 nt, Homo sapiens
  source 1..10241: mol_type = mRNA
ccggcgtcggcggcgcgcgcgctccctcctctcggagagagggctgtggtaaaagccgtccggaaaatggccgccgccgccgccgccgcgccgagcggaggaggaggaggaggcgaggaggagagactgctccataaaaatacagactcaccagttcctgctttgatgtgacatgtgactccccagaatacaccttgcttctgtagaccagctccaacaggattccatggtagctgggatgttagggctcagggaagaaaagtcagaagaccaggacctccagggcctcaaggacaaacccctcaagtttaaaaaggtgaagaaagataagaaagaagagaaagagggcaagcatgagcccgtgcagccatcagcccaccactctgctgagcccgcagaggcaggcaaagcagagacatcagaagggtcaggctccgccccggctgtgccggaagcttctgcctcccccaaacagcggcgctccatcatccgtgaccggggacccatgtatgatgaccccaccctgcctgaaggctggacacggaagcttaagcaaaggaaatctggccgctctgctgggaagtatgatgtgtatttgatcaatccccagggaaaagcctttcgctctaaagtggagttgattgcgtacttcgaaaaggtaggcgacacatccctggaccctaatgattttgacttcacggtaactgggagagggagcccctcccggcgagagcagaaaccacctaagaagcccaaatctcccaaagctccaggaactggcagaggccggggacgccccaaagggagcggcaccacgagacccaaggcggccacgtcagagggtgtgcaggtgaaaagggtcctggagaaaagtcctgggaagctccttgtcaagatgccttttcaaacttcgccagggggcaaggctgaggggggtggggccaccacatccacccaggtcatggtgatcaaacgccccggcaggaagcgaaaagctgaggccgaccctcaggccattcccaagaaacggggccgaaagccggggagtgtggtggcagccgctgccgccgaggccaaaaagaaagccgtgaaggagtcttctatccgatctgtgcaggagaccgtactccccatcaagaagcgcaagacccgggagacggtcagcatcgaggtcaaggaagtggtgaagcccctgctggtgtccaccctcggtgagaagagcgggaaaggactgaagacctgtaagagccctgggcggaaaagcaaggagagcagccccaaggggcgcagcagcagcgcctcctcaccccccaagaaggagcaccaccaccatcaccaccactcagagtccccaaaggcccccgtgccactgctcccacccctgcccccacctccacctgagcccgagagctccgaggaccccaccagcccccctgagccccaggacttgagcagcagcgtctgcaaagaggagaagatgcccagaggaggctcactggagagcgacggctgccccaaggagccagctaagactcagcccgcggttgccaccgccgccacggccgcagaaaagtacaaacaccgaggggagggagagcgcaaagacattgtttcatcctccatgccaaggccaaacagagaggagcctgtggacagccggacgcccgtgaccgagagagttagctgactttacacggagcggattgcaaagcaaaccaacaagaataaaggcagctgttgtctcttctccttatgggtagggctctgacaaagcttcccgattaactgaaataaaaaatatttttttttctttcagtaaacttagagtttcgtggcttcagggtgggagtagttggagcattggggatgtttttcttaccgacaagcacagtcaggttgaagacctaaccagggccagaagtagctttgcacttttctaaactaggctccttcaacaaggcttgctgcagatactactgaccagacaagctgttgaccaggcacctcccctcccgcccaaacctttcccccatgtggtcgttagagacagagcgacagagcagttgagaggacactcccgttttcggtgccatcagtgccccgtctacagctcccccagctccccccacctcccccactcccaaccacgttgggacagggaggtgtgaggcaggagagacagttggattctttagagaagatggatatgaccagtggctatggcctgtgcgatcccacccgtggtggctcaagtctggccccacaccagccccaatccaaaactggcaaggacgcttcacaggacaggaaagtggcacctgtctgctccagctctggcatggctaggaggggggagtcccttgaactactgggtgtagactggcctgaaccacaggagaggatggcccagggtgaggtggcatggtccattctcaagggacgtcctccaacgggtggcgctagaggccatggaggcagtaggacaaggtgcaggcaggctggcctggggtcaggccgggcagagcacagcggggtgagagggattcctaatcactcagagcagtctgtgacttagtggacaggggagggggcaaagggggaggagaagaaaatgttcttccagttactttccaattctcctttagggacagcttagaattatttgcactattgagtcttcatgttcccacttcaaaacaaacagatgctctgagagcaaactggcttgaattggtgacatttagtccctcaagccaccagatgtgacagtgttgagaactacctggatttgtatatatacctgcgcttgttttaaagtgggctcagcacatagggttcccacgaagctccgaaactctaagtgtttgctgcaattttataaggacttcctgattggtttctcttctccccttccatttctgccttttgttcatttcatcctttcacttctttcccttcctccgtcctcctccttcctagttcatcccttctcttccaggcagccgcggtgcccaaccacacttgtcggctccagtccccagaactctgcctgccctttgtcctcctgctgccagtaccagccccaccctgttttgagccctgaggaggccttgggctctgctgagtccgacctggcctgtctgtgaagagcaagagagcagcaaggtcttgctctcctaggtagccccctcttccctggtaagaaaaagcaaaaggcatttcccaccctgaacaacgagccttttcacccttctactctagagaagtggactggaggagctgggcccgatttggtagttgaggaaagcacagaggcctcctgtggcctgccagtcatcgagtggcccaacaggggctccatgccagccgaccttgacctcactcagaagtccagagtctagcgtagtgcagcagggcagtagcggtaccaatgcagaactcccaagacccgagctgggaccagtacctgggtccccagcccttcctctgctcccccttttccctcggagttcttcttgaatggcaatgttttgcttttgctcgatgcagacagggggccagaacaccacacatttcactgtctgtctggtccatagctgtggtgtaggggcttagaggcatgggcttgctgtgggtttttaattgatcagttttcatgtgggatcccatctttttaacctctgttcaggaagtccttatctagctgcatatcttcatcatattggtatatccttttctgtgtttacagagatgtctcttatatctaaatctgtccaactgagaagtaccttatcaaagtagcaaatgagacagcagtcttatgcttccagaaacacccacaggcatgtcccatgtgagctgctgccatgaactgtcaagtgtgtgttgtcttgtgtatttcagttattgtccctggcttccttactatggtgtaatcatgaaggagtgaaacatcatagaaactgtctagcacttccttgccagtctttagtgatcaggaaccatagttgacagttccaatcagtagcttaagaaaaaaccgtgtttgtctcttctggaatggttagaagtgagggagtttgccccgttctgtttgtagagtctcatagttggactttctagcatatatgtgtccatttccttatgctgtaaaagcaagtcctgcaaccaaactcccatcagcccaatccctgatccctgatcccttccacctgctctgctgatgacccccccagcttcacttctgactcttccccaggaagggaaggggggtcagaagagagggtgagtcctccagaactcttcctccaaggacagaaggctcctgcccccatagtggcctcgaactcctggcactaccaaaggacacttatccacgagagcgcagcatccgaccaggttgtcactgagaagatgtttattttggtcagttgggtttttatgtattatacttagtcaaatgtaatgtggcttctggaatcattgtccagagctgcttccccgtcacctgggcgtcatctggtcctggtaagaggagtgcgtggcccaccaggcccccctgtcacccatgacagttcattcagggccgatggggcagtcgtggttgggaacacagcatttcaagcgtcactttatttcattcgggccccacctgcagctccctcaaagaggcagttgcccagcctctttcccttccagtttattccagagctgccagtggggcctgaggctccttagggttttctctctatttccccctttcttcctcattccctcgtctttcccaaaggcatcacgagtcagtcgcctttcagcaggcagccttggcggtttatcgccctggcaggcaggggccctgcagctctcatgctgcccctgccttggggtcaggttgacaggaggttggagggaaagccttaagctgcaggattctcaccagctgtgtccggcccagttttggggtgtgacctcaatttcaattttgtctgtacttgaacattatgaagatgggggcctctttcagtgaatttgtgaacagcagaattgaccgacagctttccagtacccatggggctaggtcattaaggccacatccacagtctcccccacccttgttccagttgttagttactacctcctctcctgacaatactgtatgtcgtcgagctccccccaggtctacccctcccggccctgcctgctggtgggcttgtcatagccagtgggattgccggtcttgacagctcagtgagctggagatacttggtcacagccaggcgctagcacagctcccttctgttgatgctgtattcccatatcaaaagacacaggggacacccagaaacgccacatcccccaatccatcagtgccaaactagccaacggccccagcttctcagctcgctggatggcggaagctgctactcgtgagcgccagtgcgggtgcagacaatcttctgttgggtggcatcattccaggcccgaagcatgaacagtgcacctgggacagggagcagccccaaattgtcacctgcttctctgcccagcttttcattgctgtgacagtgatggcgaaagagggtaataaccagacacaaactgccaagttgggtggagaaaggagtttctttagctgacagaatctctgaattttaaatcacttagtaagcggctcaagcccaggagggagcagagggatacgagcggagtcccctgcgcgggaccatctggaattggtttagcccaagtggagcctgacagccagaactctgtgtcccccgtctaaccacagctccttttccagagcattccagtcaggctctctgggctgactgggccaggggaggttacaggtaccagttctttaagaagatctttgggcatatacatttttagcctgtgtcattgccccaaatggattcctgtttcaagttcacacctgcagattctaggacctgtgtcctagacttcagggagtcagctgtttctagagttcctaccatggagtgggtctggaggacctgcccggtgggggggcagagccctgctccctccgggtcttcctactcttctctctgctctgacgggatttgttgattctctccattttggtgtctttctcttttagatattgtatcaatctttagaaaaggcatagtctacttgttataaatcgttaggatactgcctcccccagggtctaaaattacatattagaggggaaaagctgaacactgaagtcagttctcaacaatttagaaggaaaacctagaaaacatttggcagaaaattacatttcgatgtttttgaatgaatacgagcaagcttttacaacagtgctgatctaaaaatacttagcacttggcctgagatgcctggtgagcattacaggcaaggggaatctggaggtagccgacctgaggacatggcttctgaacctgtcttttgggagtggtatggaaggtggagcgttcaccagtgacctggaaggcccagcaccaccctccttcccactcttctcatcttgacagagcctgccccagcgctgacgtgtcaggaaaacacccagggaactaggaaggcacttctgcctgaggggcagcctgccttgcccactcctgctctgctcgcctcggatcagctgagccttctgagctggcctctcactgcctccccaaggccccctgcctgccctgtcaggaggcagaaggaagcaggtgtgagggcagtgcaaggagggagcacaacccccagctcccgctccgggctccgacttgtgcacaggcagagcccagaccctggaggaaatcctacctttgaattcaagaacatttggggaatttggaaatctctttgcccccaaacccccattctgtcctacctttaatcaggtcctgctcagcagtgagagcagatgaggtgaaaaggccaagaggtttggctcctgcccactgatagcccctctccccgcagtgtttgtgtgtcaagtggcaaagctgttcttcctggtgaccctgattatatccagtaacacatagactgtgcgcataggcctgctttgtctcctctatcctgggcttttgttttgctttttagttttgcttttagtttttctgtcccttttatttaacgcaccgactagacacacaaagcagttgaatttttatatatatatctgtatattgcacaattataaactcattttgcttgtggctccacacacacaaaaaaagacctgttaaaattatacctgttgcttaattacaatatttctgataaccatagcataggacaagggaaaataaaaaaagaaaaaaaagaaaaaaaaacgacaaatctgtctgctggtcacttcttctgtccaagcagattcgtggtcttttcctcgcttctttcaagggctttcctgtgccaggtgaaggaggctccaggcagcacccaggttttgcactcttgtttctcccgtgcttgtgaaagaggtcccaaggttctgggtgcaggagcgctcccttgacctgctgaagtccggaacgtagtcggcacagcctggtcgccttccacctctgggagctggagtccactggggtggcctgactcccccagtccccttcccgtgacctggtcagggtgagcccatgtggagtcagcctcgcaggcctccctgccagtagggtccgagtgtgtttcatccttcccactctgtcgagcctgggggctggagcggagacgggaggcctggcctgtctcggaacctgtgagctgcaccaggtagaacgccagggaccccagaatcatgtgcgtcagtccaaggggtcccctccaggagtagtgaagactccagaaatgtccctttcttctcccccatcctacgagtaattgcatttgcttttgtaattcttaatgagcaatatctgctagagagtttagctgtaacagttctttttgatcatctttttttaataattagaaacaccaaaaaaatccagaaacttgttcttccaaagcagagagcattataatcaccagggccaaaagcttccctccctgctgtcattgcttcttctgaggcctgaatccaaaagaaaaacagccataggccctttcagtggccgggctacccgtgagcccttcggaggaccagggctggggcagcctctgggcccacatccggggccagctccggcgtgtgttcagtgttagcagtgggtcatgatgctctttcccacccagcctgggataggggcagaggaggcgaggaggccgttgccgctgatgtttggccgtgaacaggtgggtgtctgcgtgcgtccacgtgcgtgttttctgactgacatgaaatcgacgcccgagttagcctcacccggtgacctctagccctgcccggatggagcggggcccacccggttcagtgtttctggggagctggacagtggagtgcaaaaggcttgcagaacttgaagcctgctccttcccttgctaccacggcctcctttccgtttgatttgtcactgcttcaatcaataacagccgctccagagtcagtagtcaatgaatatatgaccaaatatcaccaggactgttactcaatgtgtgccgagcccttgcccatgctgggctcccgtgtatctggacactgtaacgtgtgctgtgtttgctccccttccccttccttctttgccctttacttgtctttctggggtttttctgtttgggtttggtttggtttttatttctccttttgtgttccaaacatgaggttctctctactggtcctcttaactgtggtgttgaggcttatatttgtgtaatttttggtgggtgaaaggaattttgctaagtaaatctcttctgtgtttgaactgaagtctgtattgtaactatgtttaaagtaattgttccagagacaaatatttctagacactttttctttacaaacaaaagcattcggagggagggggatggtgactgagatgagaggggagagctgaacagatgacccctgcccagatcagccagaagccacccaaagcagtggagcccaggagtcccactccaagccagcaagccgaatagctgatgtgttgccactttccaagtcactgcaaaaccaggttttgttccgcccagtggattcttgttttgcttcccctccccccgagattattaccaccatcccgtgcttttaaggaaaggcaagattgatgtttccttgaggggagccaggaggggatgtgtgtgtgcagagctgaagagctggggagaatggggctgggcccacccaagcaggaggctgggacgctctgctgtgggcacaggtcaggctaatgttggcagatgcagctcttcctggacaggccaggtggtgggcattctctctccaaggtgtgccccgtgggcattactgtttaagacacttccgtcacatcccaccccatcctccagggctcaacactgtgacatctctattccccaccctccccttcccagggcaataaaatgaccatggagggggcttgcactctcttggctgtcacccgatcgccagcaaaacttagatgtgagaaaaccccttcccattccatggcgaaaacatctccttagaaaagccattaccctcattaggcatggttttgggctcccaaaacacctgacagcccctccctcctctgagaggcggagagtgctgactgtagtgaccattgcatgccgggtgcagcatctggaagagctaggcagggtgtctgccccctcctgagttgaagtcatgctcccctgtgccagcccagaggccgagagctatggacagcattgccagtaacacaggccaccctgtgcagaagggagctggctccagcctggaaacctgtctgaggttgggagaggtgcacttggggcacagggagaggccgggacacacttagctggagatgtctctaaaagccctgtatcgtattcaccttcagtttttgtgttttgggacaattactttagaaaataagtaggtcgttttaaaaacaaaaattattgattgcttttttgtagtgttcagaaaaaaggttctttgtgtatagccaaatgactgaaagcactgatatatttaaaaacaaaaggcaatttattaaggaaatttgtaccatttcagtaaacctgtctgaatgtacctgtatacgtttcaaaaacaccccccccccactgaatccctgtaacctatttattatataaagagtttgccttataaattt

SEQ ID NO: 3 - DNA, 20 bp, synthetic construct
  source 1..20: mol_type = other DNA
tatttgatcaatccccaggg

SEQ ID NO: 4 - DNA, 20 bp, synthetic construct
  source 1..20: mol_type = other DNA
ctccctctcccagttaccgt

SEQ ID NO: 5 - DNA, 22 bp, synthetic construct
  source 1..22: mol_type = other DNA
aggagagactggaagaaaagtc

SEQ ID NO: 6 - DNA, 20 bp, synthetic construct
  source 1..20: mol_type = other DNA
cttgaggggtttgtccttga

SEQ ID NO: 7 - DNA, 23 bp, synthetic construct
  source 1..23: mol_type = other DNA
ctcaccagttcctgctttgatgt

SEQ ID NO: 8 - DNA, 22 bp, synthetic construct
  source 1..22: mol_type = other DNA
aggagagactggaggaaaagtc

SEQ ID NO: 9 - DNA, 25 bp, synthetic construct
  source 1..25: mol_type = other DNA
cttaaacttcagtggcttgtctctg

SEQ ID NO: 10 - DNA, 21 bp, synthetic construct
  source 1..21: mol_type = other DNA
cgggggacataaaagttattg

SEQ ID NO: 11 - DNA, 22 bp, synthetic construct
  source 1..22: mol_type = other DNA
tgcattgttttaccagtgtcaa

SEQ ID NO: 12 - DNA, 25 bp, synthetic construct
  source 1..25: mol_type = other DNA
tgaaggagtcttctatccgatctgt

SEQ ID NO: 13 - DNA, 21 bp, synthetic construct
  source 1..21: mol_type = other DNA
cacttccttgacctcgatgct

SEQ ID NO: 14 - DNA, 26 bp, synthetic construct
  source 1..26: mol_type = other DNA
agaccgtactccccatcaagaagcgc

SEQ ID NO: 15 - DNA, 20 bp, synthetic construct
  source 1..20: mol_type = other DNA
gtgcgcgcgagcccgaaatc

SEQ ID NO: 16 - DNA, 20 bp, synthetic construct
  source 1..20: mol_type = other DNA
ctctccgagaggagggagcg

SEQ ID NO: 17 - DNA, 20 bp, synthetic construct
  source 1..20: mol_type = other DNA
gccattttccggacggcttt

SEQ ID NO: 18 - DNA, 20 bp, synthetic construct
  source 1..20: mol_type = other DNA
tctctcctcctcgcctcctc

SEQ ID NO: 19 - DNA, 20 bp, synthetic construct
  source 1..20: mol_type = other DNA
acccccgccccccggcaagg

SEQ ID NO: 20 - DNA, 20 bp, synthetic construct
  source 1..20: mol_type = other DNA
agagacctcaacttgtcacg

SEQ ID NO: 21 - DNA, 20 bp, synthetic construct
  source 1..20: mol_type = other DNA
cattaagataaccatcattt

SEQ ID NO: 22 - DNA, 20 bp, synthetic construct
  source 1..20: mol_type = other DNA
ggaactggtgagtctgtatt

SEQ ID NO: 23 - DNA, 20 bp, synthetic construct
  source 1..20: mol_type = other DNA
gaagcaaggtgtattctggg

SEQ ID NO: 24 - DNA, 20 bp, synthetic construct
  source 1..20: mol_type = other DNA
ctaccatggaatcctgttgg

SEQ ID NO: 25 - DNA, 20 bp, synthetic construct
  source 1..20: mol_type = other DNA
ttttctataaatccatgtat

SEQ ID NO: 26 - DNA, 20 bp, synthetic construct
  source 1..20: mol_type = other DNA
tagccccactcccggataag

SEQ ID NO: 27 - DNA, 20 bp, synthetic construct
  source 1..20: mol_type = other DNA
actcaagcccaaggagttca

SEQ ID NO: 28 - DNA, 20 bp, synthetic construct
  source 1..20: mol_type = other DNA
gctttaatgctttattttta

SEQ ID NO: 29 - DNA, 20 bp, synthetic construct
  source 1..20: mol_type = other DNA
tgccaacagcaggcccagcg

SEQ ID NO: 30 - DNA, 20 bp, synthetic construct
  source 1..20: mol_type = other DNA
gatatcagtgaggaagttgt

SEQ ID NO: 31 - DNA, 20 bp, synthetic construct
  source 1..20: mol_type = other DNA
cgtgccatggaagtccttcc

SEQ ID NO: 32 - DNA, 20 bp, synthetic construct
  source 1..20: mol_type = other DNA
ggtgagctgatgctatatga

SEQ ID NO: 33 - DNA, 20 bp, synthetic construct
  source 1..20: mol_type = other DNA
aggcggcagtggcttacgcc

SEQ ID NO: 34 - DNA, 20 bp, synthetic construct
  source 1..20: mol_type = other DNA
agccccttaattttgttctc

SEQ ID NO: 35 - DNA, 20 bp, synthetic construct
  source 1..20: mol_type = other DNA
tggcggctcaagaaccagcc

SEQ ID NO: 36 - DNA, 20 bp, synthetic construct
  source 1..20: mol_type = other DNA
caaatattagaatagactca

SEQ ID NO: 37 - DNA, 20 bp, synthetic construct
  source 1..20: mol_type = other DNA
tgggactcagattctatagg

SEQ ID NO: 38 - DNA, 20 bp, synthetic construct
  source 1..20: mol_type = other DNA
gtcctggaacgacaggcttg

SEQ ID NO: 39 - DNA, 20 bp, synthetic construct
  source 1..20: mol_type = other DNA
ccaaatttataacttaagaa

SEQ ID NO: 40 - DNA, 20 bp, synthetic construct
  source 1..20: mol_type = other DNA
ggtgatgtgtattttactac

SEQ ID NO: 41 - DNA, 20 bp, synthetic construct
  source 1..20: mol_type = other DNA
tggtgggacaaaaattgtgg

SEQ ID NO: 42 - DNA, 20 bp, synthetic construct
  source 1..20: mol_type = other DNA
aaataagcatctggcatttg

SEQ ID NO: 43 - DNA, 20 bp, synthetic construct
  source 1..20: mol_type = other DNA
tacattgaaaaacagccaga

SEQ ID NO: 44 - DNA, 20 bp, synthetic construct
  source 1..20: mol_type = other DNA
ggatccatgcgagagaagca

SEQ ID NO: 45 - DNA, 20 bp, synthetic construct
  source 1..20: mol_type = other DNA
tataatatcattcagcctca

SEQ ID NO: 46 - DNA, 20 bp, synthetic construct
  source 1..20: mol_type = other DNA
cagcaggaagagtccagaga

SEQ ID NO: 47 - DNA, 20 bp, synthetic construct
  source 1..20: mol_type = other DNA
agaaacctgccaggtgtggt

SEQ ID NO: 48 - DNA, 20 bp, synthetic construct
  source 1..20: mol_type = other DNA
ccaggtgtggcccagggtgg

SEQ ID NO: 49 - DNA, 20 bp, synthetic construct
  source 1..20: mol_type = other DNA
ggcatcctacaacccacaga

SEQ ID NO: 50 - DNA, 20 bp, synthetic construct
  source 1..20: mol_type = other DNA
tgacttttcttccctgagcc

SEQ ID NO: 51 - DNA, 20 bp, synthetic construct
  source 1..20: mol_type = other DNA
gggtttgtccttgaggccct

SEQ ID NO: 52 - DNA, 20 bp, synthetic construct
  source 1..20: mol_type = other DNA
ctcttctttcttatctttct

SEQ ID NO: 53 - DNA, 20 bp, synthetic construct
  source 1..20: mol_type = other DNA
cttgccctctttctcttctt

SEQ ID NO: 54 - DNA, 20 bp, synthetic construct
  source 1..20: mol_type = other DNA
tggctgcacgggctcatgct

SEQ ID NO: 55 - DNA, 20 bp, synthetic construct
  source 1..20: mol_type = other DNA
gtggtgggctgatggctgca

SEQ ID NO: 56 - DNA, 20 bp, synthetic construct
  source 1..20: mol_type = other DNA
ctgctttgcctgcctctgcg

SEQ ID NO: 57 - DNA, 20 bp, synthetic construct
  source 1..20: mol_type = other DNA
aagcttccggcacagccggg

SEQ ID NO: 58 - DNA, 20 bp, synthetic construct
  source 1..20: mol_type = other DNA
ggtcacggatgatggagcgc

SEQ ID NO: 59 - DNA, 20 bp, synthetic construct
  source 1..20: mol_type = other DNA
ttccgtgtccagccttcagg

SEQ ID NO: 60 - DNA, 20 bp, synthetic construct
  source 1..20: mol_type = other DNA
cagcagagcggccagatttc

SEQ ID NO: 61 - DNA, 20 bp, synthetic construct
  source 1..20: mol_type = other DNA
tgtccctgccctccctgccc

SEQ ID NO: 62 - DNA, 20 bp, synthetic construct
  source 1..20: mol_type = other DNA
gcgaaaggcttttccctggg

SEQ ID NO: 63 - DNA, 20 bp, synthetic construct
  source 1..20: mol_type = other DNA
gaagtacgcaatcaactcca

SEQ ID NO: 64 - DNA, 20 bp, synthetic construct
  source 1..20: mol_type = other DNA
gggatgtgtcgcctaccttt

SEQ ID NO: 65 - DNA, 20 bp, synthetic construct
  source 1..20: mol_type = other DNA
cgtgaagtcaaaatcattag

SEQ ID NO: 66 - DNA, 20 bp, synthetic construct
  source 1..20: mol_type = other DNA
ttaggtggtttctgctctcg

SEQ ID NO: 67 - DNA, 20 bp, synthetic construct
  source 1..20: mol_type = other DNA
cggcctctgccagttcctgg

SEQ ID NO: 68 - DNA, 20 bp, synthetic construct
  source 1..20: mol_type = other DNA
acccttttcacctgcacacc

SEQ ID NO: 69 - DNA, 20 bp, synthetic construct
  source 1..20: mol_type = other DNA
aaggagcttcccaggacttt

SEQ ID NO: 70 - DNA, 20 bp, synthetic construct
  source 1..20: mol_type = other DNA
tggcgaagtttgaaaaggca

SEQ ID NO: 71 - DNA, 20 bp, synthetic construct
  source 1..20: mol_type = other DNA
agccttgccccctggcgaag

SEQ ID NO: 72 - DNA, 20 bp, synthetic construct
  source 1..20: mol_type = other DNA
tggatgtggtggccccaccc

SEQ ID NO: 73 - DNA, 20 bp, synthetic construct
  source 1..20: mol_type = other DNA
gcttttcgcttcctgccggg

SEQ ID NO: 74 - DNA, 20 bp, synthetic construct
  source 1..20: mol_type = other DNA
gtttcttgggaatggcctga

SEQ ID NO: 75 - DNA, 20 bp, synthetic construct
  source 1..20: mol_type = other DNA
ggctgccaccacactccccg

SEQ ID NO: 76 - DNA, 20 bp, synthetic construct
  source 1..20: mol_type = other DNA
ttcacggctttctttttggc

SEQ ID NO: 77 - DNA, 20 bp, synthetic construct
  source 1..20: mol_type = other DNA
ctcctgcacagatcggatag

SEQ ID NO: 78 - DNA, 20 bp, synthetic construct
  source 1..20: mol_type = other DNA
tctcccgggtcttgcgcttc

SEQ ID NO: 79 - DNA, 20 bp, synthetic construct
  source 1..20: mol_type = other DNA
cttcaccacttccttgacct

SEQ ID NO: 80 - DNA, 20 bp, synthetic construct
  source 1..20: mol_type = other DNA
tcagtcctttcccgctcttc

SEQ ID NO: 81 - DNA, 20 bp, synthetic construct
  source 1..20: mol_type = other DNA
cttgcttttccgcccagggc

SEQ ID NO: 82 - DNA, 20 bp, synthetic construct
  source 1..20: mol_type = other DNA
ggtgatggtggtggtgctcc

SEQ ID NO: 83 - DNA, 20 bp, synthetic construct
  source 1..20: mol_type = other DNA
gctgctgctcaagtcctggg

SEQ ID NO: 84 - DNA, 20 bp, synthetic construct
  source 1..20: mol_type = other DNA
ctccagtgagcctcctctgg

SEQ ID NO: 85 - DNA, 20 bp, synthetic construct
  source 1..20: mol_type = other DNA
aaccgcgggctgagtcttag

SEQ ID NO: 86 - DNA, 20 bp, synthetic construct
  source 1..20: mol_type = other DNA
tggcggcggtggcaaccgcg

SEQ ID NO: 87 - DNA, 20 bp, synthetic construct
  source 1..20: mol_type = other DNA
ttttctgcggccgtggcggc

SEQ ID NO: 88 - DNA, 20 bp, synthetic construct
  source 1..20: mol_type = other DNA
ctctccctcccctcggtgtt

SEQ ID NO: 89 - DNA, 20 bp, synthetic construct
  source 1..20: mol_type = other DNA
cttggcatggaggatgaaac

SEQ ID NO: 90 - DNA, 20 bp, synthetic construct
  source 1..20: mol_type = other DNA
tccggctgtccacaggctcc

SEQ ID NO: 91 - DNA, 20 bp, synthetic construct
  source 1..20: mol_type = other DNA
aatccgctccgtgtaaagtc

SEQ ID NO: 92 - DNA, 20 bp, synthetic construct
  source 1..20: mol_type = other DNA
cagctgcctttattcttgtt

SEQ ID NO: 93 - DNA, 20 bp, synthetic construct
  source 1..20: mol_type = other DNA
gtcagagccctacccataag

SEQ ID NO: 94 - DNA, 20 bp, synthetic construct
  source 1..20: mol_type = other DNA
agcgcgcgcgccgccgacgc

SEQ ID NO: 95 - DNA, 20 bp, synthetic construct
  source 1..20: mol_type = other DNA
cttttaccacagccctctct

SEQ ID NO: 96 - DNA, 20 bp, synthetic construct
  source 1..20: mol_type = other DNA
ccgctcggcgcggcggcggc

SEQ ID NO: 97 - DNA, 20 bp, synthetic construct
  source 1..20: mol_type = other DNA
tcagtttgggtgattcggtc

SEQ ID NO: 98 - DNA, 20 bp, synthetic construct
  source 1..20: mol_type = other DNA
cagcacagcgggaacacatt

SEQ ID NO: 99 - DNA, 20 bp, synthetic construct
  source 1..20: mol_type = other DNA
tatttttatggagcagtctc

SEQ ID NO: 100 - DNA, 20 bp, synthetic construct
  source 1..20: mol_type = other DNA
atgtcacatcaaagcaggaa

SEQ ID NO: 101 - DNA, 20 bp, synthetic construct
  source 1..20: mol_type = other DNA
ttggagctggtctacagaag

SEQ ID NO: 102 - DNA, 20 bp, synthetic construct
  source 1..20: mol_type = other DNA
agccctaacatcccagctac

SEQ ID NO: 103 - DNA, 20 bp, synthetic construct
  source 1..20: mol_type = other DNA
cacactgacctttcagggct

SEQ ID NO: 104 - DNA, 20 bp, synthetic construct
  source 1..20: mol_type = other DNA
taaaaaaggatttcctaagt

SEQ ID NO: 105 - DNA, 20 bp, synthetic construct
  source 1..20: mol_type = other DNA
gtacacacacgctttttttt

SEQ ID NO: 106 - DNA, 20 bp, synthetic construct
  source 1..20: mol_type = other DNA
gaaagccgagcctggccggg

SEQ ID NO: 107 - DNA, 20 bp, synthetic construct
  source 1..20: mol_type = other DNA
gaagaaaatgtggatttttt

SEQ ID NO: 108 - DNA, 20 bp, synthetic construct
  source 1..20: mol_type = other DNA
cgagaatgagactccgtatc

SEQ ID NO: 109 - DNA, 20 bp, synthetic construct
  source 1..20: mol_type = other DNA
aaacccaaaccaccttaccc

SEQ ID NO: 110 - DNA, 20 bp, synthetic construct
  source 1..20: mol_type = other DNA
aaaataaagtcaggaggctg

SEQ ID NO: 111 - DNA, 20 bp, synthetic construct
  source 1..20: mol_type = other DNA
aaaaatggagggcacagtgg

SEQ ID NO: 112 - DNA, 20 bp, synthetic construct
  source 1..20: mol_type = other DNA
ggtttttctcctttattatc

SEQ ID NO: 113 - DNA, 20 bp, synthetic construct
  source 1..20: mol_type = other DNA
tatgttggcctagaactcct

SEQ ID NO: 114 - DNA, 20 bp, synthetic construct
  source 1..20: mol_type = other DNA
tgctctcatattcacccacg

SEQ ID NO: 115 - DNA, 20 bp, synthetic construct
  source 1..20: mol_type = other DNA
gtgcagagactcaagggagg

SEQ ID NO: 116 - DNA, 20 bp, synthetic construct
  source 1..20: mol_type = other DNA
gctaagcctcctggtgaacc

SEQ ID NO: 117 - DNA, 20 bp, synthetic construct
  source 1..20: mol_type = other DNA
gtatgaacatcagctgacgc

SEQ ID NO: 118 - DNA, 20 bp, synthetic construct
  source 1..20: mol_type = other DNA
aggcgcgctggtgcaagcct

SEQ ID NO: 119 - DNA, 20 bp, synthetic construct
  source 1..20: mol_type = other DNA
cagccactctttttttttga

SEQ ID NO: 120 - DNA, 20 bp, synthetic construct
  source 1..20: mol_type = other DNA
gtacctgggaggaactacaa

SEQ ID NO: 121 - DNA, 20 bp, synthetic construct
  source 1..20: mol_type = other DNA
agggcgagagatccaggact

SEQ ID NO: 122 - DNA, 20 bp, synthetic construct
  source 1..20: mol_type = other DNA
ggattagggaattagatgca

SEQ ID NO: 123 - DNA, 20 bp, synthetic construct
  source 1..20: mol_type = other DNA
ggaaagcctgtcttttaaaa

SEQ ID NO: 124 - DNA, 20 bp, synthetic construct
  source 1..20: mol_type = other DNA
ccagatggtgtttccaattc

SEQ ID NO: 125 - DNA, 20 bp, synthetic construct
  source 1..20: mol_type = other DNA
acttctagaccgggcgcagt

SEQ ID NO: 126 - DNA, 20 bp, synthetic construct
  source 1..20: mol_type = other DNA
gtacaatgaatgaacttttt

SEQ ID NO: 127 - DNA, 20 bp, synthetic construct
  source 1..20: mol_type = other DNA
caaacatatctactgcattc

SEQ ID NO: 128 - DNA, 20 bp, synthetic construct
  source 1..20: mol_type = other DNA
acaggtaaccccatctaggc

SEQ ID NO: 129 - DNA, 20 bp, synthetic construct
  source 1..20: mol_type = other DNA
ggaggtcctggtcttctgac

SEQ ID NO: 130 - DNA, 20 bp, synthetic construct
  source 1..20: mol_type = other DNA
ttatctttcttcaccttttt

SEQ ID NO: 131 - DNA, 20 bp, synthetic construct
  source 1..20: mol_type = other DNA
ctctttctcttctttcttat

SEQ ID NO: 132 - DNA, 20 bp, synthetic construct
  source 1..20: mol_type = other DNA
cacgggctcatgcttgccct

SEQ ID NO: 133 - DNA, 20 bp, synthetic construct
  source 1..20: mol_type = other DNA
ggctgatggctgcacgggct

SEQ ID NO: 134 - DNA, 20 bp, synthetic construct
  source 1..20: mol_type = other DNA
tgcgggctcagcagagtggt

SEQ ID NO: 135 - DNA, 20 bp, synthetic construct
  source 1..20: mol_type = other DNA
gacccttctgatgtctctgc

SEQ ID NO: 136 - DNA, 20 bp, synthetic construct
  source 1..20: mol_type = other DNA
aggcagaagcttccggcaca

SEQ ID NO: 137 - DNA, 20 bp, synthetic construct
  source 1..20: mol_type = other DNA
tcatacatgggtccccggtc

SEQ ID NO: 138 - DNA, 20 bp, synthetic construct
  source 1..20: mol_type = other DNA
tttcctttgcttaagcttcc

SEQ ID NO: 139 - DNA, 20 bp, synthetic construct
  source 1..20: mol_type = other DNA
tacacatcatacttcccagc

SEQ ID NO: 140 - DNA, 20 bp, synthetic construct
  source 1..20: mol_type = other DNA
tcaactccactttagagcga

SEQ ID NO: 141 - DNA, 20 bp, synthetic construct
  source 1..20: mol_type = other DNA
gcctaccttttcgaagtacg

SEQ ID NO: 142 - DNA, 20 bp, synthetic construct
  source 1..20: mol_type = other DNA
ggtccagggatgtgtcgcct

SEQ ID NO: 143 - DNA, 20 bp, synthetic construct
  source 1..20: mol_type = other DNA
tccctctcccagttaccgtg

SEQ ID NO: 144 - DNA, 20 bp, synthetic construct
  source 1..20: mol_type = other DNA
tggagctttgggagatttgg

SEQ ID NO: 145 - DNA, 20 bp, synthetic construct
  source 1..20: mol_type = other DNA
cgtggccgccttgggtctcg

SEQ ID NO: 146 - DNA, 20 bp, synthetic construct
  source 1..20: mol_type = other DNA
aggacttttctccaggaccc

SEQ ID NO: 147 - DNA, 20 bp, synthetic construct
  source 1..20: mol_type = other DNA
aggcatcttgacaaggagct

SEQ ID NO: 148 - DNA, 20 bp, synthetic construct
  source 1..20: mol_type = other DNA
gccccctggcgaagtttgaa

SEQ ID NO: 149 - DNA, 20 bp, synthetic construct
  source 1..20: mol_type = other DNA
ccccacccccctcagccttg

SEQ ID NO: 150 - DNA, 20 bp, synthetic construct
  source 1..20: mol_type = other DNA
ccatgacctgggtggatgtg

SEQ ID NO: 151 - DNA, 20 bp, synthetic construct
  source 1..20: mol_type = other DNA
ctgagggtcggcctcagctt

SEQ ID NO: 152 - DNA, 20 bp, synthetic construct
  source 1..20: mol_type = other DNA
cccggctttcggccccgttt

SEQ ID NO: 153 - DNA, 20 bp, synthetic construct
  source 1..20: mol_type = other DNA
tggcctcggcggcagcggct

SEQ ID NO: 154 - DNA, 20 bp, synthetic construct
  source 1..20: mol_type = other DNA
tcggatagaagactccttca

SEQ ID NO: 155 - DNA, 20 bp, synthetic construct
  source 1..20: mol_type = other DNA
tacggtctcctgcacagatc

SEQ ID NO: 156 - DNA, 20 bp, synthetic construct
  source 1..20: mol_type = other DNA
acctcgatgctgaccgtctc

SEQ ID NO: 157 - DNA, 20 bp, synthetic construct
  source 1..20: mol_type = other DNA
cttctcaccgagggtggaca

SEQ ID NO: 158 - DNA, 20 bp, synthetic construct
  source 1..20: mol_type = other DNA
gggctcttacaggtcttcag

SEQ ID NO: 159 - DNA, 20 bp, synthetic construct
  source 1..20: mol_type = other DNA
ctgctgctgcgccccttggg

SEQ ID NO: 160 - DNA, 20 bp, synthetic construct
  source 1..20: mol_type = other DNA
tcgggctcaggtggaggtgg

SEQ ID NO: 161 - DNA, 20 bp, synthetic construct
  source 1..20: mol_type = other DNA
ctgggcatcttctcctcttt

SEQ ID NO: 162 - DNA, 20 bp, synthetic construct
  source 1..20: mol_type = other DNA
gtcttagctggctccttggg

SEQ ID NO: 163 - DNA, 20 bp, synthetic construct
  source 1..20: mol_type = other DNA
ggtggcaaccgcgggctgag

SEQ ID NO: 164 - DNA, 20 bp, synthetic construct
  source 1..20: mol_type = other DNA
cggccgtggcggcggtggca

SEQ ID NO: 165 - DNA, 20 bp, synthetic construct
  source 1..20: mol_type = other DNA
tgtttgtacttttctgcggc

SEQ ID NO: 166 - DNA, 20 bp, synthetic construct
  source 1..20: mol_type = other DNA
aaacaatgtctttgcgctct

SEQ ID NO: 167 - DNA, 20 bp, synthetic construct
  source 1..20: mol_type = other DNA
ctcctctctgtttggccttg

SEQ ID NO: 168 - DNA, 20 bp, synthetic construct
  source 1..20: mol_type = other DNA
agtcagctaactctctcggt

SEQ ID NO: 169 - DNA, 20 bp, synthetic construct
  source 1..20: mol_type = other DNA
tgttggtttgctttgcaatc

SEQ ID NO: 170 - DNA, 20 bp, synthetic construct
  source 1..20: mol_type = other DNA
taaggagaagagacaacagc

SEQ ID NO: 171 - DNA, 20 bp, synthetic construct
  source 1..20: mol_type = other DNA
ttaatcgggaagctttgtca

SEQ ID NO: 172 - DNA, 20 bp, synthetic construct
  source 1..20: mol_type = other DNA
gaggagggagcgcgcgcgcc

SEQ ID NO: 173 - DNA, 20 bp, synthetic construct
  source 1..20: mol_type = other DNA
ccggacggcttttaccacag

SEQ ID NO: 174 - DNA, 20 bp, synthetic construct
  source 1..20: mol_type = other DNA
ctcctcctccgctcggcgcg

SEQ ID NO: 175 - DNA, 20 bp, synthetic construct
  source 1..20: mol_type = other DNA
atgcttcatttttacagtat

SEQ ID NO: 176 - DNA, 20 bp, synthetic construct
  source 1..20: mol_type = other DNA
gagccagaggctgggtgcgg

SEQ ID NO: 177 - DNA, 20 bp, synthetic construct
  source 1..20: mol_type = other DNA
tgagtctgtatttttatgga

SEQ ID NO: 178 - DNA, 20 bp, synthetic construct
  source 1..20: mol_type = other DNA
ggagtcacatgtcacatcaa

SEQ ID NO: 179 - DNA, 20 bp, synthetic construct
  source 1..20: mol_type = other DNA
gaatcctgttggagctggtc

SEQ ID NO: 180 - DNA, 20 bp, synthetic construct
  source 1..20: mol_type = other DNA
cttccctgagccctaacatc

SEQ ID NO: 181 - DNA, 20 bp, synthetic construct
  source 1..20: mol_type = other DNA
cccacagcagtaaaagagaa

SEQ ID NO: 182 - DNA, 20 bp, synthetic construct
  source 1..20: mol_type = other DNA
accccagtagttgagattac

SEQ ID NO: 183 - DNA, 20 bp, synthetic construct
  source 1..20: mol_type = other DNA
atagtagttgccagagggtg

SEQ ID NO: 184 - DNA, 20 bp, synthetic construct
  source 1..20: mol_type = other DNA
ggcttctattgtaaaactat

SEQ ID NO: 185 - DNA, 20 bp, synthetic construct
  source 1..20: mol_type = other DNA
actggtttttaagagatggg

SEQ ID NO: 186 - DNA, 20 bp, synthetic construct
  source 1..20: mol_type = other DNA
taaaatctatgggaataaaa

SEQ ID NO: 187 - DNA, 20 bp, synthetic construct
  source 1..20: mol_type = other DNA
gaaatgtgggcttggcatgg

SEQ ID NO: 188 - DNA, 20 bp, synthetic construct
  source 1..20: mol_type = other DNA
aacatggtttagtagaaacc

SEQ ID NO: 189 - DNA, 20 bp, synthetic construct
  source 1..20: mol_type = other DNA
ggtattataattttgtaatt

SEQ ID NO: 190 - DNA, 20 bp, synthetic construct
  source 1..20: mol_type = other DNA
caacattccatttatttagg

SEQ ID NO: 191 - DNA, 20 bp, synthetic construct
  source 1..20: mol_type = other DNA
attttcaccctttaaaaatc

SEQ ID NO: 192 - DNA, 20 bp, synthetic construct
  source 1..20: mol_type = other DNA
taatacagtgacaagcatcc

SEQ ID NO: 193 - DNA, 20 bp, synthetic construct
  source 1..20: mol_type = other DNA
tccatcttgcaggtggagta

SEQ ID NO: 194 - DNA, 20 bp, synthetic construct
  source 1..20: mol_type = other DNA
gaagccaaaaaagcaacaaa

SEQ ID NO: 195 - DNA, 20 bp, synthetic construct
  source 1..20: mol_type = other DNA
ccaagacaaggaaaaacggg

SEQ ID NO: 196 - DNA, 20 bp, synthetic construct
  source 1..20: mol_type = other DNA
ctagctatcagctgggcatg

SEQ ID NO: 197 - DNA, 20 bp, synthetic construct
  source 1..20: mol_type = other DNA
tgccttgttgggtagtacag

SEQ ID NO: 198 - DNA, 20 bp, synthetic construct
  source 1..20: mol_type = other DNA
gctaagttagaactccgtgg

SEQ ID NO: 199 - DNA, 20 bp, synthetic construct
  source 1..20: mol_type = other DNA
acacgcctgtaatcctgcat

SEQ ID NO: 200 - DNA, 20 bp, synthetic construct
  source 1..20: mol_type = other DNA
caactggaggccgggcgcga

SEQ ID NO: 201 - DNA, 20 bp, synthetic construct
  source 1..20: mol_type = other DNA
agcccacacagctgtctcag

SEQ ID NO: 202 - DNA, 20 bp, synthetic construct
  source 1..20: mol_type = other DNA
ttcctcatgaatgtgacctg

SEQ ID NO: 203 - DNA, 20 bp, synthetic construct
  source 1..20: mol_type = other DNA
gaggaacttgtctgagatca

SEQ ID NO: 204 - DNA, 20 bp, synthetic construct
  source 1..20: mol_type = other DNA
cagctactcgctagaaaggg

SEQ ID NO: 205 - DNA, 20 bp, synthetic construct
  source 1..20: mol_type = other DNA
ctccccataaaggagggagg

SEQ ID NO: 206 - DNA, 20 bp, synthetic construct
  source 1..20: mol_type = other DNA
ccatcatacactcagatctt

SEQ ID NO: 207 - DNA, 20 bp, synthetic construct
  source 1..20: mol_type = other DNA
ttgaggccctggaggtcctg

SEQ ID NO: 208 - DNA, 20 bp, synthetic construct
  source 1..20: mol_type = other DNA
ttctttcttatctttcttca

SEQ ID NO: 209 - DNA, 20 bp, synthetic construct
  source 1..20: mol_type = other DNA
gccctctttctcttctttct

SEQ ID NO: 210 - DNA, 20 bp, synthetic construct
  source 1..20: mol_type = other DNA
ctgcacgggctcatgcttgc

SEQ ID NO: 211 - DNA, 20 bp, synthetic construct
  source 1..20: mol_type = other DNA
gtgggctgatggctgcacgg

SEQ ID NO: 212 - DNA, 20 bp, synthetic construct
  source 1..20: mol_type = other DNA
cctgcctctgcgggctcagc

SEQ ID NO: 213 - DNA, 20 bp, synthetic construct
  source 1..20: mol_type = other DNA
cggagcctgacccttctgat

SEQ ID NO: 214 - DNA, 20 bp, synthetic construct
  source 1..20: mol_type = other DNA
gggaggcagaagcttccggc

SEQ ID NO: 215 - DNA, 20 bp, synthetic construct
  source 1..20: mol_type = other DNA
ccagccttcaggcagggtgg

SEQ ID NO: 216 - DNA, 20 bp, synthetic construct
  source 1..20: mol_type = other DNA
cggccagatttcctttgctt

SEQ ID NO: 217 - DNA, 20 bp, synthetic construct
  source 1..20: mol_type = other DNA
tgatcaaatacacatcatac

SEQ ID NO: 218 - DNA, 20 bp, synthetic construct
  source 1..20: mol_type = other DNA
gtacgcaatcaactccactt

SEQ ID NO: 219 - DNA, 20 bp, synthetic construct
  source 1..20: mol_type = other DNA
tgtgtcgcctaccttttcga

SEQ ID NO: 220 - DNA, 20 bp, synthetic construct
  source 1..20: mol_type = other DNA
caaaatcattagggtccagg

SEQ ID NO: 221 - DNA, 20 bp, synthetic construct
  source 1..20: mol_type = other DNA
tttctgctctcgccgggagg

SEQ ID NO: 222 - DNA, 20 bp, synthetic construct
  source 1..20: mol_type = other DNA
ccagttcctggagctttggg

SEQ ID NO: 223 - DNA, 20 bp, synthetic construct
  source 1..20: mol_type = other DNA
cacctgcacaccctctgacg

SEQ ID NO: 224 - DNA, 20 bp, synthetic construct
  source 1..20: mol_type = other DNA
gagcttcccaggacttttct

SEQ ID NO: 225 - DNA, 20 bp, synthetic construct
  source 1..20: mol_type = other DNA
gtttgaaaaggcatcttgac

SEQ ID NO: 226 - DNA, 20 bp, synthetic construct
  source 1..20: mol_type = other DNA
cttgccccctggcgaagttt

SEQ ID NO: 227 - DNA, 20 bp, synthetic construct
  source 1..20: mol_type = other DNA
tgtggtggccccacccccct

SEQ ID NO: 228 - DNA, 20 bp, synthetic construct
  source 1..20: mol_type = other DNA
tttgatcaccatgacctggg

SEQ ID NO: 229 - DNA, 20 bp, synthetic construct
  source 1..20: mol_type = other DNA
ggaatggcctgagggtcggc

SEQ ID NO: 230 - DNA, 20 bp, synthetic construct
  source 1..20: mol_type = other DNA
ccacactccccggctttcgg

SEQ ID NO: 231 - DNA, 20 bp, synthetic construct
  source 1..20: mol_type = other DNA
tttctttttggcctcggcgg

SEQ ID NO: 232 - DNA, 20 bp, synthetic construct
  source 1..20: mol_type = other DNA
ctgcacagatcggatagaag

SEQ ID NO: 233 - DNA, 20 bp, synthetic construct
  source 1..20: mol_type = other DNA
gtcttgcgcttcttgatggg

SEQ ID NO: 234 - DNA, 20 bp, synthetic construct
  source 1..20: mol_type = other DNA
cttccttgacctcgatgctg

SEQ ID NO: 235 - DNA, 20 bp, synthetic construct
  source 1..20: mol_type = other DNA
ttcccgctcttctcaccgag

SEQ ID NO: 236 - DNA, 20 bp, synthetic construct
  source 1..20: mol_type = other DNA
tccgcccagggctcttacag

SEQ ID NO: 237 - DNA, 20 bp, synthetic construct
  source 1..20: mol_type = other DNA
tggtggtgctccttcttggg

SEQ ID NO: 238 - DNA, 20 bp, synthetic construct
  source 1..20: mol_type = other DNA
cggagctctcgggctcaggt

SEQ ID NO: 239 - DNA, 20 bp, synthetic construct
  source 1..20: mol_type = other DNA
agcctcctctgggcatcttc

SEQ ID NO: 240 - DNA, 20 bp, synthetic construct
  source 1..20: mol_type = other DNA
cgggctgagtcttagctggc

SEQ ID NO: 241 - DNA, 20 bp, synthetic construct
  source 1..20: mol_type = other DNA
ggcggtggcaaccgcgggct

SEQ ID NO: 242 - DNA, 20 bp, synthetic construct
  source 1..20: mol_type = other DNA
tctgcggccgtggcggcggt

SEQ ID NO: 243 - DNA, 20 bp, synthetic construct
  source 1..20: mol_type = other DNA
cccctcggtgtttgtacttt

SEQ ID NO: 244 - DNA, 20 bp, synthetic construct
  source 1..20: mol_type = other DNA
ggaggatgaaacaatgtctt

SEQ ID NO: 245 - DNA, 20 bp, synthetic construct
  source 1..20: mol_type = other DNA
tccacaggctcctctctgtt

SEQ ID NO: 246 - DNA, 20 bp, synthetic construct
  source 1..20: mol_type = other DNA
ccgtgtaaagtcagctaact

SEQ ID NO: 247 - DNA, 20 bp, synthetic construct
  source 1..20: mol_type = other DNA
tttattcttgttggtttgct

SEQ ID NO: 248 - DNA, 20 bp, synthetic construct
  source 1..20: mol_type = other DNA
cctacccataaggagaagag

SEQ ID NO: 249 - DNA, 20 bp, synthetic construct
  source 1..20: mol_type = other DNA
tatttcagttaatcgggaag

SEQ ID NO: 250 - DNA, 20 bp, synthetic construct
  source 1..20: mol_type = other DNA
acagccctctctccgagagg

SEQ ID NO: 251 - DNA, 20 bp, synthetic construct
  source 1..20: mol_type = other DNA
cggcggcggccattttccgg

SEQ ID NO: 252 - DNA, 20 bp, synthetic construct
  source 1..20: mol_type = other DNA
tggagcagtctctcctcctc

SEQ ID NO: 253 - DNA, 20 bp, synthetic construct
  source 1..20: mol_type = other DNA
ttcatggaatgggcgagaag

SEQ ID NO: 254 - DNA, 20 bp, synthetic construct
  source 1..20: mol_type = other DNA
acagaggcagggcaggcacg

SEQ ID NO: 255 - DNA, 20 bp, synthetic construct
  source 1..20: mol_type = other DNA
aagattcatgcttgttagaa

SEQ ID NO: 256 - DNA, 20 bp, synthetic construct
  source 1..20: mol_type = other DNA
tcaaagcaggaactggtgag

SEQ ID NO: 257 - DNA, 20 bp, synthetic construct
  source 1..20: mol_type = other DNA
ggtctacagaagcaaggtgt

SEQ ID NO: 258 - DNA, 20 bp, synthetic construct
  source 1..20: mol_type = other DNA
catcccagctaccatggaat

SEQ ID NO: 259 - DNA, 20 bp, synthetic construct
  source 1..20: mol_type = other DNA
caccatcctgaggccaggca

SEQ ID NO: 260 - DNA, 20 bp, synthetic construct
  source 1..20: mol_type = other DNA
taacttttttctattattat

SEQ ID NO: 261 - DNA, 20 bp, synthetic construct
  source 1..20: mol_type = other DNA
acagtcacagaacaacaaag

SEQ ID NO: 262 - DNA, 20 bp, synthetic construct
  source 1..20: mol_type = other DNA
ggcctaattttttatctttg

SEQ ID NO: 263 - DNA, 20 bp, synthetic construct
  source 1..20: mol_type = other DNA
acagggttgtagccatcagc

SEQ ID NO: 264 - DNA, 20 bp, synthetic construct
  source 1..20: mol_type = other DNA
gatcactggaacacaatggt

SEQ ID NO: 265 - DNA, 20 bp, synthetic construct
  source 1..20: mol_type = other DNA
ggaagagaaaagaagggcac

SEQ ID NO: 266 - DNA, 20 bp, synthetic construct
  source 1..20: mol_type = other DNA
catttaataaataaatccct

SEQ ID NO: 267 - DNA, 20 bp, synthetic construct
  source 1..20: mol_type = other DNA
tttaccagtgccatttttcc

SEQ ID NO: 268 - DNA, 20 bp, synthetic construct
  source 1..20: mol_type = other DNA
cagcaaatttctgtggtttt

SEQ ID NO: 269 - DNA, 20 bp, synthetic construct
  source 1..20: mol_type = other DNA
gctctcagaccagaccagac

SEQ ID NO: 270 - DNA, 20 bp, synthetic construct
  source 1..20: mol_type = other DNA
acagctgatgaggagggtgg

SEQ ID NO: 271 - DNA, 20 bp, synthetic construct
  source 1..20: mol_type = other DNA
tacacaaatactaagccaca

SEQ ID NO: 272 - DNA, 20 bp, synthetic construct
  source 1..20: mol_type = other DNA
actgccaccaccatgactaa

SEQ ID NO: 273 - DNA, 20 bp, synthetic construct
  source 1..20: mol_type = other DNA
gttagaagttgattttttct

SEQ ID NO: 274 - DNA, 20 bp, synthetic construct
  source 1..20: mol_type = other DNA
atactcacatggtggagaaa

SEQ ID NO: 275 - DNA, 20 bp, synthetic construct
  source 1..20: mol_type = other DNA
gagaagaatggaagggagaa

SEQ ID NO: 276 - DNA, 20 bp, synthetic construct
  source 1..20: mol_type = other DNA
tagagggttggaggaacagg

SEQ ID NO: 277 - DNA, 20 bp, synthetic construct
  source 1..20: mol_type = other DNA
cttagaacaaagagaagaat

SEQ ID NO: 278 - DNA, 20 bp, synthetic construct
  source 1..20: mol_type = other DNA
gacactgacactgtgcatga

SEQ ID NO: 279 - DNA, 20 bp, synthetic construct
  source 1..20: mol_type = other DNA
ggagttaccatatgacctgg

SEQ ID NO: 280 - DNA, 20 bp, synthetic construct
  source 1..20: mol_type = other DNA
cgtaagcttctagcaaggag

SEQ ID NO: 281 - DNA, 20 bp, synthetic construct
  source 1..20: mol_type = other DNA
ggtaaaaatgataaaaaacg

SEQ ID NO: 282 - DNA, 20 bp, synthetic construct
  source 1..20: mol_type = other DNA
agccttctcctgcctcagct

SEQ ID NO: 283 - DNA, 20 bp, synthetic construct
  source 1..20: mol_type = other DNA
agaagcagcagccacctgcg

SEQ ID NO: 284 - DNA, 20 bp, synthetic construct
  source 1..20: mol_type = other DNA
tggtcttctgacttttcttc

SEQ ID NO: 285 - DNA, 20 bp, synthetic construct
  source 1..20: mol_type = other DNA
cacctttttaaacttgaggg

SEQ ID NO: 286 - DNA, 20 bp, synthetic construct
  source 1..20: mol_type = other DNA
tttctcttctttcttatctt

SEQ ID NO: 287 - DNA, 20 bp, synthetic construct
  source 1..20: mol_type = other DNA
tcatgcttgccctctttctc

SEQ ID NO: 288 - DNA, 20 bp, synthetic construct
  source 1..20: mol_type = other DNA
tgatggctgcacgggctcat

SEQ ID NO: 289 - DNA, 20 bp, synthetic construct
  source 1..20: mol_type = other DNA
cagcagagtggtgggctgat

SEQ ID NO: 290 - DNA, 20 bp, synthetic construct
  source 1..20: mol_type = other DNA
tgatgtctctgctttgcctg

SEQ ID NO: 291 - DNA, 20 bp, synthetic construct
  source 1..20: mol_type = other DNA
cagaagcttccggcacagcc

SEQ ID NO: 292 - DNA, 20 bp, synthetic construct
  source 1..20: mol_type = other DNA
gggtccccggtcacggatga

SEQ ID NO: 293 - DNA, 20 bp, synthetic construct
  source 1..20: mol_type = other DNA
gcttaagcttccgtgtccag

SEQ ID NO: 294 - DNA, 20 bp, synthetic construct
  source 1..20: mol_type = other DNA
atacttcccagcagagcggc

SEQ ID NO: 295 - DNA, 20 bp, synthetic construct
  source 1..20: mol_type = other DNA
agcaaccaaagagtcaggcc

SEQ ID NO: 296 - DNA, 20 bp, synthetic construct
  source 1..20: mol_type = other DNA
actttagagcgaaaggcttt

SEQ ID NO: 297 - DNA, 20 bp, synthetic construct
  source 1..20: mol_type = other DNA
ttttcgaagtacgcaatcaa

SEQ ID NO: 298 - DNA, 20 bp, synthetic construct
  source 1..20: mol_type = other DNA
ccagggatgtgtcgcctacc

SEQ ID NO: 299 - DNA, 20 bp, synthetic construct
  source 1..20: mol_type = other DNA
ccagttaccgtgaagtcaaa

SEQ ID NO: 300 - DNA, 20 bp, synthetic construct
  source 1..20: mol_type = other DNA
tgggcttcttaggtggtttc

SEQ ID NO: 301 - DNA, 20 bp, synthetic construct
  source 1..20: mol_type = other DNA
gtggtgccgctccctttggg

SEQ ID NO: 302 - DNA, 20 bp, synthetic construct
  source 1..20: mol_type = other DNA
tctccaggacccttttcacc

SEQ ID NO: 303 - DNA, 20 bp, synthetic construct
  source 1..20: mol_type = other DNA
gacaaggagcttcccaggac

SEQ ID NO: 304 - DNA, 20 bp, synthetic construct
  source 1..20: mol_type = other DNA
ccctggcgaagtttgaaaag

SEQ ID NO: 305 - DNA, 20 bp, synthetic construct
  source 1..20: mol_type = other DNA
cccctcagccttgccccctg

SEQ ID NO: 306 - DNA, 20 bp, synthetic construct
  source 1..20: mol_type = other DNA
tgggtggatgtggtggcccc

SEQ ID NO: 307 - DNA, 20 bp, synthetic construct
  source 1..20: mol_type = other DNA
cggcctcagcttttcgcttc

SEQ ID NO: 308 - DNA, 20 bp, synthetic construct
  source 1..20: mol_type = other DNA
tcggccccgtttcttgggaa

SEQ ID NO: 309 - DNA, 20 bp, synthetic construct
  source 1..20: mol_type = other DNA
gcggcagcggctgccaccac

SEQ ID NO: 310 - DNA, 20 bp, synthetic construct
  source 1..20: mol_type = other DNA
aagactccttcacggctttc

SEQ ID NO: 311 - DNA, 20 bp, synthetic construct
  source 1..20: mol_type = other DNA
ggtctcctgcacagatcgga

SEQ ID NO: 312 - DNA, 20 bp, synthetic construct
  source 1..20: mol_type = other DNA
gctgaccgtctcccgggtct

SEQ ID NO: 313 - DNA, 20 bp, synthetic construct
  source 1..20: mol_type = other DNA
cgagggtggacaccagcagg

SEQ ID NO: 314 - DNA, 20 bp, synthetic construct
  source 1..20: mol_type = other DNA
acaggtcttcagtcctttcc

SEQ ID NO: 315 - DNA, 20 bp, synthetic construct
  source 1..20: mol_type = other DNA
ctgctctccttgcttttccg

SEQ ID NO: 316 - DNA, 20 bp, synthetic construct
  source 1..20: mol_type = other DNA
ctgagtggtggtgatggtgg

SEQ ID NO: 317 - DNA, 20 bp, synthetic construct
  source 1..20: mol_type = other DNA
cttctcctctttgcagacgc

SEQ ID NO: 318 - DNA, 20 bp, synthetic construct
  source 1..20: mol_type = other DNA
ccgtcgctctccagtgagcc

SEQ ID NO: 319 - DNA, 20 bp, synthetic construct
  source 1..20: mol_type = other DNA
ggcaaccgcgggctgagtct

SEQ ID NO: 320 - DNA, 20 bp, synthetic construct
  source 1..20: mol_type = other DNA
ccgtggcggcggtggcaacc

SEQ ID NO: 321 - DNA, 20 bp, synthetic construct
  source 1..20: mol_type = other DNA
tacttttctgcggccgtggc

SEQ ID NO: 322 - DNA, 20 bp, synthetic construct
  source 1..20: mol_type = other DNA
tctttgcgctctccctcccc

SEQ ID NO: 323 - DNA, 20 bp, synthetic construct
  source 1..20: mol_type = other DNA
tgtttggccttggcatggag

SEQ ID NO: 324 - DNA, 20 bp, synthetic construct
  source 1..20: mol_type = other DNA
aactctctcggtcacgggcg

SEQ ID NO: 325 - DNA, 20 bp, synthetic construct
  source 1..20: mol_type = other DNA
tgctttgcaatccgctccgt

SEQ ID NO: 326 - DNA, 20 bp, synthetic construct
  source 1..20: mol_type = other DNA
agagacaacagctgccttta

SEQ ID NO: 327 - DNA, 20 bp, synthetic construct
  source 1..20: mol_type = other DNA
gaagctttgtcagagcccta

SEQ ID NO: 328 - DNA, 20 bp, synthetic construct
  source 1..20: mol_type = other DNA
ccttccctgaaggttcctcc

SEQ ID NO: 329 - DNA, 20 bp, synthetic construct
  source 1..20: mol_type = other DNA
  modified_base 1: mod_base = OTHER; note = 2'-O-methoxyethyl guanosine 3'-phosphorothioate
  modified_base 2: mod_base = OTHER; note = 2'-O-methoxyethyl guanosine 3'-phosphodiester
  modified_base 3..4: mod_base = OTHER; note = 2'-O-methoxyethyl adenosine 3'-phosphodiester
  modified_base 5: mod_base = OTHER; note = 2'-O-methoxyethyl 5-methylcytidine 3'-phosphodiester
  modified_base 6: mod_base = OTHER; note = 2'-deoxythymidine 3'-phosphorothioate
  modified_base 7..8: mod_base = OTHER; note = 2'-deoxyguanosine 3'-phosphorothioate
  modified_base 9: mod_base = OTHER; note = 2'-deoxythymidine 3'-phosphorothioate
  modified_base 10: mod_base = OTHER; note = 2'-deoxyguanosine 3'-phosphorothioate
  modified_base 11: mod_base = OTHER; note = 2'-deoxyadenosine 3'-phosphorothioate
  modified_base 12: mod_base = OTHER; note = 2'-deoxyguanosine 3'-phosphorothioate
  modified_base 13: mod_base = OTHER; note = 2'-deoxythymidine 3'-phosphorothioate
  modified_base 14: mod_base = OTHER; note = 5-methyl-2'-deoxycytidine 3'-phosphorothioate
  modified_base 15: mod_base = OTHER; note = 2'-deoxythymidine 3'-phosphorothioate
  modified_base 16: mod_base = OTHER; note = 2'-O-methoxyethyl guanosine 3'-phosphodiester
  modified_base 17: mod_base = OTHER; note = 2'-O-methoxyethyl thymidine 3'-phosphodiester
  modified_base 18: mod_base = OTHER; note = 2'-O-methoxyethyl adenosine 3'-phosphorothioate
  modified_base 19: mod_base = OTHER; note = 2'-O-methoxyethyl thymidine 3'-phosphorothioate
  modified_base 20: mod_base = OTHER; note = 2'-O-methoxyethyl thymidine
ggaactggtgagtctgtatt

SEQ ID NO: 330 - DNA, 20 bp, synthetic construct
  source 1..20: mol_type = other DNA
  modified_base 1: mod_base = OTHER; note = 2'-O-methoxyethyl guanosine 3'-phosphorothioate
  modified_base 2..3: mod_base = OTHER; note = 2'-O-methoxyethyl adenosine 3'-phosphodiester
  modified_base 4: mod_base = OTHER; note = 2'-O-methoxyethyl guanosine 3'-phosphodiester
  modified_base 5: mod_base = OTHER; note = 2'-O-methoxyethyl 5-methylcytidine 3'-phosphodiester
  modified_base 6..7: mod_base = OTHER; note = 2'-deoxyadenosine 3'-phosphorothioate
  modified_base 8..9: mod_base = OTHER; note = 2'-deoxyguanosine 3'-phosphorothioate
  modified_base 10: mod_base = OTHER; note = 2'-deoxythymidine 3'-phosphorothioate
  modified_base 11: mod_base = OTHER; note = 2'-deoxyguanosine 3'-phosphorothioate
  modified_base 12: mod_base = OTHER; note = 2'-deoxythymidine 3'-phosphorothioate
  modified_base 13: mod_base = OTHER; note = 2'-deoxyadenosine 3'-phosphorothioate
  modified_base 14..15: mod_base = OTHER; note = 2'-deoxythymidine 3'-phosphorothioate
  modified_base 16: mod_base = OTHER; note = 2'-O-methoxyethyl 5-methylcytidine 3'-phosphodiester
  modified_base 17: mod_base = OTHER; note = 2'-O-methoxyethyl thymidine 3'-phosphodiester
  modified_base 18..19: mod_base = OTHER; note = 2'-O-methoxyethyl guanosine 3'-phosphorothioate
  modified_base 20: mod_base = OTHER; note = 2'-O-methoxyethyl guanosine
gaagcaaggtgtattctggg

SEQ ID NO: 331 - DNA, 20 bp, synthetic construct
  source 1..20: mol_type = other DNA
  modified_base 1: mod_base = OTHER; note = 2'-O-methoxyethyl 5-methylcytidine 3'-phosphorothioate
  modified_base 2: mod_base = OTHER; note = 2'-O-methoxyethyl thymidine 3'-phosphodiester
  modified_base 3: mod_base = OTHER; note = 2'-O-methoxyethyl adenosine 3'-phosphodiester
  modified_base 4..5: mod_base = OTHER; note = 2'-O-methoxyethyl 5-methylcytidine 3'-phosphodiester
  modified_base 6: mod_base = OTHER; note = 2'-deoxyadenosine 3'-phosphorothioate
  modified_base 7: mod_base = OTHER; note = 2'-deoxythymidine 3'-phosphorothioate
  modified_base 8..9: mod_base = OTHER; note = 2'-deoxyguanosine 3'-phosphorothioate
  modified_base 10..11: mod_base = OTHER; note = 2'-deoxyadenosine 3'-phosphorothioate
  modified_base 12: mod_base = OTHER; note = 2'-deoxythymidine 3'-phosphorothioate
  modified_base 13..14: mod_base = OTHER; note = 5-methyl-2'-deoxycytidine 3'-phosphorothioate
  modified_base 15: mod_base = OTHER; note = 2'-deoxythymidine 3'-phosphorothioate
  modified_base 16: mod_base = OTHER; note = 2'-O-methoxyethyl guanosine 3'-phosphodiester
  modified_base 17: mod_base = OTHER; note = 2'-O-methoxyethyl thymidine 3'-phosphodiester
  modified_base 18: mod_base = OTHER; note = 2'-O-methoxyethyl thymidine 3'-phosphorothioate
  modified_base 19: mod_base = OTHER; note = 2'-O-methoxyethyl guanosine 3'-phosphorothioate
  modified_base 20: mod_base = OTHER; note = 2'-O-methoxyethyl guanosine
ctaccatggaatcctgttgg

SEQ ID NO: 332 - DNA, 20 bp, synthetic construct
  source 1..20: mol_type = other DNA
  modified_base 1: mod_base = OTHER; note = 2'-O-methoxyethyl adenosine 3'-phosphorothioate
  modified_base 2: mod_base = OTHER; note = 2'-O-methoxyethyl thymidine 3'-phosphodiester
  modified_base 3: mod_base = OTHER; note = 2'-O-methoxyethyl guanosine 3'-phosphodiester
  modified_base 4: mod_base = OTHER; note = 2'-O-methoxyethyl thymidine 3'-phosphodiester
  modified_base 5: mod_base = OTHER; note = 2'-O-methoxyethyl 5-methylcytidine 3'-phosphodiester
  modified_base 6: mod_base = OTHER; note = 2'-deoxyadenosine 3'-phosphorothioate
  modified_base 7: mod_base = OTHER; note = 5-methyl-2'-deoxycytidine 3'-phosphorothioate
  modified_base 8: mod_base = OTHER; note = 2'-deoxyadenosine 3'-phosphorothioate
  modified_base 9: mod_base = OTHER; note = 2'-deoxythymidine 3'-phosphorothioate
  modified_base 10: mod_base = OTHER; note = 5-methyl-2'-deoxycytidine 3'-phosphorothioate
  modified_base 11..13: mod_base = OTHER; note = 2'-deoxyadenosine 3'-phosphorothioate
  modified_base 14: mod_base = OTHER; note = 2'-deoxyguanosine 3'-phosphorothioate
  modified_base 15: mod_base = OTHER; note = 5-methyl-2'-deoxycytidine 3'-phosphorothioate
  modified_base 16: mod_base = OTHER; note = 2'-O-methoxyethyl adenosine 3'-phosphodiester
  modified_base 17: mod_base = OTHER; note = 2'-O-methoxyethyl guanosine 3'-phosphodiester
  modified_base 18: mod_base = OTHER; note = 2'-O-methoxyethyl guanosine 3'-phosphorothioate
  modified_base 19: mod_base = OTHER; note = 2'-O-methoxyethyl adenosine 3'-phosphorothioate
  modified_base 20: mod_base = OTHER; note = 2'-O-methoxyethyl adenosine
atgtcacatcaaagcaggaa

SEQ ID NO: 333 - DNA, 20 bp, synthetic construct
  source 1..20: mol_type = other DNA
  modified_base 1: mod_base = OTHER; note = 2'-O-methoxyethyl thymidine 3'-phosphorothioate
  modified_base 2: mod_base = OTHER; note = 2'-O-methoxyethyl thymidine 3'-phosphodiester
  modified_base 3..4: mod_base = OTHER; note = 2'-O-methoxyethyl guanosine 3'-phosphodiester
  modified_base 5: mod_base = OTHER; note = 2'-O-methoxyethyl adenosine 3'-phosphodiester
  modified_base 6: mod_base = OTHER; note = 2'-deoxyguanosine 3'-phosphorothioate
  modified_base 7: mod_base = OTHER; note = 5-methyl-2'-deoxycytidine 3'-phosphorothioate
  modified_base 8: mod_base = OTHER; note = 2'-deoxythymidine 3'-phosphorothioate
  modified_base 9..10: mod_base = OTHER; note = 2'-deoxyguanosine 3'-phosphorothioate
  modified_base 11: mod_base = OTHER; note = 2'-deoxythymidine 3'-phosphorothioate
  modified_base 12: mod_base = OTHER; note = 5-methyl-2'-deoxycytidine 3'-phosphorothioate
  modified_base 13: mod_base = OTHER; note = 2'-deoxythymidine 3'-phosphorothioate
  modified_base 14: mod_base = OTHER; note = 2'-deoxyadenosine 3'-phosphorothioate
  modified_base 15: mod_base = OTHER; note = 5-methyl-2'-deoxycytidine 3'-phosphorothioate
  modified_base 16: mod_base = OTHER; note = 2'-O-methoxyethyl adenosine 3'-phosphodiester
  modified_base 17: mod_base = OTHER; note = 2'-O-methoxyethyl guanosine 3'-phosphodiester
  modified_base 18..19: mod_base = OTHER; note = 2'-O-methoxyethyl adenosine 3'-phosphorothioate
  modified_base 20: mod_base = OTHER; note = 2'-O-methoxyethyl guanosine
ttggagctggtctacagaag

SEQ ID NO: 334 - DNA, 20 bp, synthetic construct
  source 1..20: mol_type = other DNA
  modified_base 1: mod_base = OTHER; note = 2'-O-methoxyethyl adenosine 3'-phosphorothioate
  modified_base 2: mod_base = OTHER; note = 2'-O-methoxyethyl guanosine 3'-phosphodiester
  modified_base 3..5: mod_base = OTHER; note = 2'-O-methoxyethyl 5-methylcytidine 3'-phosphodiester
  modified_base 6: mod_base = OTHER; note = 2'-deoxythymidine 3'-phosphorothioate
  modified_base 7..8: mod_base = OTHER; note = 2'-deoxyadenosine 3'-phosphorothioate
  modified_base 9: mod_base = OTHER; note = 5-methyl-2'-deoxycytidine 3'-phosphorothioate
  modified_base 10: mod_base = OTHER; note = 2'-deoxyadenosine 3'-phosphorothioate
  modified_base 11: mod_base = OTHER; note = 2'-deoxythymidine 3'-phosphorothioate
  modified_base 12..14: mod_base = OTHER; note = 5-methyl-2'-deoxycytidine 3'-phosphorothioate
  modified_base 15: mod_base = OTHER; note = 2'-deoxyadenosine 3'-phosphorothioate
  modified_base 16: mod_base = OTHER; note = 2'-O-methoxyethyl guanosine 3'-phosphodiester
  modified_base 17: mod_base = OTHER; note = 2'-O-methoxyethyl 5-methylcytidine 3'-phosphodiester
  modified_base 18: mod_base = OTHER; note = 2'-O-methoxyethyl thymidine 3'-phosphorothioate
  modified_base 19: mod_base = OTHER; note = 2'-O-methoxyethyl adenosine 3'-phosphorothioate
  modified_base 20: mod_base = OTHER; note = 2'-O-methoxyethyl 5-methylcytidine
agccctaacatcccagctac

SEQ ID NO: 335 - DNA, 20 bp, synthetic construct
  source 1..20: mol_type = other DNA
  modified_base 1: mod_base = OTHER; note = 2'-O-methoxyethyl thymidine 3'-phosphorothioate
  modified_base 2: mod_base = OTHER; note = 2'-O-methoxyethyl guanosine 3'-phosphodiester
  modified_base 3: mod_base = OTHER; note = 2'-O-methoxyethyl adenosine 3'-phosphodiester
  modified_base 4: mod_base = OTHER; note = 2'-O-methoxyethyl guanosine 3'-phosphodiester
  modified_base 5: mod_base = OTHER; note = 2'-O-methoxyethyl thymidine 3'-phosphodiester
  modified_base 6: mod_base = OTHER; note = 5-methyl-2'-deoxycytidine 3'-phosphorothioate
  modified_base 7: mod_base = OTHER; note = 2'-deoxythymidine 3'-phosphorothioate
  modified_base 8: mod_base = OTHER; note = 2'-deoxyguanosine 3'-phosphorothioate
  modified_base 9: mod_base = OTHER; note = 2'-deoxythymidine 3'-phosphorothioate
  modified_base 10: mod_base = OTHER; note = 2'-deoxyadenosine 3'-phosphorothioate
  modified_base 11..15: mod_base = OTHER; note = 2'-deoxythymidine 3'-phosphorothioate
  modified_base 16: mod_base = OTHER; note = 2'-O-methoxyethyl adenosine 3'-phosphodiester
  modified_base 17: mod_base = OTHER; note = 2'-O-methoxyethyl thymidine 3'-phosphodiester
  modified_base 18..19: mod_base = OTHER; note = 2'-O-methoxyethyl guanosine 3'-phosphorothioate
  modified_base 20: mod_base = OTHER; note = 2'-O-methoxyethyl adenosine
tgagtctgtatttttatgga

SEQ ID NO: 336 - DNA, 20 bp, synthetic construct
  source 1..20: mol_type = other DNA
  modified_base 1: mod_base = OTHER; note = 2'-O-methoxyethyl guanosine 3'-phosphorothioate
  modified_base 2: mod_base = OTHER; note = 2'-O-methoxyethyl guanosine 3'-phosphodiester
  modified_base 3: mod_base = OTHER; note = 2'-O-methoxyethyl adenosine 3'-phosphodiester
  modified_base 4: mod_base = OTHER; note = 2'-O-methoxyethyl guanosine 3'-phosphodiester
  modified_base 5: mod_base = OTHER; note = 2'-O-methoxyethyl thymidine 3'-phosphodiester
  modified_base 6: mod_base = OTHER; note = 5-methyl-2'-deoxycytidine 3'-phosphorothioate
  modified_base 7: mod_base = OTHER; note = 2'-deoxyadenosine 3'-phosphorothioate
  modified_base 8: mod_base = OTHER; note = 5-methyl-2'-deoxycytidine 3'-phosphorothioate
  modified_base 9: mod_base = OTHER; note = 2'-deoxyadenosine 3'-phosphorothioate
  modified_base 10: mod_base = OTHER; note = 2'-deoxythymidine 3'-phosphorothioate
  modified_base 11: mod_base = OTHER; note = 2'-deoxyguanosine 3'-phosphorothioate
  modified_base 12: mod_base = OTHER; note = 2'-deoxythymidine 3'-phosphorothioate
  modified_base 13: mod_base = OTHER; note = 5-methyl-2'-deoxycytidine 3'-phosphorothioate
  modified_base 14: mod_base = OTHER; note = 2'-deoxyadenosine 3'-phosphorothioate
  modified_base 15: mod_base = OTHER; note = 5-methyl-2'-deoxycytidine 3'-phosphorothioate
  modified_base 16: mod_base = OTHER; note = 2'-O-methoxyethyl adenosine 3'-phosphodiester
  modified_base 17: mod_base = OTHER; note = 2'-O-methoxyethyl thymidine 3'-phosphodiester
  modified_base 18: mod_base = OTHER; note = 2'-O-methoxyethyl 5-methylcytidine 3'-phosphorothioate
  modified_base 19: mod_base = OTHER; note = 2'-O-methoxyethyl adenosine 3'-phosphorothioate
  modified_base 20: mod_base = OTHER; note = 2'-O-methoxyethyl adenosine
ggagtcacatgtcacatcaa

SEQ ID NO: 337 - DNA, 20 bp, synthetic construct
  source 1..20: mol_type = other DNA
  modified_base 1: mod_base = OTHER; note = 2'-O-methoxyethyl guanosine 3'-phosphorothioate
  modified_base 2..3: mod_base = OTHER; note = 2'-O-methoxyethyl adenosine 3'-phosphodiester
  modified_base 4: mod_base = OTHER; note = 2'-O-methoxyethyl thymidine 3'-phosphodiester
  modified_base 5: mod_base = OTHER; note = 2'-O-methoxyethyl 5-methylcytidine 3'-phosphodiester
  modified_base 6: mod_base = OTHER; note = 5-methyl-2'-deoxycytidine 3'-phosphorothioate
  modified_base 7: mod_base = OTHER; note = 2'-deoxythymidine 3'-phosphorothioate
  modified_base 8: mod_base = OTHER; note = 2'-deoxyguanosine 3'-phosphorothioate
  modified_base 9..10: mod_base = OTHER; note = 2'-deoxythymidine 3'-phosphorothioate
  modified_base 11..12: mod_base = OTHER; note = 2'-deoxyguanosine 3'-phosphorothioate
  modified_base 13: mod_base = OTHER; note = 2'-deoxyadenosine 3'-phosphorothioate
  modified_base 14: mod_base = OTHER; note = 2'-deoxyguanosine 3'-phosphorothioate
  modified_base 15: mod_base = OTHER; note = 5-methyl-2'-deoxycytidine 3'-phosphorothioate
  modified_base 16: mod_base = OTHER; note = 2'-O-methoxyethyl thymidine 3'-phosphodiester
  modified_base 17: mod_base = OTHER; note = 2'-O-methoxyethyl guanosine 3'-phosphodiester
  modified_base 18: mod_base = OTHER; note = 2'-O-methoxyethyl guanosine 3'-phosphorothioate
  modified_base 19: mod_base = OTHER; note = 2'-O-methoxyethyl thymidine 3'-phosphorothioate
  modified_base 20: mod_base = OTHER; note = 2'-O-methoxyethyl 5-methylcytidine
gaatcctgttggagctggtc

SEQ ID NO: 338 - DNA, 20 bp, synthetic construct
  source 1..20: mol_type = other DNA
  modified_base 1: mod_base = OTHER; note = 2'-O-methoxyethyl thymidine 3'-phosphorothioate
  modified_base 2: mod_base = OTHER; note = 2'-O-methoxyethyl 5-methylcytidine 3'-phosphodiester
  modified_base 3..5: mod_base = OTHER; note = 2'-O-methoxyethyl adenosine 3'-phosphodiester
  modified_base 6: mod_base = OTHER; note = 2'-deoxyguanosine 3'-phosphorothioate
  modified_base 7: mod_base = OTHER; note = 5-methyl-2'-deoxycytidine 3'-phosphorothioate
  modified_base 8: mod_base = OTHER; note = 2'-deoxyadenosine 3'-phosphorothioate
  modified_base 9..10: mod_base = OTHER; note = 2'-deoxyguanosine 3'-phosphorothioate
  modified_base 11..12: mod_base = OTHER; note = 2'-deoxyadenosine 3'-phosphorothioate
  modified_base 13: mod_base = OTHER; note = 5-methyl-2'-deoxycytidine 3'-phosphorothioate
  modified_base 14: mod_base = OTHER; note = 2'-deoxythymidine 3'-phosphorothioate
  modified_base 15: mod_base = OTHER; note = 2'-deoxyguanosine 3'-phosphorothioate
  modified_base 16: mod_base = OTHER; note = 2'-O-methoxyethyl guanosine 3'-phosphodiester
  modified_base 17: mod_base = OTHER; note = 2'-O-methoxyethyl thymidine 3'-phosphodiester
  modified_base 18: mod_base = OTHER; note = 2'-O-methoxyethyl guanosine 3'-phosphorothioate
  modified_base 19: mod_base = OTHER; note = 2'-O-methoxyethyl adenosine 3'-phosphorothioate
  modified_base 20: mod_base = OTHER; note = 2'-O-methoxyethyl guanosine
tcaaagcaggaactggtgag

SEQ ID NO: 339 - DNA, 20 bp, synthetic construct
  source 1..20: mol_type = other DNA
  modified_base 1: mod_base = OTHER; note = 2'-O-methoxyethyl guanosine 3'-phosphorothioate
  modified_base 2: mod_base = OTHER; note = 2'-O-methoxyethyl guanosine 3'-phosphodiester
  modified_base 3: mod_base = OTHER; note = 2'-O-methoxyethyl thymidine 3'-phosphodiester
  modified_base 4: mod_base = OTHER; note = 2'-O-methoxyethyl 5-methylcytidine 3'-phosphodiester
  modified_base 5: mod_base = OTHER; note = 2'-O-methoxyethyl thymidine 3'-phosphodiester
  modified_base 6: mod_base = OTHER; note = 2'-deoxyadenosine 3'-phosphorothioate
  modified_base 7: mod_base = OTHER; note = 5-methyl-2'-deoxycytidine 3'-phosphorothioate
  modified_base 8: mod_base = OTHER; note = 2'-deoxyadenosine 3'-phosphorothioate
  modified_base 9: mod_base = OTHER; note = 2'-deoxyguanosine 3'-phosphorothioate
  modified_base 10..11: mod_base = OTHER; note = 2'-deoxyadenosine 3'-phosphorothioate
  modified_base 12: mod_base = OTHER; note = 2'-deoxyguanosine 3'-phosphorothioate
  modified_base 13: mod_base = OTHER; note = 5-methyl-2'-deoxycytidine 3'-phosphorothioate
  modified_base 14..15: mod_base = OTHER; note = 2'-deoxyadenosine 3'-phosphorothioate
  modified_base 16..17: mod_base = OTHER; note = 2'-O-methoxyethyl guanosine 3'-phosphodiester
  modified_base 18: mod_base = OTHER; note = 2'-O-methoxyethyl thymidine 3'-phosphorothioate
  modified_base 19: mod_base = OTHER; note = 2'-O-methoxyethyl guanosine 3'-phosphorothioate
  modified_base 20: mod_base = OTHER; note = 2'-O-methoxyethyl thymidine
ggtctacagaagcaaggtgt

SEQ ID NO: 340 - DNA, 20 bp, synthetic construct
  source 1..20: mol_type = other DNA
  modified_base 1: mod_base = OTHER; note = 2'-O-methoxyethyl 5-methylcytidine 3'-phosphorothioate
  modified_base 2: mod_base = OTHER; note = 2'-O-methoxyethyl adenosine 3'-phosphodiester
  modified_base 3: mod_base = OTHER; note = 2'-O-methoxyethyl thymidine 3'-phosphodiester
  modified_base 4..5: mod_base = OTHER; note = 2'-O-methoxyethyl 5-methylcytidine 3'-phosphodiester
  modified_base 6: mod_base = OTHER; note = 5-methyl-2'-deoxycytidine 3'-phosphorothioate
  modified_base 7: mod_base = OTHER; note = 2'-deoxyadenosine 3'-phosphorothioate
  modified_base 8: mod_base = OTHER; note = 2'-deoxyguanosine 3'-phosphorothioate
  modified_base 9: mod_base = OTHER; note = 5-methyl-2'-deoxycytidine 3'-phosphorothioate
  modified_base 10: mod_base = OTHER; note = 2'-deoxythymidine 3'-phosphorothioate
  modified_base 11: mod_base = OTHER; note = 2'-deoxyadenosine 3'-phosphorothioate
  modified_base 12..13: mod_base = OTHER; note = 5-methyl-2'-deoxycytidine 3'-phosphorothioate
  modified_base 14: mod_base = OTHER; note = 2'-deoxyadenosine 3'-phosphorothioate
  modified_base 15: mod_base = OTHER; note = 2'-deoxythymidine 3'-phosphorothioate
  modified_base 16..17: mod_base = OTHER; note = 2'-O-methoxyethyl guanosine 3'-phosphodiester
  modified_base 18..19: mod_base = OTHER; note = 2'-O-methoxyethyl adenosine 3'-phosphorothioate
  modified_base 20: mod_base = OTHER; note = 2'-O-methoxyethyl thymidine
catcccagctaccatggaat